European Patent Application EP 4 678 750 A1, published January 14, 2026. Title: Replicon DNA, cloning vector, screening kit, screening method, anti-Nobecovirus agent, Betacoronavirus growth inhibitor, pan-Betacoronavirus inhibitor, virus growth inhibitor, Hepatitis C virus growth inhibitor and screening method for therapeutic agent of virus infection. Applicant: Kagoshima University. Application WO. The sequence listing filed with the application follows.

SEQUENCE LISTING (32 sequences)

SEQ ID NO: 1 - DNA, 25080 bp, synthetic construct
  source 1..25080: mol_type = other DNA
gttgacattgattattgactagttattaatagtaatcaattacggggtcattagttcatagcccatatatggagttccgcgttacataacttacggtaaatggcccgcctggctgaccgcccaacgacccccgcccattgacgtcaataatgacgtatgttcccatagtaacgccaatagggactttccattgacgtcaatgggtggagtatttacggtaaactgcccacttggcagtacatcaagtgtatcatatgccaagtacgccccctattgacgtcaatgacggtaaatggcccgcctggcattatgcccagtacatgaccttatgggactttcctacttggcagtacatctacgtattagtcatcgctattaccatggtgatgcggttttggcagtacatcaatgggcgtggataggggtttgactcacggggatttccaagtctccaccccattgacgtcaatgggagtttgttttggcaccaaaatcaacgggactttccaaaatgtcgtaacaactccgccccattgacgcaaatgggcggtaggcgtgtacggtgggaggtctatataagcagagctcgtttagtgaaccgataaaaggtagtagctgcgtgctatcgccgatcctaacccccgtttcgtcttgtacgaatcactcttgaacgaacttaaaattgcatcatacgtcacggtaggtttcgtcttgctgtgcgtacgttgcacaccaattatagtggagctttttggttaagtacttcccccttgcgagcaacaggtgtcgtcctgtttgttagccctgcgcggtttcgtccgtgtagtgatggagggtgtgcctgacccacctaagcttaaaagtatggtggttaccactttgaagtggtgcgatccttttgctaatcccaacgtcactggttgggatattcctattgaggaggctctggaatatgcgaaacagcagttgcgcactccggaacctcagttggtgtttgtgccttattatttgagccatgcacctggtattagtggtgaccgcgttgtcataactgatagcatttggtacgctactaattttggatggcagcccattagggagcttgccatggataaggatggtgttcgttatggtaggggaggaacacatggtgttttgcttcccatgcaggacccgtcctttattatgggtgatattgatatccaaatccgtaagtacggtattggggccaactcaccgcctgatgtattaccgctctgggatgggttttcagacccaggtccggatgtggggccttatttagatttccctgataattgctgccctacaaagcctaaagcgaagaggggcggcgatgtttatctgtcagaccagtatggttttgacaataatggcatcttggtagaacctgttatgaagttactgggtgtcataaaatctgattttactctggaacagctattggctgcgctaggtaagtatcggactgaagatggatacgatttgcctgatggttacgtaaaggttgctattaaggtgggtcgtaaagctgtgcctgttttgaagcagtcaatttttactgttgtaggggttacagaacaactagtgccgggttattattacccgttttcaacatctagtgttgttgaacacactaagcctactaggggtggacctgtgggtaagacagttgaggctgttatgctcagtctttatggcaccaacaactacaatcctgcgacgcctgtggcgcgcttgaaatgtagttattgtgattattatggttggacacctcttaaggacataggcactgttaattgcctgtgtggtgcagagtttcaactcacgtcatcgtgcgtagatgcagagtctgcaggtgtgattaaaccaggttgtgtcatgttgttggacaagagtccaggcatgcgccttatacctggtaatcgcacatatgtgtcttttggtggcgctatatggtcgcctattggtaaagtcaatggtgtcactgtatgggttcctagagcctattctattgtggcaggtgagcactctggggccgtaggctcgggtgatacagttgccataaacaaggaacttgtggagtaccttattgaaggtattagagtggatgctgacacattggataaccccacttgtgccactttcatagctaatttagattgtgatactaaggctcccgttgtacatacggttgagtcattgcaggggctttgtttagctaacaagattatgttgggtgacaagccacttcctacagatgaattccatccctttatagtaggcttagcctaccatgtacagcgtgcttgctggtatggggccttggcatcccgtacatttgaagcttttagagattttgtccgtactgaagaagagcgctttgctcagtttttcggtaaagtgtgtgcacctataaatggttgcgtatacttagcttatacaactggacgtgtaactttgttttcagcgtatcaggtgttgaacacagccattgctaagagcaaagatgcttttggtggtgttgctgctatcgttgtggacatgttgaagccaattttggagtgggttttaaaaaagatgtccatagctaagggtgcttggcttccttatgcagagggtctgcttgcactgtttaaagcgcaatttaccgttgttaagggtaaatttcaatttttgcgcgcatctttgaattctaagtgtcacagtttgtgtgatttgcttactactattatgagtaagctgctcacatctgttaagtgggctggttgtaaggttgatgccttatatactggtacttattattacttttcacgaaaaggtgtgctcacagaagtgcagctatgtgctaagcgccttggcctgttgttaactcctaaacagcagaagatggaggttgaggtgcttgatggtgattttgatgcccctgtaacccttacagatttggaattagaggagtgtacaggtgtgttagaagaggtttttggagcttcagatgttaagttggttaagggtactttggtttctcttgccagcaagttgtttgtgcgtactgaggatggtttcctctaccgctatgttaaatctggtggcgttcttggtaaggctttcagattgcgtggcggtggtgtgagtaaagtgacctttggtgatgaggaggtgcataccatccctaatactgtaactgtaaattttagttatgacgtttgtgaaggactcgacgcaatccttgacaaggtcatggcgccttttcaggttgaagagggaactaagcttgaagatttagcttgtgtagttcaaaaggcagtctatgaaagattgtctgatttgttttcagactgtccagcagaactccgtcctataaatttggaggattttttgacgtctgaatgctttgtatacagtaaggactatgagaagatactcatgcctgagatgtatttttctttagaagatgctgtcccagttgatgacgagatggtagatgatatcgaagacaccgttgagcaagcctctgacagtgatgatcagtggcttggtgatgagggtgctgaggattgtgataatacaattcaagatgtagatgtggctacctctatgaccacgccttgtggttatacgaagattgctgaacacgtttacattaagtgcgctgatatagtgcaggaagcacgtaattattcgtatgcagtgcttgttaatgccgccaatgttaatttacatcatggcggtggtgtggcaggtgctcttaatagagccactaataatgctatgcaaaaagaatcaagtgagtacattaaggctaatggttccctgcagcctggtgggcatgtcctgctaagttcacacggtctggcctcgcatggtatcctacatgttgttggccccgataagaggttaggacaggatcttgccttgctggatgctgtgtatgctgcttacacaggttttgatagtgtattgacgccattagtgtcggctggcatttttggttttacagttgaagaatcactttgtagtctcgtaaaaaatgttgcgtgcactacttatgttgtggtttatgatagacagctatatgagcgtgctcttgctacatcgtttgatgtgccaggaccacagtctagtgtacagcatgtacctgctattgattgggcagaggctgtagaggtgcaggagtcaattgtggaccaagttgaaacccctagtttgggggccgtagatacggttgactccaatgctgatagcggtttaaatgaaaccgcgcgttcacctgagaatgtcgttggctctgtgccagacgatgtagttgcagatgttgaatcctgcgttagggatttggtgcgtcaggttgttaagaaggtaaagcgtgataagcgtccacctcctatagtacctcagcagacagttgaacaacagcctcaggagatttcatctcctggtgattgtaatactgtattagttgatgtggtttctatgtccttttctgcgatggtgaattttggaaaggagaagggcttgttaataccagttgttatagattatccagcatttttaaaggttttaaagcgtttttcgcctaaggaaggccttttctcgtctaatggttatgagttttacggttacagtcgtgataaaccattacatgaagttagcaaagatttgaattctttaggtagacccttgattatgataccgtttggttttatagttaacggtcaaaccctagcggtttctgcagttagtatgcgtggtcttaccgttccgcatactgttgttgtgccttcagaatctagtgtcccactatatagagcttactttaatggggtttttagtggtgacactacagctgttcaggattttgttgttgacattttgctcaacggcgctcgtgattgggacgttttacagactacttgtactgtagatcgtaaagtttataaaaccatttgtaagcgtggcaatacttatttgtgttttgatgacaccaatttgtatgccataacaggtgatgtggtacttaaatttgccacagtttctaaagcgcgggcttatttggagactaagctatgtgcaccagagcctttgattaaggttttgactacagtagacggtattaattatagtactgttttagtgtctactgcacagagttacagggcacaaataggtacggtgttttgtgatggccacgattggtctaataagaatccgatgcccacggacgagggtactcatttgtataagcaggataacttctcatctgcagaagttactgctattcgtgagtattatggtgttgatgactctaatatcatagcgcgtgctatgagtattaggaaaactgtacagacatggccttatacggttgtggatggtagagttttgcttgctcaacgagattctaattgctatcttaatgtagctatctctttacttcaagatatagatgtgtcctttagtacaccatgggtgtgtagggcctatgatgcactaaaaggtggtaatcctctgcctatggcggaagttcttatagcactgggtaaggctactcctggtgttagtgatgacgctcatatggttttgtctgcagtattaaatcatggtactgttacggcgcgccgtgtgatgcaaactgtttgtgaacattgtggtgttagccaaatggtttttacaggcactgatgcttgtacattttacggctcggttgttttagatgatttatatgcaccagttagtgtggtttgccagtgtggtagacctgctatacggtatgtttcagaacaaaagtcaccttggttattgatgtcatgtacgcctacgcaggtgcctttagacactagcggtatttggaaaaccgctattgtctttagggggccagttactgctggtcattatatgtatgccgtaaatggcactttgatatctgtgtatgatgctaatacgcgtaggcgtactagtgatcttaagctgccagctacagatattctttatggacctactagttttactagtgatagtaaggttgagacctactatcttgatggtgttaaacgtactactattgatcccgactttagtaagtatgttaagagaggtgactattattttacaacagcacctatagaggttgtggctgcgccaaagctagtcacatcttatgatggattttatctgtcttcctgtcagaatcctcagctagctgagtcttttaataaggctattaatgctactaagacaggacctatgaagttgctaaccatgtatcccaatgttgcgggtgatgtggtggcaatttctgatgataatgtcgttgctcatccatatgggtctttacatatgggtaaaccggtattgtttgttacgcgccctaatacttggaagaaattagtgccgttattatctacagttgttgttaatacgcctaatacttatgacgtattggctgtagatcctttacctgttaataatgagactagtgaggaaccaattagtgttaaggccccaataccattgtatggtttaaaggcaactatggttctcaatggtacaacatatgtgccaggtaataaaggtcatttgttgtgtttaaaggaattcactttaactgatttgcaaacgttttacgtcgagggtgtccaaccttttgtattacttaaggcttctcatttgagtaaagttcttggtttacgtgttagtgatagttcactgcatgttaaccatttaagtaaaggtgtagtctatgcctatgcggctactagactcactactcgtgttaccacttcacttttaggtggattggttactaggagtgttaggaagactgcagattttgtaaggagtacaaaccctggttcaaagtgtgtaggcctcttgtgtttattttatcagctctttatgcgattttggcttttagttaagaagccacctatcgttaaagtttccggtattatagcttataatacgggttgtggtgttacaacgtgtgttttaaattatttaagatcgcgttgcggcaatatatcatggtcgcgtttgctgaagttacttcggtatatgctgtatatttggtttgtttggacttgtttgactatatgtggcgtttggttatcggaaccttatgccccaagtttagtaactcgtttcaaatattttttaggtatcgttatgccgtgtgactatgtgctagttaatgaaacgggcactggttggttgcatcatttgtgcatggctggtatggatagtttggactatcctgctttgcgtatgcagcagcataggtatggtagtccctataactacacgtatatacttatgcttttagaagccttttttgcttatttgttatatacaccagctttgcctatagtaggtatcttggcagtactccacttgatagtgttgtacttgcctataccgcttggtaatagttggttagttgttttcttgtattatattataaggttggtaccctttactagtatgttgcgcatgtatattgttatagcttttttgtggttgtgctataagggctttttgcatgttaggtatggttgcaataatgtagcatgcttaatgtgttataagaagaatgtcgctaagcgcattgagtgttcgacagttgttaatggtgtgaaacgtatgttttatgtcaatgctaatggtggtacacacttttgcactaagcataattggaattgtgtttcgtgtgatacttatacagttgatagcacttttatttgtaggcaagttgccttggatttaagtgcacaatttaaaaggcccataattcatactgatgaagcttattatgaggttacttctgttgaggttcgcaatggttatgtttattgttactttgagagtgatggtcaacgtagctatgagcgatttccgatggatgcttttactaatgttagtaagttgcattattctgagttgaagggagctgcacctgcatttaatgttttagtgtttgatgcaactaaccgtatagaggaaaatgctgtaaaaacggctgctatatattatgcccagctagcttgtaagcctattttattggttgacaagcgtatggtaggtgttgtcggtgacgatgccaccatcgcaagggctatgtttgaggcatatgcgcaaaattatctccttaagtatagcattgcaatggataaagtaaaacacttgtatagcacggcgttgcaacagatatcttcgggtatgactgttgagtccgttcttaaggtgtttgtagggtccacacgtgctgaggctaaagatttagagtcagatgttgatactaatgatttagtctcgtgtattaggctctgtcatcaggagggttgggaatggaccacggattcgtggaataatcttgttcctacctatattaagcaggatactttgagcactttagaggttggtcaatttatgactgctaatgctaaatatgttaatgcaaatatagctaaaggcgctgccgtcaatttaatatggcggtatgcggattttattaagttgagcgagtccatgcgccgccaacttaaagtggctgcgcgtaagacaggtcttaacttattagttacaacatctagcttaaaggcagatgttccttgtatggtgacaccttttaaaattattggtggccatagacgtattgtatcgtggagacgtgttttaatacatgtcttcatgttattggttgttttaaacccgcagtggtttacaccttggtatataatgaggccaattgagtataatgtcgtggactttaaagttattgacaatgctgtaataagggatataacttctgcagatcagtgctttgctaacaaatttagtgcttttgaaaactggtattctaatagatatggtagttatgttaattcgcgtggttgtcctatggtggtaggtgttgttagtgacatcgtgggtagtcttgttcctggtttaccggcaagatttctacgtgtgggtaccacacttttaccattggtcaattacggtctgggtgcagtaggtagtgtgtgctacacaccgcactatgctattaactacgatgtttttgataccagtgcttgtgtattagctgctacctgtacgcttttttctagtgcgagtggtgaacgtatgccttactgtgctgatgccgcattaatacaaaatgcaagtcgttatgacatgttaaagccacacgtaatgtacccattttatgaacattctggttacatacgttttcctgaagttatttcagctggtgttcacatagttagaactatggctatggagtactgtaaagtgggtcgttgtgacgtttctgaagccggattgtgcatgtcgctacaacctcggtgggtcgtcaacaatgcttattttagacaacagtcaggtgtttactgtggtacaagtgcatttgatttatttatgaatatgctgctgcctatatttactcccgtaggtgctgttgatataacaacatctatactcatgggtgcattattggctgtagtagtttctatgtctctttattaccttttaaggtttagaagagcatttggtgattattcaggagtcatttttactaatattttggcttttgtgttgaatgttatagtactgtgtttagagggtccttaccctatgttacccagtatatatgctatggtgttcttatatgctacttgctactttggtagtgatatagcatgtatgatgcatgtttcatttttaataatgtttgctggtgtagtgcccttgtgggttactgttttgtacatagttgtggttttgagtaggcatatattgtggtttgctagtttatgcacaaagcgtacagtgcaggtaggtgaccttgcttttcactcctttcaggatgcagctttgcagacgtttatgcttgacaaagaggtgtttttacgccttaagcgtgaaatatcctcggatgcttattttaagtacttggctatgtataataagtacaagtattatagtggaccaatggatacagctgcttatagagaagccgcttgttcacatttggtgatggccttagagaaatattctaatggtggtggtgatactatatatcaacccccacggtgtagtgttgcctctgcggcactacaagccggcctgacacgtatggctcacccttcaggtttagtagagccgtgccttgttaaagtaaattatggttccatgactcttaatggtatatggttggataattttgttatatgtcctaggcatgttatgtgttctagggatgagttagctaatcctgattaccctcgtttgtctatgcgagctgctaattatgattttcacgtgtctcaaaatggtcataatattcgtgttataggccatactatggaaggttcgcttttaaagctaacagttgatgtgaataatcctaaaacacccgcttattcatttatacgggtgagtacgggtcaagctatgagtttgttggcatgttatgatggtttaccaactggtgtgtatacgtgcactttacggtcgaatggtactatgagagcatcatttttatgtggctcttgtggtagtcctggctttgtcatgaatggcaaagaagttcaattttgttacctacaccagcttgaattaccaaatggtactcatactggtacagatttttctggtgtcttttatggtccatttgaagacaagcaagtgcctcaattagcggcgcctgattgtactataactgttaatgttttagcatggctttatgcagctgtgttaagtggtgagaattggtttttaaccaagtctagtatttcaccggctgaatttaataattgtgctgttaagtacatgtgtcagtcagtaacgagtgaaagcttgcaagttttgcaaccacttgcagctaaaacaggtatctctgttgagcgcatgctttcagcgttgaaggtattgctctcagctggattttgtggccgtactattatgggctcctgttctttagaggatgagcatacaccgtatgatattggccgtcaaatgttaggtgttaaattgcaaggtaaatttcagtctatgtttagatggacactacagtggtttgctataatttttgtacttaccatactcattttgttgcagcttgcgcagtggacctttgtgggtgcgctgccatttactctgctgctgcccctaatagggtttgtggcagtttgtgtggggtttgtttcattgcttattaagcataagcatacctaccttacggtttatctgttaccagttgcgatggtaacagcatattataattttcagtacacgccagagggtgtacaaggttatttgcttagtttgtacaattacgttaatcctggtcgtattgacgttattggtacagatttgttaacaatgcttattataagtgttgcatgtactttgttaagtgttcgtatggtgagaactgatgcgtatagccgtatttggtacgtatgtactgcagtaggttggttgtataactgctggaccggtagtgctgatactgttgctatcagctaccttacatttatggtctcagtttttactaattacacgggcgttgcctgtgcttccttgtatgcagcacaatttatggtgtgggttcttaaatttttagaccctaccattttgttgttgtatggtaggtttagatgcgtgcttgtttgttatttgttagttggctatctttgcacatgttactttggtgtttttaaccttattaataggttatttagatgcaccttgggtaattatgaatatgtcgttagctctcaggagctgcgatatatgaattctcatggtttgttaccgcccacaaattcttggcaggcgcttatgttaaacattaagttggccggtatagggggtattcctatttatagggtgtccactatacagtcaaacatgacagatttaaaatgcacaagtgttgttttgctgtctgtattacaacaattacgtgttgaatccagtagtaaactatgggcactgtgcgttaagttgcacaatgaaatattagcctcaaattcgccaacagaggcatttgaggcatttgtttcattgttgtctgtgttgttatccttaccaggtgctataaacttggatgagttgtgtagtagcattttggaaaataattctgttctccaagctgttgctagtgagtttagtaatttatcatcctatgtggattacgaaaatgctcagaaggcctatgatacagctgttgccacaggtgcaccagcatctactgttaatgccttgaagaaagctatgaatgtagctaagagtgtgctcgataaagatgtagctactacccgtaagctggagcgtatgtctgagttagctatgactgcaatgtataagcaggctcgtgccgaagacaggcgctctaaagttacggccgctatgcaaactatgttgttcaacatgatacgtcgtcttgatagtgacgctcttagtaacattttgaacaatgcacgtaatggtgttgtaccactgggtgtcatacctagaacagcagctaacaagctgctgcttgtggtgcctgatttttctgtttacacagcaaccataactatgcctacgcttacctatgcgggtagtgcgtgggatgttatgcaagttgctgatgcagatggaaaaacagttaatgcaacggatattacacgcgagaatagtgtaaacttggcatggccgttagtagtgacggcgcagcggcagcaggccacatcacctgtcaagttacagaataatgagcttatgcctcagacagtgaagcgtatgaatgtcgttgcgggtgtgagccaaactgcttgtgttactgatgctgtagcttattataatgctacaaaagaaggccgacatgtgatggctattttagctgacacagacggtctcgcctttgctaaggttgaaaagtctacaggtgatggttttgtaattcttgaattagaaccaccctgtaagtttatggtcgacacccctaaaggtccggctcttaaatatttatattttaccaaagggcttaagaatttgtgccgtggcactgtattgggtactttggcttgtacagttagactgcatgcgggttctgctacggaagtagcaagtaactcatctattctttctttatgttcttttagtgtagaccctgaggctacgtataaagattatttagataatggtggttcccctataggtaactgcgttaaaatgctaactccccataccggtactgggttggctattacagctaagcctgatgccaatatagaccaagagtcctttggtggggcgtcatgctgtttgtactgtcgttgtcatatagaacatcccggtgcaagtggcgtatgtaaatataagggcaagtttgtacaaatacccttagttggtgtcaatgacccaataggtttttgtataagaaatgtcgtttgtgctgtatgtaacatgtggcaaggctatggttgtccctgctctagtttacgtgaaatcaacctacaggctagggatgagtgctttttaaacgagtcaggggtactagtggagtagcccgtctagtacccctaggttctggtgtccaaccagatatagtattaagggcttttgatatatgtaacacaaaagtagcaggttttggcttgcatttaaagaataattgttgtaggtatcaagaattggatgctgatggcactcaacttgattcctatttcgttgtaaaacgccatactgagagtaattatttacttgagcaacgctgttatgagaagcttaaggattgtggcgtcgttgcgcgtcatgatttctttaagttcaatatagaaggtgttatgacacctcatgtgtcacgtgaacgccttactaagtatacaatggcggatttagtatatagtttgcgccattttgataacaacaactgtgatacattaaaggaaatacttgtgttacgtggttgttgtactgcagattacttcgacaggaaggattggtatgaccctgtcgagaatccagatattattagggtttaccataacttaggtgaaactgttagaaaggccgtactctccgctgtgaagatggcagactctatggttgagcaaggactaattggtgttttaaccctggataatcaggacttaaatggccaatggtatgattttggtgacttcattgaagggccggcaggtgcgggtgttgccgtaatggatacttattattcattggctatgcccgtttatactatgacgaatatgctggccgctgaatgccacgttgatggagactttagtaaacctaaacgcgtgtgggacatatgtaagtatgattacacacagtttaagtattcattgttctccaagtattttaaatattgggacatgcaatatcacccaaattgtgttgcgtgtgccgatgaccgttgcattttgcattgtgctaattttaatatactttttagtatggtgttgcctaatacatcctttgggcctttagttcaaaagatttacgtggatggtgtgccgtttgtagtttctactggttaccattacagggagcttggtgtggtgatgaatcaagatattcgtcagcatgctcaacgtttgtcgttgcgtgaactacttgtgtatgcagcagatcctgctatgcatgtagcggctagtaacgcattggctgataaacgtactgtttgtatgtcggtggctgcaatgaccacgggcgttacttttcagactgtcaaaccaggacagtttaatgaagatttttataattttgctgtaaagtgtggcttcttcaaggaaggaagtaccatatcctttaagcattttttctatgcacaggatggcaatgctgccatctctgattatgattattataggtataatttgcctacaatgtgtgacattaaacaactccttttttctttagaagtagttgataaatattttgattgctatgacggcggatgcctacaggcaagtcaggttgttgtagctaattatgataagtcagcaggttttccattcaataagtttggtaaggcccgtctgtattatgaatctctcagttatgctgaccaggatgagctttttgcatacaccaaacgcaatgtcctacccacaattactcagatgaatttgaagtatgctataagtgctaaaaatcgcgctcgcactgtagctggtgtttctatagcatctactatgacaaatagacaatttcatcagaagatgcttaagtctatagctgcagcacgtggtgcatctgttgttataggtaccactaaattttatggagggtggaatcgcatgcttcgcactttgtgtgaaggtgtagaaaatccacatttgatgggttgggactatcctaaatgtgatagagctatgcctaatttattgcgtatatttgccagccttattttagcgcgtaagcatgcgacttgttgcaatgcttcagagaggttttatcggttggctaatgaatgtgctcaggttttgagtgaaatggttctctgtggaggcggtttttacgtgaaacctggtggtaccagtagtggagattccacaactgcatatgctaatagtgtttttaatatttgtcaagctgttagtgctaatcttaatacctttttatctatagatggtaataagatttacactacttatgttcaggaattgcagaggcggttatacttgggtatataccgtagtaatactgtagataatgagttagttttggattattataactatttgcgtaagcattttagtatgatgatccttagtgatgatggtgtggtctgctataatgcggactacgcacaaaaaggctatgttgctgacatacagggctttaaggagttgctgtattttcagaacaatgtgtttatgtctgaatctaagtgttgggtagaaccggatataactaaaggtcctcatgaattttgctctcaacatactatgttggttgatatgaagggtgaacaagtttacctgccatatccagatccttctagaatattgggagcagggtgctttgtggatgacttattgaagactgatggtactcttatgatggagcggtatgtgtcacttgctattgatgcctatccacttacgaagcatcccgatcctgagtaccagaatgttttctggtgttatctgcaatatataaagaagttgcatgaggagttaacaggtcatttattagatacatatagtgtaatgttggctagtgataacgcttctaagtactgggaggtagaattctatgagaatatgtatatggaatctgccacattacagagtgtaggtacatgtgttgtgtgtaattcacaaacatcattaagatgtggtggctgcatacgtagacccttcctctgttgtaaatgttgttatgaccatgtcgtgtctactacacacaagttagtgttgtctgttacaccatatgtttgtaacaaccctagttgtgatgttgcagatgtaacccaattgtatttgggtggcatgtcttattattgtagagaccatagaccaccaatatcgttccctttgtgtgcgaatggtcaggtgtttggtctctacaaaaatatatgtactggtagtccggatgtagcggacttcaatagtctagctacttgtgattggagtaacagtaaagattatgtcttagctaatacggctacagagcgtttaaagctctttgccgctgagacattacgtgcgactgaagaaaatgctaaacaagcatatgcttcagcagttgttaaagaggtccttagtgatagggaacttgtgctttcatgggaaactggcaagacccgacctcccttaaataggaattatgtattcacggggtttcatattactaagaatagtaaggtgcaactgggtgaatacatttttgaaaagggtgactacggtgacgtagttaactatcgttctagtaccacttataaattacaggttggtgattactttgtgcttacatcacattcggtgcaaccacttagttcacctactttgttacctcaggagcgatacactaagttagtcggtttgtatccagctatgaatgtgccagagagctttgctagtaacgttgtacattaccaacgtgttggtatgtcgcgttacactactgtacagggtccacctggtacgggtaagagccacttgtccataggacttgcgctctactacccgtctgctaaaatcgtttacacagcatgcagtcatgcagctgtagatgcattgtgtgagaaggcgcataagaatttacctattaataggtgtagtcgtattgtgccagctaaggcacgtgttgagtgtttctcaaagttcaaagttaacgatgtgggtgctcaatacgttttctctactataaatgccctaccagaaacaactgcggacattcttgttgtagatgaggtcagtatgtgtactaactatgacctgagtatgattaatgcaagggttcgcgcaaaacatattgtgtatgtaggtgaccctgcacaattaccggcgcctagaactcttcttacgaagggtacgcttgcacctgaacattttaattcagtgtgcaggcttatggttgccgtaggtcctgacattttccttgccacctgctatagatgtcctaaggaaatagttgatacagttagcgctttagtttatgataaaaagctaaaggctaataaggttaccactggggagtgttataagtgctactataaaggtagtgtcactcatgactcgtctagcgctattaataagcctcagcttggcttagttaaagagttcttaattaagaatcctaagtggcagagtgcagtgtttatttcaccctataatagtcaaaactctgtagcacgtcgtatgctaggtttgcagacacagactgttgactcctctcagggttctgagttcgactatgttatttattgtcaaacttccgacacagcccatgcattgaatgtaaataggtttaatgtagctatcactagagctaaaaagggcattctgtgtgtgatgtcagactctacgttatatgagtctctcgagtttacaccactggatgtgaatgattatgtaaaaccaaaaatgcagtctgaagttactgtaggtttgtttaaagattgtgctaaagcagagccattaggcccagcctatgcacctacttttgtgtccgtaaatgacaagttcaaattgaatgagtcactttgtgtacattttgacacaacggaattacagatgccttataatagactcatttctaaaatgggttttaagtttgatttaaacatacccggttatagcaagttatttataactcgtgaacaggctattagagaagtacgtggctgggtagggtttgatgttgagggtgcacatgcttgtggtcccaacattggcactaacctgccactacaaatagggttttctactggcgtaaactttgtagttacgcctagtggttatatagatacagaatctggttctagattggctaatgtggtgtctaaggcaccacctggtgaccaatttaaacatttgataccactaatgcgtaagggcgagccttggagcgtcgttcgtaagcgtatagtggagatgctttgtgatactctagatggtgtcagtgacaccgttacatttgtaacttgggcacatgggtttgaactcacgacccttcattacttcgctaaagtaggacctgaacgcaaatgttttatgtgtcctaggcgtgcaaccttatttagtagtgtttatggggcatattcatgctggagtcaccatagacacattggcggcgcggactttgtatataacccatttttggtcgatgtacagcaatggggttatgtaggtaatttacaggtaaaccatgataatgtctgcgatgtccataagggtgcacatgtggctagctgtgatgccataatgactaggtgtttagctatccatgactgtttctgtggtgaagtcaattgggatgtagagtatcctattatagctaatgagttggctataaatagggcgtgtcgtagtgttcagcgagtcgtattaaaggctgctgtgaaggcactacatatagaaacaatttatgatattggtaacccaaaggctattaaagtctatggtgtcaatgtcaataattggaatttttatgacactaatcctgttgtggaaggtgttaagcagttacattatgtttatgatgtacatagagaccagttcaaagatggactagctatgttttggaattgcaatgtggattgttatccacataatgcgttggtttgtaggtttgacacacgtgtgttgtcaaaattaaatttagcagggtgcaatggtggttcgctttatgtgaatcagcatgcgttccatactgatgcatttaataaaaatgcttttgttaatttgaagccactcccattcttttattattcagatacggcatgtgaaaatgctactggtgtgtctactaattatgtcagtgaagtagattatgtacccctcaaatcaaatgtgtgtataacgcgttgtaatttgggtggtgcagtttgtaagaaacatgctgacgagtacagaaattttctggaaagttataatactatggtgagcgcaggtttcaccttgtgggttgataaaacctttgacgtgtttaatttatggtctacatttgtaaagctacaatctctagagaatgtagcttacaatgtcttaaagtcaggccattttacagcagttgccggtgagttaccggtagctattttaaatgaccgactctatataaaggaggacggtgctgataaattgttgtttactaataatacatgtttgcccactaatgtagcttttgagctatgggctaaacgttcagtgaacgtagtaccagaagttaagttattacgtaacttaggtgttacgtgtacatataacttagttatctgggattatgaaagtaatgctccactagtgccaaatactgtgggcatttgtacttatactgatttaacaaagttagatgaccaggttgtgctagttgatggcagacagctagatgcctatagtaagttttgtcagttgaaaaatgccatttacttttcacctagtaaacctaagtgcgtgtgtaccagaggaccaactcacgcatctataaatggtgttgttgtagaggcccctgatagaggtactgcattttggtatgctatgagaaaagatggtgcatttgtgcaacctactgatggctattttacacagtcccgtactgtggacgattttcagccacgtacacaattagaaatagatttccttgatcttgagcagtcatgttttcttgataaatatgacttacatgatctaggtttagaacatatcgtgtatggtcaatttgatggaaccataggcggcttgcatttattaataggtgccgtacgccgtaagcgcacggcgcatttagttatggagaccgtgctaggtactgacacggtcacatcttatgctgttatagaccaaccaactgcttctagtaagcaagtttgtagtgttgttgatattattttagatgactttattgcgcttataaaagctcaagataggtcagttgttagtaaggtagttcagtgctgcttggattttaaagtgtttaggtttatgttatggtgtaagggtggtaagatttccaccttttatcctcaattgcaggctaaacaagattggaaacctggttatagtatgccagcgctttataaggtgcaaaatgccgtgctagaaccatgtttgttacacaattacggtcaggcggcaagattgccgtccggtaccttaatgaatgtggctaaatacactcagttgtgtcagtacctgaatacctgttcattagctgttccggctaaaatgcgtgttatgcattttggtgcaggcagtgataaaggtgtttgtccaggtactgctgtgttaaaacaatggttgccagctgacgcttacttggtagataatgatttgtgttattgtgcatctgatgcagatagtacgtatgtaggtagttgtgagacattcttttctgttaataagtgggattttatttttagtgacatgtatgatgcacgcactaagaatacttctggtgataatacgtctaaagaaggattttttacgtatttaacaggttttataaggtcaaaactagctcttggaggtagtattgccattaagattacagagcactcttggagtgctgatctgtatgctattatgggccactttaattggtggacttgtttttgtacatctgttaatagctcttcgtccgaagcgtttttgataggtgtaaattatattggtgtaggtgcattattagatgggtggcaaatgcatgctaattacgtcttttggcgtaatagcactgttatgcaattgtctagttatagtctgtatgatttgcagcgtttcccattgcgcttgaaaggcactcctgttatgagtttgaaggaagatcaattgaacgaacttgttttaaacttgattagagcaggtcgcctaatagtccgcgatgctgttgatattggtgttaggggtgtcgcttgcagcggcgtctagaccatgaactccttctccacaagcgccttcggtccagttgccttctccctgggcctgctcctggtgttgcctgctgccttccctgccccagtcttcacactcgaagatttcgttggggactggcgacagacagccggctacaacctggaccaagtccttgaacagggaggtgtgtccagtttgtttcagaatctcggggtgtccgtaactccgatccaaaggattgtcctgagcggtgaaaatgggctgaagatcgacatccatgtcatcatcccgtatgaaggtctgagcggcgaccaaatgggccagatcgaaaaaatttttaaggtggtgtaccctgtggatgatcatcactttaaggtgatcctgcactatggcacactggtaatcgacggggttacgccgaacatgatcgactatttcggacggccgtatgaaggcatcgccgtgttcgacggcaaaaagatcactgtaacagggaccctgtggaacggcaacaaaattatcgacgagcgcctgatcaaccccgacggctccctgctgttccgagtaaccatcaacggagtgaccggctggcggctgtgcgaacgcattctggcgtaactcttgaacgaacgcgaagaattactttgtgacaatgattgaacaagatggattgcacgcaggttctccggccgcttgggtggagaggctattcggctatgactgggcacaacagacaatcggctgctctgatgccgccgtgttccggctgtcagcgcaggggcgcccggttctttttgtcaagaccgacctgtccggtgccctgaatgaactgcaagacgaggcagcgcggctatcgtggctggccacgacgggcgttccttgcgcagctgtgctcgacgttgtcactgaagcgggaagggactggctgctattgggcgaagtgccggggcaggatctcctgtcatctcaccttgctcctgccgagaaagtatccatcatggctgatgcaatgcggcggctgcatacgcttgatccggctacctgcccattcgaccaccaagcgaaacatcgcatcgagcgagcacgtactcggatggaagccggtcttgtcgatcaggatgatctggacgaagagcatcaggggctcgcgccagccgaactgttcgccaggctcaaggcgagcatgcccgacggcgaggatctcgtcgtgacccatggcgatgcctgcttgccgaatatcatggtggaaaatggccgcttttctggattcatcgactgtggccggctgggtgtggcggaccgctatcaggacatagcgttggctacccgtgatattgctgaagagcttggcggcgaatgggctgaccgcttcctcgtgctttacggtatcgccgctcccgattcgcagcgcatcgccttctatcgccttcttgacgagttcttctgaagttatatatattgttacatgttgtatatatttccttctttataatttgaacgaacctattatgtctggaaggaacagatctagatctggtacaccttcccctaaggtcacgttcaaacaagaatctgacggttctgactccgaatctgagcgccgtaatggtaaccgtaatggtgcccgccctaaaaataataatagtagaggtagtgctcccaagcctgagaagcctaaggcggcccctcctcagaatgtttcctggtttgcaccgttggttcaaaccggtaaagctgagttgcgtttccctagaggtgaaggagtgcccgtgagccaaggtgttgattccacttacgagcacgggtactggctgcgtacacagaggtctttccagaaaggtggtaagcaagttttggctaacccccgctggtacttctattatactggcactggtcgctttggtgaccttcgttttgggactaagaacccggacatagtctgggttggccaagaaggtgctaatatcaaccgtctcggtgatatgggcacacgtaaccccagtaatgatggtgctataccagtgcaattagctggtggcatacctaagggcttctatgctgaggggcgtggctcccgtggtaatagccgcagtagttcacgcaactcaagcagagcatcatcgcgtggtaactcacgtgctagctcccgtggtgcatcacccggtagacctgctgctaacccgtccactgagccgtggatggcttatcttgtacagaagttggaaagactggagagtcaggttagtggtactaagccagctaccaagaacccagttcaagttactaagaatgaggctgccgccaatgctaagaagctcaggcataaacgcactgcgcataagggcagtggtgttactgtgaattacggcagacgtggcccaggtgatctggagggtaattttggggatcgtgaaatgatcaaacttggtactgatgatcccaggtttgctgccgctgcgcaaatggcccctaatgtttcatcttttctgtttatgtctcatttatccacgagggatgaagatgatgctctgtggctccattataaaggtgccataaagcttcctaaagatgatcccaactatgagcagtggactaagattttggcagaaaacttgaacgcctacaaagatttccctcctactgagcccaaaaaggataaaaagaagaaggaagagaccgcccaagacactgtcatctttgaagatgcgtctactggaacagaccaaacagttgttaaggtctgggtaaaagatcaggacgcacaaactgatgatgagtggctgggtggtgatgaaaccgtttatgaagatgaggacgaccgtccaaagacccagaggagacacaagaagagaggatcaactgcctctcgtgtgactattgcggaccctactaatgcaggtgccgaaagatcttagtcgctgtggcctactcttatacagaatggaatcctagtgtacagtggtataagtaagctgtgcattcgctatgtttaggtttagaatgtagtttagtgctagctgattagagtgtgttaaagacttgtagagcgccttagggaagagctaatcagtaatacattatacaaaattttaagcaacccctaatcatagtatgctttatagaggatttgcaaaaaaaaaaaaaaaaaaaaaaaaaaaaaaaaggccggcatggtcccagcctcctcgctggcgccggctgggcaacattccgaggggaccgtcccctcggtaatggcgaatgggacccactgtgccttctagttgccagccatctgttgtttgcccctcccccgtgccttccttgaccctggaaggtgccactcccactgtcctttcctaataaaatgaggaaattgcatcgcattgtctgagtaggtgtcattctattctggggggtggggtggggcaggacagcaagggggaggattgggaagacaatagcaggcatgctggggatgcggtgggctctatgg

SEQ ID NO: 2 - protein, 6930 aa, Nobecovirus
MEGVPDPPKLKSMVVTTLKWCDPFANPNVTGWDIPIEEALEYAKQQLRTPEPQLVFVPYYLSHAPGISGDRVVITDSIWYATNFGWQPIRELAMDKDGVRYGRGGTHGVLLPMQDPSFIMGDIDIQIRKYGIGANSPPDVLPLWDGFSDPGPDVGPYLDFPDNCCPTKPKAKRGGDVYLSDQYGFDNNGILVEPVMKLLGVIKSDFTLEQLLAALGKYRTEDGYDLPDGYVKVAIKVGRKAVPVLKQSIFTVVGVTEQLVPGYYYPFSTSSVVEHTKPTRGGPVGKTVEAVMLSLYGTNNYNPATPVARLKCSYCDYYGWTPLKDIGTVNCLCGAEFQLTSSCVDAESAGVIKPGCVMLLDKSPGMRLIPGNRTYVSFGGAIWSPIGKVNGVTVWVPRAYSIVAGEHSGAVGSGDTVAINKELVEYLIEGIRVDADTLDNPTCATFIANLDCDTKAPVVHTVESLQGLCLANKIMLGDKPLPTDEFHPFIVGLAYHVQRACWYGALASRTFEAFRDFVRTEEERFAQFFGKVCAPINGCVYLAYTTGRVTLFSAYQVLNTAIAKSKDAFGGVAAIVVDMLKPILEWVLKKMSIAKGAWLPYAEGLLALFKAQFTVVKGKFQFLRASLNSKCHSLCDLLTTIMSKLLTSVKWAGCKVDALYTGTYYYFSRKGVLTEVQLCAKRLGLLLTPKQQKMEVEVLDGDFDAPVTLTDLELEECTGVLEEVFGASDVKLVKGTLVSLASKLFVRTEDGFLYRYVKSGGVLGKAFRLRGGGVSKVTFGDEEVHTIPNTVTVNFSYDVCEGLDAILDKVMAPFQVEEGTKLEDLACVVQKAVYERLSDLFSDCPAELRPINLEDFLTSECFVYSKDYEKILMPEMYFSLEDAVPVDDEMVDDIEDTVEQASDSDDQWLGDEGAEDCDNTIQDVDVATSMTTPCGYTKIAEHVYIKCADIVQEARNYSYAVLVNAANVNLHHGGGVAGALNRATNNAMQKESSEYIKANGSLQPGGHVLLSSHGLASHGILHVVGPDKRLGQDLALLDAVYAAYTGFDSVLTPLVSAGIFGFTVEESLCSLVKNVACTTYVVVYDRQLYERALATSFDVPGPQSSVQHVPAIDWAEAVEVQESIVDQVETPSLGAVDTVDSNADSGLNETARSPENVVGSVPDDVVADVESCVRDLVRQVVKKVKRDKRPPPIVPQQTVEQQPQEISSPGDCNTVLVDVVSMSFSAMVNFGKEKGLLIPVVIDYPAFLKVLKRFSPKEGLFSSNGYEFYGYSRDKPLHEVSKDLNSLGRPLIMIPFGFIVNGQTLAVSAVSMRGLTVPHTVVVPSESSVPLYRAYFNGVFSGDTTAVQDFVVDILLNGARDWDVLQTTCTVDRKVYKTICKRGNTYLCFDDTNLYAITGDVVLKFATVSKARAYLETKLCAPEPLIKVLTTVDGINYSTVLVSTAQSYRAQIGTVFCDGHDWSNKNPMPTDEGTHLYKQDNFSSAEVTAIREYYGVDDSNIIARAMSIRKTVQTWPYTVVDGRVLLAQRDSNCYLNVAISLLQDIDVSFSTPWVCRAYDALKGGNPLPMAEVLIALGKATPGVSDDAHMVLSAVLNHGTVTARRVMQTVCEHCGVSQMVFTGTDACTFYGSVVLDDLYAPVSVVCQCGRPAIRYVSEQKSPWLLMSCTPTQVPLDTSGIWKTAIVFRGPVTAGHYMYAVNGTLISVYDANTRRRTSDLKLPATDILYGPTSFTSDSKVETYYLDGVKRTTIDPDFSKYVKRGDYYFTTAPIEVVAAPKLVTSYDGFYLSSCQNPQLAESFNKAINATKTGPMKLLTMYPNVAGDVVAISDDNVVAHPYGSLHMGKPVLFVTRPNTWKKLVPLLSTVVVNTPNTYDVLAVDPLPVNNETSEEPISVKAPIPLYGLKATMVLNGTTYVPGNKGHLLCLKEFTLTDLQTFYVEGVQPFVLLKASHLSKVLGLRVSDSSLHVNHLSKGVVYAYAATRLTTRVTTSLLGGLVTRSVRKTADFVRSTNPGSKCVGLLCLFYQLFMRFWLLVKKPPIVKVSGIIAYNTGCGVTTCVLNYLRSRCGNISWSRLLKLLRYMLYIWFVWTCLTICGVWLSEPYAPSLVTRFKYFLGIVMPCDYVLVNETGTGWLHHLCMAGMDSLDYPALRMQQHRYGSPYNYTYILMLLEAFFAYLLYTPALPIVGILAVLHLIVLYLPIPLGNSWLVVFLYYIIRLVPFTSMLRMYIVIAFLWLCYKGFLHVRYGCNNVACLMCYKKNVAKRIECSTVVNGVKRMFYVNANGGTHFCTKHNWNCVSCDTYTVDSTFICRQVALDLSAQFKRPIIHTDEAYYEVTSVEVRNGYVYCYFESDGQRSYERFPMDAFTNVSKLHYSELKGAAPAFNVLVFDATNRIEENAVKTAAIYYAQLACKPILLVDKRMVGVVGDDATIARAMFEAYAQNYLLKYSIAMDKVKHLYSTALQQISSGMTVESVLKVFVGSTRAEAKDLESDVDTNDLVSCIRLCHQEGWEWTTDSWNNLVPTYIKQDTLSTLEVGQFMTANAKYVNANIAKGAAVNLIWRYADFIKLSESMRRQLKVAARKTGLNLLVTTSSLKADVPCMVTPFKIIGGHRRIVSWRRVLIHVFMLLVVLNPQWFTPWYIMRPIEYNVVDFKVIDNAVIRDITSADQCFANKFSAFENWYSNRYGSYVNSRGCPMVVGVVSDIVGSLVPGLPARFLRVGTTLLPLVNYGLGAVGSVCYTPHYAINYDVFDTSACVLAATCTLFSSASGERMPYCADAALIQNASRYDMLKPHVMYPFYEHSGYIRFPEVISAGVHIVRTMAMEYCKVGRCDVSEAGLCMSLQPRWVVNNAYFRQQSGVYCGTSAFDLFMNMLLPIFTPVGAVDITTSILMGALLAVVVSMSLYYLLRFRRAFGDYSGVIFTNILAFVLNVIVLCLEGPYPMLPSIYAMVFLYATCYFGSDIACMMHVSFLIMFAGVVPLWVTVLYIVVVLSRHILWFASLCTKRTVQVGDLAFHSFQDAALQTFMLDKEVFLRLKREISSDAYFKYLAMYNKYKYYSGPMDTAAYREAACSHLVMALEKYSNGGGDTIYQPPRCSVASAALQAGLTRMAHPSGLVEPCLVKVNYGSMTLNGIWLDNFVICPRHVMCSRDELANPDYPRLSMRAANYDFHVSQNGHNIRVIGHTMEGSLLKLTVDVNNPKTPAYSFIRVSTGQAMSLLACYDGLPTGVYTCTLRSNGTMRASFLCGSCGSPGFVMNGKEVQFCYLHQLELPNGTHTGTDFSGVFYGPFEDKQVPQLAAPDCTITVNVLAWLYAAVLSGENWFLTKSSISPAEFNNCAVKYMCQSVTSESLQVLQPLAAKTGISVERMLSALKVLLSAGFCGRTIMGSCSLEDEHTPYDIGRQMLGVKLQGKFQSMFRWTLQWFAIIFVLTILILLQLAQWTFVGALPFTLLLPLIGFVAVCVGFVSLLIKHKHTYLTVYLLPVAMVTAYYNFQYTPEGVQGYLLSLYNYVNPGRIDVIGTDLLTMLIISVACTLLSVRMVRTDAYSRIWYVCTAVGWLYNCWTGSADTVAISYLTFMVSVFTNYTGVACASLYAAQFMVWVLKFLDPTILLLYGRFRCVLVCYLLVGYLCTCYFGVFNLINRLFRCTLGNYEYVVSSQELRYMNSHGLLPPTNSWQALMLNIKLAGIGGIPIYRVSTIQSNMTDLKCTSVVLLSVLQQLRVESSSKLWALCVKLHNEILASNSPTEAFEAFVSLLSVLLSLPGAINLDELCSSILENNSVLQAVASEFSNLSSYVDYENAQKAYDTAVATGAPASTVNALKKAMNVAKSVLDKDVATTRKLERMSELAMTAMYKQARAEDRRSKVTAAMQTMLFNMIRRLDSDALSNILNNARNGVVPLGVIPRTAANKLLLVVPDFSVYTATITMPTLTYAGSAWDVMQVADADGKTVNATDITRENSVNLAWPLVVTAQRQQATSPVKLQNNELMPQTVKRMNVVAGVSQTACVTDAVAYYNATKEGRHVMAILADTDGLAFAKVEKSTGDGFVILELEPPCKFMVDTPKGPALKYLYFTKGLKNLCRGTVLGTLACTVRLHAGSATEVASNSSILSLCSFSVDPEATYKDYLDNGGSPIGNCVKMLTPHTGTGLAITAKPDANIDQESFGGASCCLYCRCHIEHPGASGVCKYKGKFVQIPLVGVNDPIGFCIRNVVCAVCNMWQGYGCPCSSLREINLQARDECFLNRVRGTSGVARLVPLGSGVQPDIVLRAFDICNTKVAGFGLHLKNNCCRYQELDADGTQLDSYFVVKRHTESNYLLEQRCYEKLKDCGVVARHDFFKFNIEGVMTPHVSRERLTKYTMADLVYSLRHFDNNNCDTLKEILVLRGCCTADYFDRKDWYDPVENPDIIRVYHNLGETVRKAVLSAVKMADSMVEQGLIGVLTLDNQDLNGQWYDFGDFIEGPAGAGVAVMDTYYSLAMPVYTMTNMLAAECHVDGDFSKPKRVWDICKYDYTQFKYSLFSKYFKYWDMQYHPNCVACADDRCILHCANFNILFSMVLPNTSFGPLVQKIYVDGVPFVVSTGYHYRELGVVMNQDIRQHAQRLSLRELLVYAADPAMHVAASNALADKRTVCMSVAAMTTGVTFQTVKPGQFNEDFYNFAVKCGFFKEGSTISFKHFFYAQDGNAAISDYDYYRYNLPTMCDIKQLLFSLEVVDKYFDCYDGGCLQASQVVVANYDKSAGFPFNKFGKARLYYESLSYADQDELFAYTKRNVLPTITQMNLKYAISAKNRARTVAGVSIASTMTNRQFHQKMLKSIAAARGASVVIGTTKFYGGWNRMLRTLCEGVENPHLMGWDYPKCDRAMPNLLRIFASLILARKHATCCNASERFYRLANECAQVLSEMVLCGGGFYVKPGGTSSGDSTTAYANSVFNICQAVSANLNTFLSIDGNKIYTTYVQELQRRLYLGIYRSNTVDNELVLDYYNYLRKHFSMMILSDDGVVCYNADYAQKGYVADIQGFKELLYFQNNVFMSESKCWVEPDITKGPHEFCSQHTMLVDMKGEQVYLPYPDPSRILGAGCFVDDLLKTDGTLMMERYVSLAIDAYPLTKHPDPEYQNVFWCYLQYIKKLHEELTGHLLDTYSVMLASDNASKYWEVEFYENMYMESATLQSVGTCVVCNSQTSLRCGGCIRRPFLCCKCCYDHVVSTTHKLVLSVTPYVCNNPSCDVADVTQLYLGGMSYYCRDHRPPISFPLCANGQVFGLYKNICTGSPDVADFNSLATCDWSNSKDYVLANTATERLKLFAAETLRATEENAKQAYASAVVKEVLSDRELVLSWETGKTRPPLNRNYVFTGFHITKNSKVQLGEYIFEKGDYGDVVNYRSSTTYKLQVGDYFVLTSHSVQPLSSPTLLPQERYTKLVGLYPAMNVPESFASNVVHYQRVGMSRYTTVQGPPGTGKSHLSIGLALYYPSAKIVYTACSHAAVDALCEKAHKNLPINRCSRIVPAKARVECFSKFKVNDVGAQYVFSTINALPETTADILVVDEVSMCTNYDLSMINARVRAKHIVYVGDPAQLPAPRTLLTKGTLAPEHFNSVCRLMVAVGPDIFLATCYRCPKEIVDTVSALVYDKKLKANKVTTGECYKCYYKGSVTHDSSSAINKPQLGLVKEFLIKNPKWQSAVFISPYNSQNSVARRMLGLQTQTVDSSQGSEFDYVIYCQTSDTAHALNVNRFNVAITRAKKGILCVMSDSTLYESLEFTPLDVNDYVKPKMQSEVTVGLFKDCAKAEPLGPAYAPTFVSVNDKFKLNESLCVHFDTTELQMPYNRLISKMGFKFDLNIPGYSKLFITREQAIREVRGWVGFDVEGAHACGPNIGTNLPLQIGFSTGVNFVVTPSGYIDTESGSRLANVVSKAPPGDQFKHLIPLMRKGEPWSVVRKRIVEMLCDTLDGVSDTVTFVTWAHGFELTTLHYFAKVGPERKCFMCPRRATLFSSVYGAYSCWSHHRHIGGADFVYNPFLVDVQQWGYVGNLQVNHDNVCDVHKGAHVASCDAIMTRCLAIHDCFCGEVNWDVEYPIIANELAINRACRSVQRVVLKAAVKALHIETIYDIGNPKAIKVYGVNVNNWNFYDTNPVVEGVKQLHYVYDVHRDQFKDGLAMFWNCNVDCYPHNALVCRFDTRVLSKLNLAGCNGGSLYVNQHAFHTDAFNKNAFVNLKPLPFFYYSDTACENATGVSTNYVSEVDYVPLKSNVCITRCNLGGAVCKKHADEYRNFLESYNTMVSAGFTLWVDKTFDVFNLWSTFVKLQSLENVAYNVLKSGHFTAVAGELPVAILNDRLYIKEDGADKLLFTNNTCLPTNVAFELWAKRSVNVVPEVKLLRNLGVTCTYNLVIWDYESNAPLVPNTVGICTYTDLTKLDDQVVLVDGRQLDAYSKFCQLKNAIYFSPSKPKCVCTRGPTHASINGVVVEAPDRGTAFWYAMRKDGAFVQPTDGYFTQSRTVDDFQPRTQLEIDFLDLEQSCFLDKYDLHDLGLEHIVYGQFDGTIGGLHLLIGAVRRKRTAHLVMETVLGTDTVTSYAVIDQPTASSKQVCSVVDIILDDFIALIKAQDRSVVSKVVQCCLDFKVFRFMLWCKGGKISTFYPQLQAKQDWKPGYSMPALYKVQNAVLEPCLLHNYGQAARLPSGTLMNVAKYTQLCQYLNTCSLAVPAKMRVMHFGAGSDKGVCPGTAVLKQWLPADAYLVDNDLCYCASDADSTYVGSCETFFSVNKWDFIFSDMYDARTKNTSGDNTSKEGFFTYLTGFIRSKLALGGSIAIKITEHSWSADLYAIMGHFNWWTCFCTSVNSSSSEAFLIGVNYIGVGALLDGWQMHANYVFWRNSTVMQLSSYSLYDLQRFPLRLKGTPVMSLKEDQLNELVLNLIRAGRLIVRDAVDIGVRGVACSGV

SEQ ID NO: 3 - protein, 4248 aa, Nobecovirus
MEGVPDPPKLKSMVVTTLKWCDPFANPNVTGWDIPIEEALEYAKQQLRTPEPQLVFVPYYLSHAPGISGDRVVITDSIWYATNFGWQPIRELAMDKDGVRYGRGGTHGVLLPMQDPSFIMGDIDIQIRKYGIGANSPPDVLPLWDGFSDPGPDVGPYLDFPDNCCPTKPKAKRGGDVYLSDQYGFDNNGILVEPVMKLLGVIKSDFTLEQLLAALGKYRTEDGYDLPDGYVKVAIKVGRKAVPVLKQSIFTVVGVTEQLVPGYYYPFSTSSVVEHTKPTRGGPVGKTVEAVMLSLYGTNNYNPATPVARLKCSYCDYYGWTPLKDIGTVNCLCGAEFQLTSSCVDAESAGVIKPGCVMLLDKSPGMRLIPGNRTYVSFGGAIWSPIGKVNGVTVWVPRAYSIVAGEHSGAVGSGDTVAINKELVEYLIEGIRVDADTLDNPTCATFIANLDCDTKAPVVHTVESLQGLCLANKIMLGDKPLPTDEFHPFIVGLAYHVQRACWYGALASRTFEAFRDFVRTEEERFAQFFGKVCAPINGCVYLAYTTGRVTLFSAYQVLNTAIAKSKDAFGGVAAIVVDMLKPILEWVLKKMSIAKGAWLPYAEGLLALFKAQFTVVKGKFQFLRASLNSKCHSLCDLLTTIMSKLLTSVKWAGCKVDALYTGTYYYFSRKGVLTEVQLCAKRLGLLLTPKQQKMEVEVLDGDFDAPVTLTDLELEECTGVLEEVFGASDVKLVKGTLVSLASKLFVRTEDGFLYRYVKSGGVLGKAFRLRGGGVSKVTFGDEEVHTIPNTVTVNFSYDVCEGLDAILDKVMAPFQVEEGTKLEDLACVVQKAVYERLSDLFSDCPAELRPINLEDFLTSECFVYSKDYEKILMPEMYFSLEDAVPVDDEMVDDIEDTVEQASDSDDQWLGDEGAEDCDNTIQDVDVATSMTTPCGYTKIAEHVYIKCADIVQEARNYSYAVLVNAANVNLHHGGGVAGALNRATNNAMQKESSEYIKANGSLQPGGHVLLSSHGLASHGILHVVGPDKRLGQDLALLDAVYAAYTGFDSVLTPLVSAGIFGFTVEESLCSLVKNVACTTYVVVYDRQLYERALATSFDVPGPQSSVQHVPAIDWAEAVEVQESIVDQVETPSLGAVDTVDSNADSGLNETARSPENVVGSVPDDVVADVESCVRDLVRQVVKKVKRDKRPPPIVPQQTVEQQPQEISSPGDCNTVLVDVVSMSFSAMVNFGKEKGLLIPVVIDYPAFLKVLKRFSPKEGLFSSNGYEFYGYSRDKPLHEVSKDLNSLGRPLIMIPFGFIVNGQTLAVSAVSMRGLTVPHTVVVPSESSVPLYRAYFNGVFSGDTTAVQDFVVDILLNGARDWDVLQTTCTVDRKVYKTICKRGNTYLCFDDTNLYAITGDVVLKFATVSKARAYLETKLCAPEPLIKVLTTVDGINYSTVLVSTAQSYRAQIGTVFCDGHDWSNKNPMPTDEGTHLYKQDNFSSAEVTAIREYYGVDDSNIIARAMSIRKTVQTWPYTVVDGRVLLAQRDSNCYLNVAISLLQDIDVSFSTPWVCRAYDALKGGNPLPMAEVLIALGKATPGVSDDAHMVLSAVLNHGTVTARRVMQTVCEHCGVSQMVFTGTDACTFYGSVVLDDLYAPVSVVCQCGRPAIRYVSEQKSPWLLMSCTPTQVPLDTSGIWKTAIVFRGPVTAGHYMYAVNGTLISVYDANTRRRTSDLKLPATDILYGPTSFTSDSKVETYYLDGVKRTTIDPDFSKYVKRGDYYFTTAPIEVVAAPKLVTSYDGFYLSSCQNPQLAESFNKAINATKTGPMKLLTMYPNVAGDVVAISDDNVVAHPYGSLHMGKPVLFVTRPNTWKKLVPLLSTVVVNTPNTYDVLAVDPLPVNNETSEEPISVKAPIPLYGLKATMVLNGTTYVPGNKGHLLCLKEFTLTDLQTFYVEGVQPFVLLKASHLSKVLGLRVSDSSLHVNHLSKGVVYAYAATRLTTRVTTSLLGGLVTRSVRKTADFVRSTNPGSKCVGLLCLFYQLFMRFWLLVKKPPIVKVSGIIAYNTGCGVTTCVLNYLRSRCGNISWSRLLKLLRYMLYIWFVWTCLTICGVWLSEPYAPSLVTRFKYFLGIVMPCDYVLVNETGTGWLHHLCMAGMDSLDYPALRMQQHRYGSPYNYTYILMLLEAFFAYLLYTPALPIVGILAVLHLIVLYLPIPLGNSWLVVFLYYIIRLVPFTSMLRMYIVIAFLWLCYKGFLHVRYGCNNVACLMCYKKNVAKRIECSTVVNGVKRMFYVNANGGTHFCTKHNWNCVSCDTYTVDSTFICRQVALDLSAQFKRPIIHTDEAYYEVTSVEVRNGYVYCYFESDGQRSYERFPMDAFTNVSKLHYSELKGAAPAFNVLVFDATNRIEENAVKTAAIYYAQLACKPILLVDKRMVGVVGDDATIARAMFEAYAQNYLLKYSIAMDKVKHLYSTALQQISSGMTVESVLKVFVGSTRAEAKDLESDVDTNDLVSCIRLCHQEGWEWTTDSWNNLVPTYIKQDTLSTLEVGQFMTANAKYVNANIAKGAAVNLIWRYADFIKLSESMRRQLKVAARKTGLNLLVTTSSLKADVPCMVTPFKIIGGHRRIVSWRRVLIHVFMLLVVLNPQWFTPWYIMRPIEYNVVDFKVIDNAVIRDITSADQCFANKFSAFENWYSNRYGSYVNSRGCPMVVGVVSDIVGSLVPGLPARFLRVGTTLLPLVNYGLGAVGSVCYTPHYAINYDVFDTSACVLAATCTLFSSASGERMPYCADAALIQNASRYDMLKPHVMYPFYEHSGYIRFPEVISAGVHIVRTMAMEYCKVGRCDVSEAGLCMSLQPRWVVNNAYFRQQSGVYCGTSAFDLFMNMLLPIFTPVGAVDITTSILMGALLAVVVSMSLYYLLRFRRAFGDYSGVIFTNILAFVLNVIVLCLEGPYPMLPSIYAMVFLYATCYFGSDIACMMHVSFLIMFAGVVPLWVTVLYIVVVLSRHILWFASLCTKRTVQVGDLAFHSFQDAALQTFMLDKEVFLRLKREISSDAYFKYLAMYNKYKYYSGPMDTAAYREAACSHLVMALEKYSNGGGDTIYQPPRCSVASAALQAGLTRMAHPSGLVEPCLVKVNYGSMTLNGIWLDNFVICPRHVMCSRDELANPDYPRLSMRAANYDFHVSQNGHNIRVIGHTMEGSLLKLTVDVNNPKTPAYSFIRVSTGQAMSLLACYDGLPTGVYTCTLRSNGTMRASFLCGSCGSPGFVMNGKEVQFCYLHQLELPNGTHTGTDFSGVFYGPFEDKQVPQLAAPDCTITVNVLAWLYAAVLSGENWFLTKSSISPAEFNNCAVKYMCQSVTSESLQVLQPLAAKTGISVERMLSALKVLLSAGFCGRTIMGSCSLEDEHTPYDIGRQMLGVKLQGKFQSMFRWTLQWFAIIFVLTILILLQLAQWTFVGALPFTLLLPLIGFVAVCVGFVSLLIKHKHTYLTVYLLPVAMVTAYYNFQYTPEGVQGYLLSLYNYVNPGRIDVIGTDLLTMLIISVACTLLSVRMVRTDAYSRIWYVCTAVGWLYNCWTGSADTVAISYLTFMVSVFTNYTGVACASLYAAQFMVWVLKFLDPTILLLYGRFRCVLVCYLLVGYLCTCYFGVFNLINRLFRCTLGNYEYVVSSQELRYMNSHGLLPPTNSWQALMLNIKLAGIGGIPIYRVSTIQSNMTDLKCTSVVLLSVLQQLRVESSSKLWALCVKLHNEILASNSPTEAFEAFVSLLSVLLSLPGAINLDELCSSILENNSVLQAVASEFSNLSSYVDYENAQKAYDTAVATGAPASTVNALKKAMNVAKSVLDKDVATTRKLERMSELAMTAMYKQARAEDRRSKVTAAMQTMLFNMIRRLDSDALSNILNNARNGVVPLGVIPRTAANKLLLVVPDFSVYTATITMPTLTYAGSAWDVMQVADADGKTVNATDITRENSVNLAWPLVVTAQRQQATSPVKLQNNELMPQTVKRMNVVAGVSQTACVTDAVAYYNATKEGRHVMAILADTDGLAFAKVEKSTGDGFVILELEPPCKFMVDTPKGPALKYLYFTKGLKNLCRGTVLGTLACTVRLHAGSATEVASNSSILSLCSFSVDPEATYKDYLDNGGSPIGNCVKMLTPHTGTGLAITAKPDANIDQESFGGASCCLYCRCHIEHPGASGVCKYKGKFVQIPLVGVNDPIGFCIRNVVCAVCNMWQGYGCPCSSLREINLQARDECFLNESGVLVE

SEQ ID NO: 4 - protein, 468 aa, Nobecovirus
MSGRNRSRSGTPSPKVTFKQESDGSDSESERRNGNRNGARPKNNNSRGSAPKPEKPKAAPPQNVSWFAPLVQTGKAELRFPRGEGVPVSQGVDSTYEHGYWLRTQRSFQKGGKQVLANPRWYFYYTGTGRFGDLRFGTKNPDIVWVGQEGANINRLGDMGTRNPSNDGAIPVQLAGGIPKGFYAEGRGSRGNSRSSSRNSSRASSRGNSRASSRGASPGRPAANPSTEPWMAYLVQKLERLESQVSGTKPATKNPVQVTKNEAAANAKKLRHKRTAHKGSGVTVNYGRRGPGDLEGNFGDREMIKLGTDDPRFAAAAQMAPNVSSFLFMSHLSTRDEDDALWLHYKGAIKLPKDDPNYEQWTKILAENLNAYKDFPPTEPKKDKKKKEETAQDTVIFEDASTGTDQTVVKVWVKDQDAQTDDEWLGGDETVYEDEDDRPKTQRRHKKRGSTASRVTIADPTNAGAERS

SEQ ID NO: 5 - DNA, 955 bp, synthetic construct
  misc_feature 1..955: note = Artificial gene
  source 1..955: mol_type = other DNA
gcggccgcgacaacttggccagagaccgtacggtctcaagctgtccacgtggaattctaagcttaggatccactcgagccaatgtgatggactgaccctatagtgagtcgtattaatttaaatcataccaacatggtcaaataaaacgaaaggctcagtcgaaagactgggcctttcgttttaatctgatcggcacgtaagaggttccaactttcaccataatgaaataagatcactaccgggcgtattttttgagttatcgagattttcaggagctaaggaagctaaaatggagaaaaaaatcactggatataccaccgttgatatatcccaatggcatcgtaaagaacattttgaggcatttcagtcagttgctcaatgtacctataaccagaccgttcagctggatattacggcctttttaaagaccgtaaagaaaaataagcacaagttttatccggcctttattcacattcttgcccgcctgatgaatgctcatccggaatttcgtatggcaatgaaagacggtgagctggtgatatgggatagtgttcacccttgttacaccgttttccatgagcaaactgaaacgttttcatcgctctggagtgaataccacgacgatttccggcagtttctacacatatattcgcaagatgtggcgtgttacggtgaaaacctggcctatttccctaaagggtttattgagaatatgtttttcgtctcagccaatccctgggtgagtttcaccagttttgatttaaacgtggccaatatggacaacttcttcgcccccgttttcaccatgggcaaatattatacgcaaggcgacaaggtgctgatgccgctggcgattcaggttcatcatgccgtttgtgatggcttccatgtcggcagaatgcttaatgaattacaacagtactgcgatgagtggcagggcggggcgtaacctagg

SEQ ID NO: 6 - DNA, 927 bp, synthetic construct
  misc_feature 1..927: note = Template for PCR
  source 1..927: mol_type = other DNA
cagttaacccctacattctacgacaatagctgtcccaacgtgtccaacatcgttcgcgacacaatcgtcaacgagctcagatccgatcccaggatcgctgcttcaatattacgtctgcacttccatgactgcttcgtgaatggttgcgacgctagcatattactggacaacaccaccagtttccgcactgaaaaggatgcattcgggaacgctaacagcgccaggggctttccagtgatcgatcgcatgaaggctgccgttgagtcagcatgcccacgaacagtcagttgtgcagacctgctgactatagctgcgcaacagagcgtgactcttgcaggcggaccgtcctggagagtgccgctcggtcgacgtgactccctacaggcattcctagatctggccaacgccaacttgcctgctccattcttcaccctgccccagctgaaggatagctttagaaacgtgggtctgaatcgctcgagtgaccttgtggctctgtccggaggacacacatttggaaagaaccagtgtaggttcatcatggataggctctacaatttcagcaacactgggttacctgaccccacgctgaacactacgtatctccagacactgagaggcttgtgcccactgaatggcaacctcagtgcactagtggactttgatctgcggaccccaaccatcttcgataacaagtactatgtgaatctagaggagcagaaaggcctgatacagagtgatcaagaactgtttagcagtccaaacgccactgacaccatcccactggtgagaagttttgctaactctactcaaaccttctttaacgccttcgtggaagccatggaccgtatgggtaacattacccctctgacgggtacccaaggccagattcgtctgaactgcagagtggtcaacagcaactcttaa

SEQ ID NO: 7 - DNA, 42 bp, synthetic construct
  misc_feature 1..42: note = Forward primer for PCR fragment A
  source 1..42: mol_type = other DNA
ggaattcggtctcaggcccagttaacccctacattctacgac

SEQ ID NO: 8 - DNA, 44 bp, synthetic construct
  misc_feature 1..44: note = Reverse primer for PCR fragment A
  source 1..44: mol_type = other DNA
cgggatccggtctcaccatttaagagttgctgttgaccactctg

SEQ ID NO: 9 - DNA, 964 bp, synthetic construct
  misc_feature 1..964: note = PCR fragment A
  source 1..964: mol_type = other DNA
ggaattcggtctcaggcccagttaacccctacattctacgacaatagctgtcccaacgtgtccaacatcgttcgcgacacaatcgtcaacgagctcagatccgatcccaggatcgctgcttcaatattacgtctgcacttccatgactgcttcgtgaatggttgcgacgctagcatattactggacaacaccaccagtttccgcactgaaaaggatgcattcgggaacgctaacagcgccaggggctttccagtgatcgatcgcatgaaggctgccgttgagtcagcatgcccacgaacagtcagttgtgcagacctgctgactatagctgcgcaacagagcgtgactcttgcaggcggaccgtcctggagagtgccgctcggtcgacgtgactccctacaggcattcctagatctggccaacgccaacttgcctgctccattcttcaccctgccccagctgaaggatagctttagaaacgtgggtctgaatcgctcgagtgaccttgtggctctgtccggaggacacacatttggaaagaaccagtgtaggttcatcatggataggctctacaatttcagcaacactgggttacctgaccccacgctgaacactacgtatctccagacactgagaggcttgtgcccactgaatggcaacctcagtgcactagtggactttgatctgcggaccccaaccatcttcgataacaagtactatgtgaatctagaggagcagaaaggcctgatacagagtgatcaagaactgtttagcagtccaaacgccactgacaccatcccactggtgagaagttttgctaactctactcaaaccttctttaacgccttcgtggaagccatggaccgtatgggtaacattacccctctgacgggtacccaaggccagattcgtctgaactgcagagtggtcaacagcaactcttaaatggtgagaccggatcccg

SEQ ID NO: 10 - DNA, 42 bp, synthetic construct
  misc_feature 1..42: note = Forward primer for PCR fragment B
  source 1..42: mol_type = other DNA
ggaattcggtctcacctccagttaacccctacattctacgac

SEQ ID NO: 11 - DNA, 44 bp, synthetic construct
  misc_feature 1..44: note = Reverse primer for PCR fragment B
  source 1..44: mol_type = other DNA
cgggatccggtctcaagctttaagagttgctgttgaccactctg

SEQ ID NO: 12 - DNA, 964 bp, synthetic construct
  misc_feature 1..964: note = PCR fragment B
  source 1..964: mol_type = other DNA
ggaattcggtctcacctccagttaacccctacattctacgacaatagctgtcccaacgtgtccaacatcgttcgcgacacaatcgtcaacgagctcagatccgatcccaggatcgctgcttcaatattacgtctgcacttccatgactgcttcgtgaatggttgcgacgctagcatattactggacaacaccaccagtttccgcactgaaaaggatgcattcgggaacgctaacagcgccaggggctttccagtgatcgatcgcatgaaggctgccgttgagtcagcatgcccacgaacagtcagttgtgcagacctgctgactatagctgcgcaacagagcgtgactcttgcaggcggaccgtcctggagagtgccgctcggtcgacgtgactccctacaggcattcctagatctggccaacgccaacttgcctgctccattcttcaccctgccccagctgaaggatagctttagaaacgtgggtctgaatcgctcgagtgaccttgtggctctgtccggaggacacacatttggaaagaaccagtgtaggttcatcatggataggctctacaatttcagcaacactgggttacctgaccccacgctgaacactacgtatctccagacactgagaggcttgtgcccactgaatggcaacctcagtgcactagtggactttgatctgcggaccccaaccatcttcgataacaagtactatgtgaatctagaggagcagaaaggcctgatacagagtgatcaagaactgtttagcagtccaaacgccactgacaccatcccactggtgagaagttttgctaactctactcaaaccttctttaacgccttcgtggaagccatggaccgtatgggtaacattacccctctgacgggtacccaaggccagattcgtctgaactgcagagtggtcaacagcaactcttaaagcttgagaccggatcccg

SEQ ID NO: 13 - DNA, 44 bp, synthetic construct
  misc_feature 1..44: note = Forward primer for PCR fragment C
  source 1..44: mol_type = other DNA
cccaagcttggtctcaatggcagttaacccctacattctacgac

SEQ ID NO: 14 - DNA, 44 bp, synthetic construct
  misc_feature 1..44: note = Reverse primer for PCR fragment C
  source 1..44: mol_type = other DNA
cgggatccggtctcagaggttaagagttgctgttgaccactctg

SEQ ID NO: 15 - DNA, 966 bp, synthetic construct
  misc_feature 1..966: note = PCR fragment C
  source 1..966: mol_type = other DNA
cccaagcttggtctcaatggcagttaacccctacattctacgacaatagctgtcccaacgtgtccaacatcgttcgcgacacaatcgtcaacgagctcagatccgatcccaggatcgctgcttcaatattacgtctgcacttccatgactgcttcgtgaatggttgcgacgctagcatattactggacaacaccaccagtttccgcactgaaaaggatgcattcgggaacgctaacagcgccaggggctttccagtgatcgatcgcatgaaggctgccgttgagtcagcatgcccacgaacagtcagttgtgcagacctgctgactatagctgcgcaacagagcgtgactcttgcaggcggaccgtcctggagagtgccgctcggtcgacgtgactccctacaggcattcctagatctggccaacgccaacttgcctgctccattcttcaccctgccccagctgaaggatagctttagaaacgtgggtctgaatcgctcgagtgaccttgtggctctgtccggaggacacacatttggaaagaaccagtgtaggttcatcatggataggctctacaatttcagcaacactgggttacctgaccccacgctgaacactacgtatctccagacactgagaggcttgtgcccactgaatggcaacctcagtgcactagtggactttgatctgcggaccccaaccatcttcgataacaagtactatgtgaatctagaggagcagaaaggcctgatacagagtgatcaagaactgtttagcagtccaaacgccactgacaccatcccactggtgagaagttttgctaactctactcaaaccttctttaacgccttcgtggaagccatggaccgtatgggtaacattacccctctgacgggtacccaaggccagattcgtctgaactgcagagtggtcaacagcaactcttaacctctgagaccggatcccg

SEQ ID NO: 16 - DNA, 25562 bp, synthetic construct
  misc_feature 1..25562: note = SC2R
  source 1..25562: mol_type = other DNA
gttgacattgattattgactagttattaatagtaatcaattacggggtcattagttcatagcccatatatggagttccgcgttacataacttacggtaaatggcccgcctggctgaccgcccaacgacccccgcccattgacgtcaataatgacgtatgttcccatagtaacgccaatagggactttccattgacgtcaatgggtggagtatttacggtaaactgcccacttggcagtacatcaagtgtatcatatgccaagtacgccccctattgacgtcaatgacggtaaatggcccgcctggcattatgcccagtacatgaccttatgggactttcctacttggcagtacatctacgtattagtcatcgctattaccatggtgatgcggttttggcagtacatcaatgggcgtggataggggtttgactcacggggatttccaagtctccaccccattgacgtcaatgggagtttgttttggcaccaaaatcaacgggactttccaaaatgtcgtaacaactccgccccattgacgcaaatgggcggtaggcgtgtacggtgggaggtctatataagcagagctcgtttagtgaaccattaaaggtttataccttcccaggtaacaaaccaaccaactttcgatctcttgtagatctgttctctaaacgaactttaaaatctgtgtggctgtcactcggctgcatgcttagtgcactcacgcagtataattaataactaattactgtcgttgacaggacacgagtaactcgtctatcttctgcaggctgcttacggtttcgtccgtgttgcagccgatcatcagcacatctaggtttcgtccgggtgtgaccgaaaggtaagatggagagccttgtccctggtttcaacgagaaaacacacgtccaactcagtttgcctgttttacaggttcgcgacgtgctcgtacgtggctttggagactccgtggaggaggtcttatcagaggcacgtcaacatcttaaagatggcacttgtggcttagtagaagttgaaaaaggcgttttgcctcaacttgaacagccctatgtgttcatcaaacgttcggatgctcgaactgcacctcatggtcatgttatggttgagctggtagcagaactcgaaggcattcagtacggtcgtagtggtgagacacttggtgtccttgtccctcatgtgggcgaaataccagtggcttaccgcaaggttcttcttcgtaagaacggtaataaaggagctggtggccatagttacggcgccgatctaaagtcatttgacttaggcgacgagcttggcactgatccttatgaagattttcaagaaaactggaacactaaacatagcagtggtgttacccgtgaactcatgcgtgagcttaacggaggggcatacactcgctatgtcgataacaacttctgtggccctgatggctaccctcttgagtgcattaaagaccttctagcacgtgctggtaaagcttcatgcactttgtccgaacaactggactttattgacactaagaggggtgtatactgctgccgtgaacatgagcatgaaattgcttggtacacggaacgttctgaaaagagctatgaattgcagacaccttttgaaattaaattggcaaagaaatttgacaccttcaatggggaatgtccaaattttgtatttcccttaaattccataatcaagactattcaaccaagggttgaaaagaaaaagcttgatggctttatgggtagaattcgatctgtctatccagttgcgtcaccaaatgaatgcaaccaaatgtgcctttcaactctcatgaagtgtgatcattgtggtgaaacttcatggcagacgggcgattttgttaaagccacttgcgaattttgtggcactgagaatttgactaaagaaggtgccactacttgtggttacttaccccaaaatgctgttgttaaaatttattgtccagcatgtcacaattcagaagtaggacctgagcatagtcttgccgaataccataatgaatctggcttgaaaaccattcttcgtaagggtggtcgcactattgcctttggaggctgtgtgttctcttatgttggttgccataacaagtgtgcctattgggttccacgtgctagcgctaacataggttgtaaccatacaggtgttgttggagaaggttccgaaggtcttaatgacaaccttcttgaaatactccaaaaagagaaagtcaacatcaatattgttggtgactttaaacttaatgaagagatcgccattattttggcatctttttctgcttccacaagtgcttttgtggaaactgtgaaaggtttggattataaagcattcaaacaaattgttgaatcctgtggtaattttaaagttacaaaaggaaaagctaaaaaaggtgcctggaatattggtgaacagaaatcaatactgagtcctctttatgcatttgcatcagaggctgctcgtgttgtacgatcaattttctcccgcactcttgaaactgctcaaaattctgtgcgtgttttacagaaggccgctataacaatactagatggaatttcacagtattcactgagactcattgatgctatgatgttcacatctgatttggctactaacaatctagttgtaatggcctacattacaggtggtgttgttcagttgacttcgcagtggctaactaacatctttggcactgtttatgaaaaactcaaacccgtccttgattggcttgaagagaagtttaaggaaggtgtagagtttcttagagacggttgggaaattgttaaatttatctcaacctgtgcttgtgaaattgtcggtggacaaattgtcacctgtgcaaaggaaattaaggagagtgttcagacattctttaagcttgtaaataaatttttggctttgtgtgctgactctatcattattggtggagctaaacttaaagccttgaatttaggtgaaacatttgtcacgcactcaaagggattgtacagaaagtgtgttaaatccagagaagaaactggcctactcatgcctctaaaagccccaaaagaaattatcttcttagagggagaaacacttcccacagaagtgttaacagaggaagttgtcttgaaaactggtgatttacaaccattagaacaacctactagtgaagctgttgaagctccattggttggtacaccagtttgtattaacgggcttatgttgctcgaaatcaaagacacagaaaagtactgtgcccttgcacctaatatgatggtaacaaacaataccttcacactcaaaggcggtgcaccaacaaaggttacttttggtgatgacactgtgatagaagtgcaaggttacaagagtgtgaatatcacttttgaacttgatgaaaggattgataaagtacttaatgagaagtgctctgcctatacagttgaactcggtacagaagtaaatgagttcgcctgtgttgtggcagatgctgtcataaaaactttgcaaccagtatctgaattacttacaccactgggcattgatttagatgagtggagtatggctacatactacttatttgatgagtctggtgagtttaaattggcttcacatatgtattgttctttctaccctccagatgaggatgaagaagaaggtgattgtgaagaagaagagtttgagccatcaactcaatatgagtatggtactgaagatgattaccaaggtaaacctttggaatttggtgccacttctgctgctcttcaacctgaagaagagcaagaagaagattggttagatgatgatagtcaacaaactgttggtcaacaagacggcagtgaggacaatcagacaactactattcaaacaattgttgaggttcaacctcaattagagatggaacttacaccagttgttcagactattgaagtgaatagttttagtggttatttaaaacttactgacaatgtatacattaaaaatgcagacattgtggaagaagctaaaaaggtaaaaccaacagtggttgttaatgcagccaatgtttaccttaaacatggaggaggtgttgcaggagccttaaataaggctactaacaatgccatgcaagttgaatctgatgattacatagctactaatggaccacttaaagtgggtggtagttgtgttttaagcggacacaatcttgctaaacactgtcttcatgttgtcggcccaaatgttaacaaaggtgaagacattcaacttcttaagagtgcttatgaaaattttaatcagcacgaagttctacttgcaccattattatcagctggtatttttggtgctgaccctatacattctttaagagtttgtgtagatactgttcgcacaaatgtctacttagctgtctttgataaaaatctctatgacaaacttgtttcaagctttttggaaatgaagagtgaaaagcaagttgaacaaaagatcgctgagattcctaaagaggaagttaagccatttataactgaaagtaaaccttcagttgaacagagaaaacaagatgataagaaaatcaaagcttgtgttgaagaagttacaacaactctggaagaaactaagttcctcacagaaaacttgttactttatattgacattaatggcaatcttcatccagattctgccactcttgttagtgacattgacatcactttcttaaagaaagatgctccatatatagtgggtgatgttgttcaagagggtgttttaactgctgtggttatacctactaaaaaggctggtggcactactgaaatgctagcgaaagctttgagaaaagtgccaacagacaattatataaccacttacccgggtcagggtttaaatggttacactgtagaggaggcaaagacagtgcttaaaaagtgtaaaagtgccttttacattctaccatctattatctctaatgagaagcaagaaattcttggaactgtttcttggaatttgcgagaaatgcttgcacatgcagaagaaacacgcaaattaatgcctgtctgtgtggaaactaaagccatagtttcaactatacagcgtaaatataagggtattaaaatacaagagggtgtggttgattatggtgctagattttacttttacaccagtaaaacaactgtagcgtcacttatcaacacacttaacgatctaaatgaaactcttgttacaatgccacttggctatgtaacacatggcttaaatttggaagaagctgctcggtatatgagatctctcaaagtgccagctacagtttctgtttcttcacctgatgctgttacagcgtataatggttatcttacttcttcttctaaaacacctgaagaacattttattgaaaccatctcacttgctggttcctataaagattggtcctattctggacaatctacacaactaggtatagaatttcttaagagaggtgataaaagtgtatattacactagtaatcctaccacattccacctagatggtgaagttatcacctttgacaatcttaagacacttctttctttgagagaagtgaggactattaaggtgtttacaacagtagacaacattaacctccacacgcaagttgtggacatgtcaatgacatatggacaacagtttggtccaacttatttggatggagctgatgttactaaaataaaacctcataattcacatgaaggtaaaacattttatgttttacctaatgatgacactctacgtgttgaggcttttgagtactaccacacaactgatcctagttttctgggtaggtacatgtcagcattaaatcacactaaaaagtggaaatacccacaagttaatggtttaacttctattaaatgggcagataacaactgttatcttgccactgcattgttaacactccaacaaatagagttgaagtttaatccacctgctctacaagatgcttattacagagcaagggctggtgaagctgctaacttttgtgcacttatcttagcctactgtaataagacagtaggtgagttaggtgatgttagagaaacaatgagttacttgtttcaacatgccaatttagattcttgcaaaagagtcttgaacgtggtgtgtaaaacttgtggacaacagcagacaacccttaagggtgtagaagctgttatgtacatgggcacactttcttatgaacaatttaagaaaggtgttcagataccttgtacgtgtggtaaacaagctacaaaatatctagtacaacaggagtcaccttttgttatgatgtcagcaccacctgctcagtatgaacttaagcatggtacatttacttgtgctagtgagtacactggtaattaccagtgtggtcactataaacatataacttctaaagaaactttgtattgcatagacggtgctttacttacaaagtcctcagaatacaaaggtcctattacggatgttttctacaaagaaaacagttacacaacaaccataaaaccagttacttataaattggatggtgttgtttgtacagaaattgaccctaagttggacaattattataagaaagacaattcttatttcacagagcaaccaattgatcttgtaccaaaccaaccatatccaaacgcaagcttcgataattttaagtttgtatgtgataatatcaaatttgctgatgatttaaaccagttaactggttataagaaacctgcttcaagagagcttaaagttacatttttccctgacttaaatggtgatgtggtggctattgattataaacactacacaccctcttttaagaaaggagctaaattgttacataaacctattgtttggcatgttaacaatgcaactaataaagccacgtataaaccaaatacctggtgtatacgttgtctttggagcacaaaaccagttgaaacatcaaattcgtttgatgtactgaagtcagaggacgcgcagggaatggataatcttgcctgcgaagatctaaaaccagtctctgaagaagtagtggaaaatcctaccatacagaaagacgttcttgagtgtaatgtgaaaactaccgaagttgtaggagacattatacttaaaccagcaaataatagtttaaaaattacagaagaggttggccacacagatctaatggctgcttatgtagacaattctagtcttactattaagaaacctaatgaattatctagagtattaggtttgaaaacccttgctactcatggtttagctgctgttaatagtgtcccttgggatactatagctaattatgctaagccttttcttaacaaagttgttagtacaactactaacatagttacacggtgtttaaaccgtgtttgtactaattatatgccttatttctttactttattgctacaattgtgtacttttactagaagtacaaattctagaattaaagcatctatgccgactactatagcaaagaatactgttaagagtgtcggtaaattttgtctagaggcttcatttaattatttgaagtcacctaatttttctaaactgataaatattataatttggtttttactattaagtgtttgcctaggttctttaatctactcaaccgctgctttaggtgttttaatgtctaatttaggcatgccttcttactgtactggttacagagaaggctatttgaactctactaatgtcactattgcaacctactgtactggttctataccttgtagtgtttgtcttagtggtttagattctttagacacctatccttctttagaaactatacaaattaccatttcatcttttaaatgggatttaactgcttttggcttagttgcagagtggtttttggcatatattcttttcactaggtttttctatgtacttggattggctgcaatcatgcaattgtttttcagctattttgcagtacattttattagtaattcttggcttatgtggttaataattaatcttgtacaaatggccccgatttcagctatggttagaatgtacatcttctttgcatcattttattatgtatggaaaagttatgtgcatgttgtagacggttgtaattcatcaacttgtatgatgtgttacaaacgtaatagagcaacaagagtcgaatgtacaactattgttaatggtgttagaaggtccttttatgtctatgctaatggaggtaaaggcttttgcaaactacacaattggaattgtgttaattgtgatacattctgtgctggtagtacatttattagtgatgaagttgcgagagacttgtcactacagtttaaaagaccaataaatcctactgaccagtcttcttacatcgttgatagtgttacagtgaagaatggttccatccatctttactttgataaagctggtcaaaagacttatgaaagacattctctctctcattttgttaacttagacaacctgagagctaataacactaaaggttcattgcctattaatgttatagtttttgatggtaaatcaaaatgtgaagaatcatctgcaaaatcagcgtctgtttactacagtcagcttatgtgtcaacctatactgttactagatcaggcattagtgtctgatgttggtgatagtgcggaagttgcagttaaaatgtttgatgcttacgttaatacgttttcatcaacttttaacgtaccaatggaaaaactcaaaacactagttgcaactgcagaagctgaacttgcaaagaatgtgtccttagacaatgtcttatctacttttatttcagcagctcggcaagggtttgttgattcagatgtagaaactaaagatgttgttgaatgtcttaaattgtcacatcaatctgacatagaagttactggcgatagttgtaataactatatgctcacctataacaaagttgaaaacatgacaccccgtgaccttggtgcttgtattgactgtagtgcgcgtcatattaatgcgcaggtagcaaaaagtcacaacattgctttgatatggaacgttaaagatttcatgtcattgtctgaacaactacgaaaacaaatacgtagtgctgctaaaaagaataacttaccttttaagttgacatgtgcaactactagacaagttgttaatgttgtaacaacaaagatagcacttaagggtggtaaaattgttaataattggttgaagcagttaattaaagttacacttgtgttcctttttgttgctgctattttctatttaataacacctgttcatgtcatgtctaaacatactgacttttcaagtgaaatcataggatacaaggctattgatggtggtgtcactcgtgacatagcatctacagatacttgttttgctaacaaacatgctgattttgacacatggtttagccagcgtggtggtagttatactaatgacaaagcttgcccattgattgctgcagtcataacaagagaagtgggttttgtcgtgcctggtttgcctggcacgatattacgcacaactaatggtgactttttgcatttcttacctagagtttttagtgcagttggtaacatctgttacacaccatcaaaacttatagagtacactgactttgcaacatcagcttgtgttttggctgctgaatgtacaatttttaaagatgcttctggtaagccagtaccatattgttatgataccaatgtactagaaggttctgttgcttatgaaagtttacgccctgacacacgttatgtgctcatggatggctctattattcaatttcctaacacctaccttgaaggttctgttagagtggtaacaacttttgattctgagtactgtaggcacggcacttgtgaaagatcagaagctggtgtttgtgtatctactagtggtagatgggtacttaacaatgattattacagatctttaccaggagttttctgtggtgtagatgctgtaaatttacttactaatatgtttacaccactaattcaacctattggtgctttggacatatcagcatctatagtagctggtggtattgtagctatcgtagtaacatgccttgcctactattttatgaggtttagaagagcttttggtgaatacagtcatgtagttgcctttaatactttactattccttatgtcattcactgtactctgtttaacaccagtttactcattcttacctggtgtttattctgttatttacttgtacttgacattttatcttactaatgatgtttcttttttagcacatattcagtggatggttatgttcacacctttagtacctttctggataacaattgcttatatcatttgtatttccacaaagcatttctattggttctttagtaattacctaaagagacgtgtagtctttaatggtgtttcctttagtacttttgaagaagctgcgctgtgcacctttttgttaaataaagaaatgtatctaaagttgcgtagtgatgtgctattacctcttacgcaatataatagatacttagctctttataataagtacaagtattttagtggagcaatggatacaactagctacagagaagctgcttgttgtcatctcgcaaaggctctcaatgacttcagtaactcaggttctgatgttctttaccaaccaccacaaacctctatcacctcagctgttttgcagagtggttttagaaaaatggcattcccatctggtaaagttgagggttgtatggtacaagtaacttgtggtacaactacacttaacggtctttggcttgatgacgtagtttactgtccaagacatgtgatctgcacctctgaagacatgcttaaccctaattatgaagatttactcattcgtaagtctaatcataatttcttggtacaggctggtaatgttcaactcagggttattggacattctatgcaaaattgtgtacttaagcttaaggttgatacagccaatcctaagacacctaagtataagtttgttcgcattcaaccaggacagactttttcagtgttagcttgttacaatggttcaccatctggtgtttaccaatgtgctatgaggcccaatttcactattaagggttcattccttaatggttcatgtggtagtgttggttttaacatagattatgactgtgtctctttttgttacatgcaccatatggaattaccaactggagttcatgctggcacagacttagaaggtaacttttatggaccttttgttgacaggcaaacagcacaagcagctggtacggacacaactattacagttaatgttttagcttggttgtacgctgctgttataaatggagacaggtggtttctcaatcgatttaccacaactcttaatgactttaaccttgtggctatgaagtacaattatgaacctctaacacaagaccatgttgacatactaggacctctttctgctcaaactggaattgccgttttagatatgtgtgcttcattaaaagaattactgcaaaatggtatgaatggacgtaccatattgggtagtgctttattagaagatgaatttacaccttttgatgttgttagacaatgctcaggtgttactttccaaagtgcagtgaaaagaacaatcaagggtacacaccactggttgttactcacaattttgacttcacttttagttttagtccagagtactcaatggtctttgttcttttttttgtatgaaaatgcctttttaccttttgctatgggtattattgctatgtctgcttttgcaatgatgtttgtcaaacataagcatgcatttctctgtttgtttttgttaccttctcttgccactgtagcttattttaatatggtctatatgcctgctagttgggtgatgcgtattatgacatggttggatatggttgatactagtttgtctggttttaagctaaaagactgtgttatgtatgcatcagctgtagtgttactaatccttatgacagcaagaactgtgtatgatgatggtgctaggagagtgtggacacttatgaatgtcttgacactcgtttataaagtttattatggtaatgctttagatcaagccatttccatgtgggctcttataatctctgttacttctaactactcaggtgtagttacaactgtcatgtttttggccagaggtattgtttttatgtgtgttgagtattgccctattttcttcataactggtaatacacttcagtgtataatgctagtttattgtttcttaggctatttttgtacttgttactttggcctcttttgtttactcaaccgctactttagactgactcttggtgtttatgattacttagtttctacacaggagtttagatatatgaattcacagggactactcccacccaagaatagcatagatgccttcaaactcaacattaaattgttgggtgttggtggcaaaccttgtatcaaagtagccactgtacagtctaaaatgtcagatgtaaagtgcacatcagtagtcttactctcagttttgcaacaactcagagtagaatcatcatctaaattgtgggctcaatgtgtccagttacacaatgacattctcttagctaaagatactactgaagcctttgaaaaaatggtttcactactttctgttttgctttccatgcagggtgctgtagacataaacaagctttgtgaagaaatgctggacaacagggcaaccttacaagctatagcctcagagtttagttcccttccatcatatgcagcttttgctactgctcaagaagcttatgagcaggctgttgctaatggtgattctgaagttgttcttaaaaagttgaagaagtctttgaatgtggctaaatctgaatttgaccgtgatgcagccatgcaacgtaagttggaaaagatggctgatcaagctatgacccaaatgtataaacaggctagatctgaggacaagagggcaaaagttactagtgctatgcagacaatgcttttcactatgcttagaaagttggataatgatgcactcaacaacattatcaacaatgcaagagatggttgtgttcccttgaacataatacctcttacaacagcagccaaactaatggttgtcataccagactataacacatataaaaatacgtgtgatggtacaacatttacttatgcatcagcattgtgggaaatccaacaggttgtagatgcagatagtaaaattgttcaacttagtgaaattagtatggacaattcacctaatttagcatggcctcttattgtaacagctttaagggccaattctgctgtcaaattacagaataatgagcttagtcctgttgcactacgacagatgtcttgtgctgccggtactacacaaactgcttgcactgatgacaatgcgttagcttactacaacacaacaaagggaggtaggtttgtacttgcactgttatccgatttacaggatttgaaatgggctagattccctaagagtgatggaactggtactatctatacagaactggaaccaccttgtaggtttgttacagacacacctaaaggtcctaaagtgaagtatttatactttattaaaggattaaacaacctaaatagaggtatggtacttggtagtttagctgccacagtacgtctacaagctggtaatgcaacagaagtgcctgccaattcaactgtattatctttctgtgcttttgctgtagatgctgctaaagcttacaaagattatctagctagtgggggacaaccaatcactaattgtgttaagatgttgtgtacacacactggtactggtcaggcaataacagttacaccggaagccaatatggatcaagaatcctttggtggtgcatcgtgttgtctgtactgccgttgccacatagatcatccaaatcctaaaggattttgtgacttaaaaggtaagtatgtacaaatacctacaacttgtgctaatgaccctgtgggttttacacttaaaaacacagtctgtaccgtctgcggtatgtggaaaggttatggctgtagttgtgatcaactccgcgaacccatgcttcagtcagctgatgcacaatcgtttttaaacgggtttgcggtgtaagtgcagcccgtcttacaccgtgcggcacaggcactagtactgatgtcgtatacagggcttttgacatctacaatgataaagtagctggttttgctaaattcctaaaaactaattgttgtcgcttccaagaaaaggacgaagatgacaatttaattgattcttactttgtagttaagagacacactttctctaactaccaacatgaagaaacaatttataatttacttaaggattgtccagctgttgctaaacatgacttctttaagtttagaatagacggtgacatggtaccacatatatcacgtcaacgtcttactaaatacacaatggcagacctcgtctatgctttaaggcattttgatgaaggtaattgtgacacattaaaagaaatacttgtcacatacaattgttgtgatgatgattatttcaataaaaaggactggtatgattttgtagaaaacccagatatattacgcgtatacgccaacttaggtgaacgtgtacgccaagctttgttaaaaacagtacaattctgtgatgccatgcgaaatgctggtattgttggtgtactgacattagataatcaagatctcaatggtaactggtatgatttcggtgatttcatacaaaccacgccaggtagtggagttcctgttgtagattcttattattcattgttaatgcctatattaaccttgaccagggctttaactgcagagtcacatgttgacactgacttaacaaagccttacattaagtgggatttgttaaaatatgacttcacggaagagaggttaaaactctttgaccgttattttaaatattgggatcagacataccacccaaattgtgttaactgtttggatgacagatgcattctgcattgtgcaaactttaatgttttattctctacagtgttcccacctacaagttttggaccactagtgagaaaaatatttgttgatggtgttccatttgtagtttcaactggataccacttcagagagctaggtgttgtacataatcaggatgtaaacttacatagctctagacttagttttaaggaattacttgtgtatgctgctgaccctgctatgcacgctgcttctggtaatctattactagataaacgcactacgtgcttttcagtagctgcacttactaacaatgttgcttttcaaactgtcaaacccggtaattttaacaaagacttctatgactttgctgtgtctaagggtttctttaaggaaggaagttctgttgaattaaaacacttcttctttgctcaggatggtaatgctgctatcagcgattatgactactatcgttataatctaccaacaatgtgtgatatcagacaactactatttgtagttgaagttgttgataagtactttgattgttacgatggtggctgtattaatgctaaccaagtcatcgtcaacaacctagacaaatcagctggttttccatttaataaatggggtaaggctagactttattatgattcaatgagttatgaggatcaagatgcacttttcgcatatacaaaacgtaatgtcatccctactataactcaaatgaatcttaagtatgccattagtgcaaagaatagagctcgcaccgtagctggtgtctctatctgtagtactatgaccaatagacagtttcatcaaaaattattgaaatcaatagccgccactagaggagctactgtagtaattggaacaagcaaattctatggtggttggcacaacatgttaaaaactgtttatagtgatgtagaaaaccctcaccttatgggttgggattatcctaaatgtgatagagccatgcctaacatgcttagaattatggcctcacttgttcttgctcgcaaacatacaacgtgttgtagcttgtcacaccgtttctatagattagctaatgagtgtgctcaagtattgagtgaaatggtcatgtgtggcggttcactatatgttaaaccaggtggaacctcatcaggagatgccacaactgcttatgctaatagtgtttttaacatttgtcaagctgtcacggccaatgttaatgcacttttatctactgatggtaacaaaattgccgataagtatgtccgcaatttacaacacagactttatgagtgtctctatagaaatagagatgttgacacagactttgtgaatgagttttacgcatatttgcgtaaacatttctcaatgatgatactctctgacgatgctgttgtgtgtttcaatagcacttatgcatctcaaggtctagtggctagcataaagaactttaagtcagttctttattatcaaaacaatgtttttatgtctgaagcaaaatgttggactgagactgaccttactaaaggacctcatgaattttgctctcaacatacaatgctagttaaacagggtgatgattatgtgtaccttccttacccagatccatcaagaatcctaggggccggctgttttgtagatgatatcgtaaaaacagatggtacacttatgattgaacggttcgtgtctttagctatagatgcttacccacttactaaacatcctaatcaggagtatgctgatgtctttcatttgtacttacaatacataagaaagctacatgatgagttaacaggacacatgttagacatgtattctgttatgcttactaatgataacacttcaaggtattgggaacctgagttttatgaggctatgtacacaccgcatacagtcttacaggctgttggggcttgtgttctttgcaattcacagacttcattaagatgtggtgcttgcatacgtagaccattcttatgttgtaaatgctgttacgaccatgtcatatcaacatcacataaattagtcttgtctgttaatccgtatgtttgcaatgctccaggttgtgatgtcacagatgtgactcaactttacttaggaggtatgagctattattgtaaatcacataaaccacccattagttttccattgtgtgctaatggacaagtttttggtttatataaaaatacatgtgttggtagcgataatgttactgactttaatgcaattgcaacatgtgactggacaaatgctggtgattacattttagctaacacctgtactgaaagactcaagctttttgcagcagaaacgctcaaagctactgaggagacatttaaactgtcttatggtattgctactgtacgtgaagtgctgtctgacagagaattacatctttcatgggaagttggtaaacctagaccaccacttaaccgaaattatgtctttactggttatcgtgtaactaaaaacagtaaagtacaaataggagagtacacctttgaaaaaggtgactatggtgatgctgttgtttaccgaggtacaacaacttacaaattaaatgttggtgattattttgtgctgacatcacatacagtaatgccattaagtgcacctacactagtgccacaagagcactatgttagaattactggcttatacccaacactcaatatctcagatgagttttctagcaatgttgcaaattatcaaaaggttggtatgcaaaagtattctacactccagggaccacctggtactggtaagagtcattttgctattggcctagctctctactacccttctgctcgcatagtgtatacagcttgctctcatgccgctgttgatgcactatgtgagaaggcattaaaatatttgcctatagataaatgtagtagaattatacctgcacgtgctcgtgtagagtgttttgataaattcaaagtgaattcaacattagaacagtatgtcttttgtactgtaaatgcattgcctgagacgacagcagatatagttgtctttgatgaaatttcaatggccacaaattatgatttgagtgttgtcaatgccagattacgtgctaagcactatgtgtacattggcgaccctgctcaattacctgcaccacgcacattgctaactaagggcacactagaaccagaatatttcaattcagtgtgtagacttatgaaaactataggtccagacatgttcctcggaacttgtcggcgttgtcctgctgaaattgttgacactgtgagtgctttggtttatgataataagcttaaagcacataaagacaaatcagctcaatgctttaaaatgttttataagggtgttatcacgcatgatgtttcatctgcaattaacaggccacaaataggcgtggtaagagaattccttacacgtaaccctgcttggagaaaagctgtctttatttcaccttataattcacagaatgctgtagcctcaaagattttgggactaccaactcaaactgttgattcatcacagggctcagaatatgactatgtcatattcactcaaaccactgaaacagctcactcttgtaatgtaaacagatttaatgttgctattaccagagcaaaagtaggcatactttgcataatgtctgatagggacctttatgacaagttgcaatttacaagtcttgaaattccacgtaggaatgtggcaactttacaagctgaaaatgtaacaggactctttaaagattgtagtaaggtaatcactgggttacatcctacacaggcacctacacacctcagtgttgacactaaattcaaaactgaaggtttatgtgttgacatacctggcatacctaaggacatgacctatagaagactcatctctatgatgggttttaaaatgaattatcaagttaatggttaccctaacatgtttatcacccgcgaagaagctataagacatgtacgtgcatggattggcttcgatgtcgaggggtgtcatgctactagagaagctgttggtaccaatttacctttacagctaggtttttctacaggtgttaacctagttgctgtacctacaggttatgttgatacacctaataatacagatttttccagagttagtgctaaaccaccgcctggagatcaatttaaacacctcataccacttatgtacaaaggacttccttggaatgtagtgcgtataaagattgtacaaatgttaagtgacacacttaaaaatctctctgacagagtcgtatttgtcttatgggcacatggctttgagttgacatctatgaagtattttgtgaaaataggacctgagcgcacctgttgtctatgtgatagacgtgccacatgcttttccactgcttcagacacttatgcctgttggcatcattctattggatttgattacgtctataatccgtttatgattgatgttcaacaatggggttttacaggtaacctacaaagcaaccatgatctgtattgtcaagtccatggtaatgcacatgtagctagttgtgatgcaatcatgactaggtgtctagctgtccacgagtgctttgttaagcgtgttgactggactattgaatatcctataattggtgatgaactgaagattaatgcggcttgtagaaaggttcaacacatggttgttaaagctgcattattagcagacaaattcccagttcttcacgacattggtaaccctaaagctattaagtgtgtacctcaagctgatgtagaatggaagttctatgatgcacagccttgtagtgacaaagcttataaaatagaagaattattctattcttatgccacacattctgacaaattcacagatggtgtatgcctattttggaattgcaatgtcgatagatatcctgctaattccattgtttgtagatttgacactagagtgctatctaaccttaacttgcctggttgtgatggtggcagtttgtatgtaaataaacatgcattccacacaccagcttttgataaaagtgcttttgttaatttaaaacaattaccatttttctattactctgacagtccatgtgagtctcatggaaaacaagtagtgtcagatatagattatgtaccactaaagtctgctacgtgtataacacgttgcaatttaggtggtgctgtctgtagacatcatgctaatgagtacagattgtatctcgatgcttataacatgatgatctcagctggctttagcttgtgggtttacaaacaatttgatacttataacctctggaacacttttacaagacttcagagtttagaaaatgtggcttttaatgttgtaaataagggacactttgatggacaacagggtgaagtaccagtttctatcattaataacactgtttacacaaaagttgatggtgttgatgtagaattgtttgaaaataaaacaacattacctgttaatgtagcatttgagctttgggctaagcgcaacattaaaccagtaccagaggtgaaaatactcaataatttgggtgtggacattgctgctaatactgtgatctgggactacaaaagagatgctccagcacatatatctactattggtgtttgttctatgactgacatagccaagaaaccaactgaaacgatttgtgcaccactcactgtcttttttgatggtagagttgatggtcaagtagacttatttagaaatgcccgtaatggtgttcttattacagaaggtagtgttaaaggtttacaaccatctgtaggtcccaaacaagctagtcttaatggagtcacattaattggagaagccgtaaaaacacagttcaattattataagaaagttgatggtgttgtccaacaattacctgaaacttactttactcagagtagaaatttacaagaatttaaacccaggagtcaaatggaaattgatttcttagaattagctatggatgaattcattgaacggtataaattagaaggctatgccttcgaacatatcgtttatggagattttagtcatagtcagttaggtggtttacatctactgattggactagctaaacgttttaaggaatcaccttttgaattagaagattttattcctatggacagtacagttaaaaactatttcataacagatgcgcaaacaggttcatctaagtgtgtgtgttctgttattgatttattacttgatgattttgttgaaataataaaatcccaagatttatctgtagtttctaaggttgtcaaagtgactattgactatacagaaatttcatttatgctttggtgtaaagatggccatgtagaaacattttacccaaaattacaatctagtcaagcgtggcaaccgggtgttgctatgcctaatctttacaaaatgcaaagaatgctattagaaaagtgtgaccttcaaaattatggtgatagtgcaacattacctaaaggcataatgatgaatgtcgcaaaatatactcaactgtgtcaatatttaaacacattaacattagctgtaccctataatatgagagttatacattttggtgctggttctgataaaggagttgcaccaggtacagctgttttaagacagtggttgcctacgggtacgctgcttgtcgattcagatcttaatgactttgtctctgatgcagattcaactttgattggtgattgtgcaactgtacatacagctaataaatgggatctcattattagtgatatgtacgaccctaagactaaaaatgttacaaaagaaaatgactctaaagagggttttttcacttacatttgtgggtttatacaacaaaagctagctcttggaggttccgtggctataaagataacagaacattcttggaatgctgatctttataagctcatgggacacttcgcatggtggacagcctttgttactaatgtgaatgcgtcatcatctgaagcatttttaattggatgtaattatcttggcaaaccacgcgaacaaatagatggttatgtcatgcatgcaaattacatattttggaggaatacaaatccaattcagttgtcttcctattctttatttgacatgagtaaatttccccttaaattaaggggtactgctgttatgtctttaaaagaaggtcaaatcaatgatatgattttatctcttcttagtaaaggtagacttataattagagaaaacaacagagttgttatttctagtgatgttcttgttaacaactaaacgaacaatgaactccttctccacaagcgccttcggtccagttgccttctccctgggcctgctcctggtgttgcctgctgccttccctgccccagtcttcacactcgaagatttcgttggggactggcgacagacagccggctacaacctggaccaagtccttgaacagggaggtgtgtccagtttgtttcagaatctcggggtgtccgtaactccgatccaaaggattgtcctgagcggtgaaaatgggctgaagatcgacatccatgtcatcatcccgtatgaaggtctgagcggcgaccaaatgggccagatcgaaaaaatttttaaggtggtgtaccctgtggatgatcatcactttaaggtgatcctgcactatggcacactggtaatcgacggggttacgccgaacatgatcgactatttcggacggccgtatgaaggcatcgccgtgttcgacggcaaaaagatcactgtaacagggaccctgtggaacggcaacaaaattatcgacgagcgcctgatcaaccccgacggctccctgctgttccgagtaaccatcaacggagtgaccggctggcggctgtgcgaacgcattctggcgtaaacgaactaaatattatattagtttttctgtttggaactttaattttagccatgattgaacaagatggattgcacgcaggttctccggccgcttgggtggagaggctattcggctatgactgggcacaacagacaatcggctgctctgatgccgccgtgttccggctgtcagcgcaggggcgcccggttctttttgtcaagaccgacctgtccggtgccctgaatgaactgcaagacgaggcagcgcggctatcgtggctggccacgacgggcgttccttgcgcagctgtgctcgacgttgtcactgaagcgggaagggactggctgctattgggcgaagtgccggggcaggatctcctgtcatctcaccttgctcctgccgagaaagtatccatcatggctgatgcaatgcggcggctgcatacgcttgatccggctacctgcccattcgaccaccaagcgaaacatcgcatcgagcgagcacgtactcggatggaagccggtcttgtcgatcaggatgatctggacgaagagcatcaggggctcgcgccagccgaactgttcgccaggctcaaggcgagcatgcccgacggcgaggatctcgtcgtgacccatggcgatgcctgcttgccgaatatcatggtggaaaatggccgcttttctggattcatcgactgtggccggctgggtgtggcggaccgctatcaggacatagcgttggctacccgtgatattgctgaagagcttggcggcgaatgggctgaccgcttcctcgtgctttacggtatcgccgctcccgattcgcagcgcatcgccttctatcgccttcttgacgagttcttctgaacgaacaaactaaaatgtctgataatggaccccaaaatcagcgaaatgcaccccgcattacgtttggtggaccctcagattcaactggcagtaaccagaatggagaacgcagtggggcgcgatcaaaacaacgtcggccccaaggtttacccaataatactgcgtcttggttcaccgctctcactcaacatggcaaggaagaccttaaattccctcgaggacaaggcgttccaattaacaccaatagcagtccagatgaccaaattggctactaccgaagagctaccagacgaattcgtggtggtgacggtaaaatgaaagatctcagtccaagatggtatttctactacctaggaactgggccagaagctggacttccctatggtgctaacaaagacggcatcatatgggttgcaactgagggagccttgaatacaccaaaagatcacattggcacccgcaatcctgctaacaatgctgcaatcgtgctacaacttcctcaaggaacaacattgccaaaaggcttctacgcagaagggagcagaggcggcagtcaagcctcttctcgttcctcatcacgtagtcgcaacagttcaagaaattcaactccaggcagcagtaggggaacttctcctgctagaatggctggcaatggcggtgatgctgctcttgctttgctgctgcttgacagattgaaccagcttgagagcaaaatgtctggtaaaggccaacaacaacaaggccaaactgtcactaagaaatctgctgctgaggcttctaagaagcctcggcaaaaacgtactgccactaaagcatacaatgtaacacaagctttcggcagacgtggtccagaacaaacccaaggaaattttggggaccaggaactaatcagacaaggaactgattacaaacattggccgcaaattgcacaatttgcccccagcgcttcagcgttcttcggaatgtcgcgcattggcatggaagtcacaccttcgggaacgtggttgacctacacaggtgccatcaaattggatgacaaagatccaaatttcaaagatcaagtcattttgctgaataagcatattgacgcatacaaaacattcccaccaacagagcctaaaaaggacaaaaagaagaaggctgatgaaactcaagccttaccgcagagacagaagaaacagcaaactgtgactcttcttcctgctgcagatttggatgatttctccaaacaattgcaacaatccatgagcagtgctgactcaactcaggcctaaactcatgcagaccacacaaggcagatgggctatataaacgttttcgcttttccgtttacgatatatagtctactcttgtgcagaatgaattctcgtaactacatagcacaagtagatgtagttaactttaatctcacatagcaatctttaatcagtgtgtaacattagggaggacttgaaagagccaccacattttcaccgaggccacgcggagtacgatcgagtgtacagtgaacaatgctagggagagctgcctatatggaagagccctaatgtgtaaaattaattttagtagtgctatccccatgtgattttaatagcttcttaggagaatgacaaaaaaaaaaaaaaaaaaaaaaaaaaaaaaaaggccggcatggtcccagcctcctcgctggcgccggctgggcaacattccgaggggaccgtcccctcggtaatggcgaatgggacccactgtgccttctagttgccagccatctgttgtttgcccctcccccgtgccttccttgaccctggaaggtgccactcccactgtcctttcctaataaaatgaggaaattgcatcgcattgtctgagtaggtgtcattctattctggggggtggggtggggcaggacagcaagggggaggattgggaagacaatagcaggcatgctggggatgcggtgggctctatgg

SEQ ID NO: 17 - DNA, 25623 bp, synthetic construct
  source 1..25623: mol_type = other DNA
gttgacattgattattgactagttattaatagtaatcaattacggggtcattagttcatagcccatatatggagttccgcgttacataacttacggtaaatggcccgcctggctgaccgcccaacgacccccgcccattgacgtcaataatgacgtatgttcccatagtaacgccaatagggactttccattgacgtcaatgggtggagtatttacggtaaactgcccacttggcagtacatcaagtgtatcatatgccaagtacgccccctattgacgtcaatgacggtaaatggcccgcctggcattatgcccagtacatgaccttatgggactttcctacttggcagtacatctacgtattagtcatcgctattaccatggtgatgcggttttggcagtacatcaatgggcgtggataggggtttgactcacggggatttccaagtctccaccccattgacgtcaatgggagtttgttttggcaccaaaatcaacgggactttccaaaatgtcgtaacaactccgccccattgacgcaaatgggcggtaggcgtgtacggtgggaggtctatataagcagagctcgtttagtgaaccatattaggtttttacctacccaggaaaagccaaccaacctcgatctcttgtagatctgttctctaaacgaactttaaaatctgtgtagctgtcgctcggctgcatgcctagtgcacctacgcagtataaacaataataaattttactgtcgttgacaagaaacgagtaactcgtccctcttctgcagactgcttacggtttcgtccgtgttgcagtcgatcatcagcatacctaggtttcgtccgggtgtgaccgaaaggtaagatggagagccttgttcttggtgtcaacgagaaaacacacgtccaactcagtttgcctgtccttcaggttagagacgtgctagtgcgtggcttcggggactctgtggaagaggccctatcggaggcacgtgaacacctcaaaaatggcacttgtggtctagtagagctggaaaaaggcgtactgccccagcttgaacagccctatgtgttcattaaacgttctgatgccttaagcaccaatcacggccacaaggtcgttgagctggttgcagaaatggacggcattcagtacggtcgtagcggtataacactgggagtactcgtgccacatgtgggcgaaaccccaattgcataccgcaatgttcttcttcgtaagaacggtaataagggagccggtggtcatagctatggcatcgatctaaagtcttatgacttaggtgacgagcttggcactgatcccattgaagattatgaacaaaactggaacactaagcatggcagtggtgcactccgtgaactcactcgtgagctcaatggaggtgcagtcactcgctatgtcgacaacaatttctgtggcccagatgggtaccctcttgattgcatcaaagattttctcgcacgcgcgggcaagtcaatgtgcactctttccgaacaacttgattacatcgagtcgaagagaggtgtctactgctgccgtgaccatgagcatgaaattgcctggttcactgagcgctctgataagagctacgagcaccagacacccttcgaaattaagagtgccaagaaatttgacactttcaaaggggaatgcccaaagtttgtgtttcctcttaactcaaaagtcaaagtcattcaaccacgtgttgaaaagaaaaagactgagggtttcatggggcgtatacgctctgtgtaccctgttgcatctccacaggagtgtaacaatatgcacttgtctaccttgatgaaatgtaatcattgcgatgaagtttcatggcagacgtgcgactttctgaaagccacttgtgaacattgtggcactgaaaatttagttattgaaggacctactacatgtgggtacctacctactaatgctgtagtgaaaatgccatgtcctgcctgtcaagacccagagattggacctgagcatagtgttgcagattatcacaaccactcaaacattgaaactcgactccgcaagggaggtaggactagatgttttggaggctgtgtgtttgcctatgttggctgctataataagcgtgcctactgggttcctcgtgctagtgctgatattggctcaggccatactggcattactggtgacaatgtggagactttgaatgaggatctccttgagatactgagtcgtgaacgtgttaacattaacattgttggcgattttcatttgaatgaagaggttgccatcattttggcatctttctctgcttctacaagtgcctttattgacactataaagagtcttgattacaagtctttcaaaaccattgttgagtcctgcggtaactataaagttaccaagggaaagcccgtaaaaggtgcttggaacattggacaacagagatcagttttaacaccactgtgtggttttccctcacaggctgctggtgttatcagatcaatttttgcgcgcacacttgatgcagcaaaccactcaattcctgatttgcaaagagcagctgtcaccatacttgatggtatttctgaacagtcattacgtcttgtcgacgccatggtttatacttcagacctgctcaccaacagtgtcattattatggcatatgtaactggtggtcttgtacaacagacttctcagtggttgtctaatcttttgggcactactgttgaaaaactcaggcctatctttgaatggattgaggcgaaacttagtgcaggagttgaatttctcaaggatgcttgggagattctcaaatttctcattacaggtgtttttgacatcgtcaagggtcaaatacaggttgcttcagataacatcaaggattgtgtaaaatgcttcattgatgttgttaacaaggcactcgaaatgtgcattgatcaagtcactatcgctggcgcaaagttgcgatcactcaacttaggtgaagtcttcatcgctcaaagcaagggactttaccgtcagtgtatacgtggcaaggagcagctgcaactactcatgcctcttaaggcaccaaaagaagtaacctttcttgaaggtgattcacatgacacagtacttacctctgaggaggttgttctcaagaacggtgaactcgaagcactcgagacgcccgttgatagcttcacaaatggagctatcgttggcacaccagtctgtgtaaatggcctcatgctcttagagattaaggacaaagaacaatactgcgcattgtctcctggtttactggctacaaacaatgtctttcgcttaaaagggggtgcaccaattaaaggtgtaacctttggagaagatactgtttgggaagttcaaggttacaagaatgtgagaatcacatttgagcttgatgaacgtgttgacaaagtgcttaatgaaaagtgctctgtctacactgttgaatccggtaccgaagttactgagtttgcatgtgttgtagcagaggctgttgtgaagactttacaaccagtttctgatctccttaccaacatgggtattgatcttgatgagtggagtgtagctacattctacttatttgatgatgctggtgaagaaaacttttcatcacgtatgtattgttccttttaccctccagatgaggaagaagaggacgatgcagagtgtgaggaagaagaaattgatgaaacctgtgaacatgagtacggtacagaggatgattatcaaggtcttcctctggaatttggtgcctcagctgaaacagttcgagttgaggaagaagaagaggaagactggctggatgatactactgagcaatcagagattgagccagaaccagaacctacacctgaagaaccagttaatcagtttactggttatttaaaacttactgacaatgttgccattaaatgtgttgacatcgttaaggaggcacaaagtgctaatcctatggtgattgtaaatgctgctaacatacacctgaaacatggtggtggtgtagcaggtgcactcaacaaggcaaccaatggtgccatgcaaaaggagagtgatgattacattaagctaaatggccctcttacagtaggagggtcttgtttgctttctggacataatcttgctaagaagtgtctgcatgttgttggacctaacctaaatgcaggtgaggacatccagcttcttaaggcagcatatgaaaatttcaattcacaggacatcttacttgcaccattgttgtcagcaggcatatttggtgctaaaccacttcagtctttacaagtgtgcgtgcagacggttcgtacacaggtttatattgcagtcaatgacaaagctctttatgagcaggttgtcatggattatcttgataacctgaagcctagagtggaagcacctaaacaagaggagccaccaaacacagaagattccaaaactgaggagaaatctgtcgtacagaagcctgtcgatgtgaagccaaaaattaaggcctgcattgatgaggttaccacaacactggaagaaactaagtttcttaccaataagttactcttgtttgctgatatcaatggtaagctttaccatgattctcagaacatgcttagaggtgaagatatgtctttccttgagaaggatgcaccttacatggtaggtgatgttatcactagtggtgatatcacttgtgttgtaataccctccaaaaaggctggtggcactactgagatgctctcaagagctttgaagaaagtgccagttgatgagtatataaccacgtaccctggacaaggatgtgctggttatacacttgaggaagctaagactgctcttaagaaatgcaaatctgcattttatgtactaccttcagaagcacctaatgctaaggaagagattctaggaactgtatcctggaatttgagagaaatgcttgctcatgctgaagagacaagaaaattaatgcctatatgcatggatgttagagccataatggcaaccatccaacgtaagtataaaggaattaaaattcaagagggcatcgttgactatggtgtccgattcttcttttatactagtaaagagcctgtagcttctattattacgaagctgaactctctaaatgagccgcttgtcacaatgccaattggttatgtgacacatggttttaatcttgaagaggctgcgcgctgtatgcgttctcttaaagctcctgccgtagtgtcagtatcatcaccagatgctgttactacatataatggatacctcacttcgtcatcaaagacatctgaggagcactttgtagaaacagtttctttggctggctcttacagagattggtcctattcaggacagcgtacagagttaggtgttgaatttcttaagcgtggtgacaaaattgtgtaccacactctggagagccccgtcgagtttcatcttgacggtgaggttctttcacttgacaaactaaagagtctcttatccctgcgggaggttaagactataaaagtgttcacaactgtggacaacactaatctccacacacagcttgtggatatgtctatgacatatggacagcagtttggtccaacatacttggatggtgctgatgttacaaaaattaaacctcatgtaaatcatgagggtaagactttctttgtactacctagtgatgacacactacgtagtgaagctttcgagtactaccatactcttgatgagagttttcttggtaggtacatgtctgctttaaaccacacaaagaaatggaaatttcctcaagttggtggtttaacttcaattaaatgggctgataacaattgttatttgtctagtgttttattagcacttcaacagcttgaagtcaaattcaatgcaccagcacttcaagaggcttattatagagcccgtgctggtgatgctgctaacttttgtgcactcatactcgcttacagtaataaaactgttggcgagcttggtgatgtcagagaaactatgacccatcttctacagcatgctaatttggaatctgcaaagcgagttcttaatgtggtgtgtaaacattgtggtcagaaaactactaccttaacgggtgtagaagctgtgatgtatatgggtactctatcttatgataatcttaagacaggtgtttccattccatgtgtgtgtggtcgtgatgctacacaatatctagtacaacaagagtcttcttttgttatgatgtctgcaccacctgctgagtataaattacagcaaggtacattcttatgtgcgaatgagtacactggtaactatcagtgtggtcattacactcatataactgctaaggagactctctatcgtattgacggagctcaccttacaaagatgtcagagtacaaaggaccagtgactgatgttttctacaaggaaacatcttacactacaaccatcaagcctgtgtcgtataaactcgatggagttacttacacagagattgaaccaaaattggatgggtattataaaaaggataatgcttactatacagagcagcctatagaccttgtaccaactcaaccattaccaaatgcgagttttgataatttcaaactcacatgttctaacacaaaatttgctgatgatttaaatcaaatgacaggcttcacaaagccagcttcacgagagctatctgtcacattcttcccagacttgaatggcgatgtagtggctattgactatagacactattcagcgagtttcaagaaaggtgctaaattactgcataagccaattgtttggcacattaaccaggctacaaccaagacaacgttcaaaccaaacacttggtgtttacgttgtctttggagtacaaagccagtagatacttcaaattcatttgaagttctggcagtagaagacacacaaggaatggacaatcttgcttgtgaaagtcaacaacccacctctgaagaagtagtggaaaatcctaccatacagaaggaagtcatagagtgtgacgtgaaaactaccgaagttgtaggcaatgtcatacttaaaccatcagatgaaggtgttaaagtaacacaagagttaggtcatgaggatcttatggctgcttatgtggaaaacacaagcattaccattaagaaacctaatgagctttcactagccttaggtttaaaaacaattgccactcatggtattgctgcaattaatagtgttccttggagtaaaattttggcttatgtcaaaccattcttaggacaagcagcaattacaacatcaaattgcgctaagagattagcacaacgtgtgtttaacaattatatgccttatgtgtttacattattgttccaattgtgtacttttactaaaagtaccaattctagaattagagcttcactacctacaactattgctaaaaatagtgttaagagtgttgctaaattatgtttggatgccggcattaattatgtgaagtcacccaaattttctaaattgttcacaatcgctatgtggctattgttgttaagtatttgcttaggttctctaatctgtgtaactgctgcttttggtgtactcttatctaattttggtgctccttcttattgtaatggcgttagagaattgtatcttaattcgtctaacgttactactatggatttctgtgaaggttcttttccttgcagcatttgtttaagtggattagactcccttgattcttatccagctcttgaaaccattcaggtgacgatttcatcgtacaagctagacttgacaattttaggtctggccgctgagtgggttttggcatatatgttgttcacaaaattcttttatttattaggtctttcagctataatgcaggtgttctttggctattttgctagtcatttcatcagcaattcttggctcatgtggtttatcattagtattgtacaaatggcacccgtttctgcaatggttaggatgtacatcttctttgcttctttctactacatatggaagagctatgttcatatcatggatggttgcacctcttcgacttgcatgatgtgctataagcgcaatcgtgccacacgcgttgagtgtacaactattgttaatggcatgaagagatctttctatgtctatgcaaatggaggccgtggcttctgcaagactcacaattggaattgtctcaattgtgacacattttgcactggtagtacattcattagtgatgaagttgctcgtgatttgtcactccagtttaaaagaccaatcaaccctactgaccagtcatcgtatattgttgatagtgttgctgtgaaaaatggcgcgcttcacctctactttgacaaggctggtcaaaagacctatgagagacatccgctctcccattttgtcaatttagacaatttgagagctaacaacactaaaggttcactgcctattaatgtcatagtttttgatggcaagtccaaatgcgacgagtctgcttctaagtctgcttctgtgtactacagtcagctgatgtgccaacctattctgttgcttgaccaagctcttgtatcagacgttggagatagtactgaagtttccgttaagatgtttgatgcttatgtcgacaccttttcagcaacttttagtgttcctatggaaaaacttaaggcacttgttgctacagctcacagcgagttagcaaagggtgtagctttagatggtgtcctttctacattcgtgtcagctgcccgacaaggtgttgttgataccgatgttgacacaaaggatgttattgaatgtctcaaactttcacatcactctgacttagaagtgacaggtgacagttgtaacaatttcatgctcacctataataaggttgaaaacatgacgcccagagatcttggcgcatgtattgactgtaatgcaaggcatatcaatgcccaagtagcaaaaagtcacaatgtttcactcatctggaatgtaaaagactacatgtctttatctgaacagctgcgtaaacaaattcgtagtgctgccaagaagaacaacataccttttagactaacttgtgctacaactagacaggttgtcaatgtcataactactaaaatctcactcaagggtggtaagattgttagtacttgttttaaacttatgcttaaggccacattattgtgcgttcttgctgcattggtttgttatatcgttatgccagtacatacattgtcaatccatgatggttacacaaatgaaatcattggttacaaagccattcaggatggtgtcactcgtgacatcatttctactgatgattgttttgcaaataaacatgctggttttgacgcatggtttagccagcgtggtggttcatacaaaaatgacaaaagctgccctgtagtagctgctatcattacaagagagattggtttcatagtgcctggcttaccgggtactgtgctgagagcaatcaatggtgacttcttgcattttctacctcgtgtttttagtgctgttggcaacatttgctacacaccttccaaactcattgagtatagtgattttgctacctctgcttgcgttcttgctgctgagtgtacaatttttaaggatgctatgggcaaacctgtgccatattgttatgacactaatttgctagagggttctatttcttatagtgagcttcgtccagacactcgttatgtgcttatggatggttccatcatacagtttcctaacacttacctggagggttctgttagagtagtaacaacttttgatgctgagtactgtagacatggtacatgcgaaaggtcagaagtaggtatttgcctatctaccagtggtagatgggttcttaataatgagcattacagagctctatcaggagttttctgtggtgttgatgcgatgaatctcatagctaacatctttactcctcttgtgcaacctgtgggtgctttagatgtgtctgcttcagtagtggctggtggtattattgccatattggtgacttgtgctgcctactactttatgaaattcagacgtgtttttggtgagtacaaccatgttgttgctgctaatgcacttttgtttttgatgtctttcactatactctgtctggtaccagcttacagctttctgccgggagtctactcagtcttttacttgtacttgacattctatttcaccaatgatgtttcattcttggctcaccttcaatggtttgccatgttttctcctattgtgcctttttggataacagcaatctatgtattctgtatttctctgaagcactgccattggttctttaacaactatcttaggaaaagagtcatgtttaatggagttacatttagtaccttcgaggaggctgctttgtgtacctttttgctcaacaaggaaatgtacctaaaattgcgtagcgagacactgttgccacttacacagtataacaggtatcttgctctatataacaagtacaagtatttcagtggagccttagatactaccagctatcgtgaagcagcttgctgccacttagcaaaggctctaaatgactttagcaactcaggtgctgatgttctctaccaaccaccacagacatcaatcacttctgctgttctgcagagtggttttaggaaaatggcattcccgtcaggcaaagttgaagggtgcatggtacaagtaacctgtggaactacaactcttaatggattgtggttggatgacacagtatactgtccaagacatgtcatttgcacagcagaagacatgcttaatcctaactatgaagatctgctcattcgcaaatccaaccatagctttcttgttcaggctggcaatgttcaacttcgtgttattggccattctatgcaaaattgtctgcttaggcttaaagttgatacttctaaccctaagacacccaagtataaatttgtccgtatccaacctggtcaaacattttcagttctagcatgctacaatggttcaccatctggtgtttatcagtgtgccatgaggcctaatcataccattaaaggttctttccttaatggatcatgtggtagtgttggttttaacattgattatgattgcgtgtctttctgctatatgcatcatatggagcttccaacaggagtacacgctggtactgacttagaaggtaaattctatggtccatttgttgacagacaaactgcacaggctgcaggtacagacacaaccataacattaaatgttttggcatggctgtatgctgctgttatcaatggtgataggtggtttcttaatagattcaccactactttgaatgactttaaccttgtggcaatgaagtacaactatgaacctttgacacaagatcatgttgacatattgggacctctttctgctcaaacaggaattgccgtcttagatatgtgtgctgctttgaaagagctgctgcagaatggtatgaatggtcgtactatccttggtagcactattttagaagatgagtttacaccatttgatgttgttagacaatgctctggtgttaccttccaaggtaagttcaagaaaattgttaagggcactcatcattggatgcttttaactttcttgacatcactattgattcttgttcaaagtacacagtggtcactgtttttctttgtttacgagaatgctttcttgccatttactcttggtattatggcaattgctgcatgtgctatgctgcttgttaagcataagcacgcattcttgtgcttgtttctgttaccttctcttgcaacagttgcttactttaatatggtctacatgcctgctagctgggtgatgcgtatcatgacatggcttgaattggctgacactagcttgtctggttataggcttaaggattgtgttatgtatgcttcagctttagttttgcttattctcatgacagctcgcactgtttatgatgatgctgctagacgtgtttggacactgatgaatgtcattacacttgtttacaaagtctactatggtaatgctttagatcaagctatttccatgtgggccttagttatttctgtaacctctaactattctggtgtcgttacgactatcatgtttttagctagagctatagtgtttgtgtgtgttgagtattacccattgttatttattactggcaacaccttacagtgtatcatgcttgtttattgtttcttaggctattgttgctgctgctactttggccttttctgtttactcaaccgttacttcaggcttactcttggtgtttatgactacttggtatctacacaagaatttaggtatatgaactcccaggggcttttgcctcctaagagtagtattgatgctttcaagcttaacattaagttgttgggtattggaggtaaaccatgtatcaaggttgctactgtacagtctaaaatgtctgacgtaaagtgcacatctgtggtactgctctcggttcttcaacaacttagagtagagtcatcttctaaattgtgggcacaatgtgtacaactccacaatgatattcttcttgcaaaagacacaactgaagctttcgagaagatggtttctcttttgtctgttttgctatccatgcagggtgctgtagacattaataggttgtgcgaggaaatgctcgataaccgtgctactcttcaggctattgcttcagaatttagttctttaccatcatatgccgcttatgccactgcccaggaggcctatgagcaggctgtagctaatggtgattctgaagtcgttctcaaaaagttaaagaaatctttgaatgtggctaaatctgagtttgaccgtgatgctgccatgcaacgcaagttggaaaagatggcagatcaggctatgacccaaatgtacaaacaggcaagatctgaggacaagagggcaaaagtaactagtgctatgcaaacaatgctcttcactatgcttaggaagcttgataatgatgcacttaacaacattatcaacaatgcgcgtgatggttgtgttccactcaacatcataccattgactacagcagccaaactcatggttgttgtccctgattatggtacctacaagaacacttgtgatggtaacacctttacatatgcatctgcactctgggaaatccagcaagttgttgatgcggatagcaagattgttcaacttagtgaaattaacatggacaattcaccaaatttggcttggcctcttattgttacagctctaagagccaactcagctgttaaactacagaataatgaactgagtccagtagcactacgacagatgtcctgtgcggctggtaccacacaaacagcttgtactgatgacaatgcacttgcctactataacaattcgaagggaggtaggtttgtgctggcattactatcagaccaccaagatctcaaatgggctagattccctaagagtgatggtacaggtacaatttacacagaactggaaccaccttgtaggtttgttacagacacaccaaaagggcctaaagtgaaatacttgtacttcatcaaaggcttaaacaacctaaatagaggtatggtgctgggcagtttagctgctacagtacgtcttcaggctggaaatgctacagaagtacctgccaattcaactgtgctttccttctgtgcttttgcagtagaccctgctaaagcatataaggattacctagcaagtggaggacaaccaatcaccaactgtgtgaagatgttgtgtacacacactggtacaggacaggcaattactgtaacaccagaagctaacatggaccaagagtcctttggtggtgcttcatgttgtctgtattgtagatgccacattgaccatccaaatcctaaaggattctgtgacttgaaaggtaagtacgtccaaatacctaccacttgtgctaatgacccagtgggttttacacttagaaacacagtctgtaccgtctgcggaatgtggaaaggttatggctgtagttgtgaccaactccgcgaacccttgatgcagtctgcggatgcatcaacgtttttaaacgggtttgcggtgtaagtgcagcccgtcttacaccgtgcggcacaggcactagtactgatgtcgtctacagggcttttgatatttacaacgaaaaagttgctggttttgcaaagttcctaaaaactaattgctgtcgcttccaggagaaggatgaggaaggcaatttattagactcttactttgtagttaagaggcatactatgtctaactaccaacatgaagagactatttataacttggttaaagattgtccagcggttgctgtccatgactttttcaagtttagagtagatggtgacatggtaccacatatatcacgtcagcgtctaactaaatacacaatggctgatttagtctatgctctacgtcattttgatgagggtaattgtgatacattaaaagaaatactcgtcacatacaattgctgtgatgatgattatttcaataagaaggattggtatgacttcgtagagaatcctgacatcttacgcgtatatgctaacttaggtgagcgtgtacgccaatcattattaaagactgtacaattctgcgatgctatgcgtgatgcaggcattgtaggcgtactgacattagataatcaggatcttaatgggaactggtacgatttcggtgatttcgtacaagtagcaccaggctgcggagttcctattgtggattcatattactcattgctgatgcccatcctcactttgactagggcattggctgctgagtcccatatggatgctgatctcgcaaaaccacttattaagtgggatttgctgaaatatgattttacggaagagagactttgtctcttcgaccgttattttaaatattgggaccagacataccatcccaattgtattaactgtttggatgataggtgtatccttcattgtgcaaactttaatgtgttattttctactgtgtttccacctacaagttttggaccactagtaagaaaaatatttgtagatggtgttccttttgttgtttcaactggataccattttcgtgagttaggagtcgtacataatcaggatgtaaacttacatagctcgcgtctcagtttcaaggaacttttagtgtatgctgctgatccagctatgcatgcagcttctggcaatttattgctagataaacgcactacatgcttttcagtagctgcactaacaaacaatgttgcttttcaaactgtcaaacccggtaattttaataaagacttttatgactttgctgtgtctaaaggtttctttaaggaaggaagttctgttgaactaaaacacttcttctttgctcaggatggcaacgctgctatcagtgattatgactattatcgttataatctgccaacaatgtgtgatatcagacaactcctattcgtagttgaagttgttgataaatactttgattgttacgatggtggctgtattaatgccaaccaagtaatcgttaacaatctggataaatcagctggtttcccatttaataaatggggtaaggctagactttattatgactcaatgagttatgaggatcaagatgcacttttcgcgtatactaagcgtaatgtcatccctactataactcaaatgaatcttaagtatgccattagtgcaaagaatagagctcgcaccgtagctggtgtctctatctgtagtactatgacaaatagacagtttcatcagaaattattgaagtcaatagccgccactagaggagctactgtggtaattggaacaagcaagttttacggtggctggcataatatgttaaaaactgtttacagtgatgtagaaactccacaccttatgggttgggattatccaaaatgtgacagagccatgcctaacatgcttaggataatggcctctcttgttcttgctcgcaaacataacacttgctgtaacttatcacaccgtttctacaggttagctaacgagtgtgcgcaagtattaagtgagatggtcatgtgtggcggctcactatatgttaaaccaggtggaacatcatccggtgatgctacaactgcttatgctaatagtgtctttaacatttgtcaagctgttacagccaatgtaaatgcacttctttcaactgatggtaataagatagctgacaagtatgtccgcaatctacaacacaggctctatgagtgtctctatagaaatagggatgttgatcatgaattcgtggatgagttttacgcttacctgcgtaaacatttctccatgatgattctttctgatgatgccgttgtgtgctataacagtaactatgcggctcaaggtttagtagctagcattaagaactttaaggcagttctttattatcaaaataatgtgttcatgtctgaggcaaaatgttggactgagactgaccttactaaaggacctcacgaattttgctcacagcatacaatgctagttaaacaaggagatgattacgtgtacctgccttacccagatccatcaagaatattaggcgcaggctgttttgtcgatgatattgtcaaaacagatggtacacttatgattgaaaggttcgtgtcactggctattgatgcttacccacttacaaaacatcctaatcaggagtatgctgatgtctttcacttgtatttacaatacattagaaagttacatgatgagcttactggccacatgttggacatgtattccgtaatgctaactaatgataacacctcacggtactgggaacctgagttttatgaggctatgtacacaccacatacagtcttgcaggctgtaggtgcttgtgtattgtgcaattcacagacttcacttcgttgcggtgcctgtattaggaggccattcctatgttgcaagtgctgctatgaccatgtcatttcaacatcacacaaattagtgttgtctgttaatccctatgtttgcaatgccccaggttgtgatgtcactgatgtgacacaactgtatctaggaggtatgagctattattgcaagtcacataagcctcccattagttttccattatgtgctaatggtcaggtttttggtttatacaaaaacacatgtgtaggcagtgacaatgtcactgacttcaatgcgatagcaacatgtgattggactaatgctggcgattacatacttgccaacacttgtactgagagactcaagcttttcgcagcagaaacgctcaaagccactgaggaaacatttaagctgtcatatggtattgccactgtacgcgaagtactctctgacagagaattgcatctttcatgggaggttggaaaacctagaccaccattgaacagaaactatgtctttactggttaccgtgtaactaaaaatagtaaagtacagattggagagtacacctttgaaaaaggtgactatggtgatgctgttgtgtacagaggtactacgacatacaagttgaatgttggtgattactttgtgttgacatctcacactgtaatgccacttagtgcacctactctagtgccacaagagcactatgtgagaattactggcttgtacccaacactcaacatctcagatgagttttctagcaatgttgcaaattatcaaaaggtcggcatgcaaaagtactctacactccaaggaccacctggtactggtaagagtcattttgccatcggacttgctctctattacccatctgctcgcatagtgtatacggcatgctctcatgcagctgttgatgccctatgtgaaaaggcattaaaatatttgcccatagataaatgtagtagaatcatacctgcgcgtgcgcgcgtagagtgttttgataaattcaaagtgaattcaacactagaacagtatgttttctgcactgtaaatgcattgccagaaacaactgctgacattgtagtctttgatgaaatctctatggctactaattatgacttgagtgttgtcaatgctagacttcgtgcaaaacactacgtctatattggcgatcctgctcaattaccagccccccgcacattgctgactaaaggcacactagaaccagaatattttaattcagtgtgcagacttatgaaaacaataggtccagacatgttccttggaacttgtcgccgttgtcctgctgaaattgttgacactgtgagtgctttagtttatgacaataagctaaaagcacacaaggataagtcagctcaatgcttcaaaatgttctacaaaggtgttattacacatgatgtttcatctgcaatcaacagacctcaaataggcgttgtaagagaatttcttacacgcaatcctgcttggagaaaagctgtttttatctcaccttataattcacagaacgctgtagcttcaaaaatcttaggattgcctacgcagactgttgattcatcacagggttctgaatatgactatgtcatattcacacaaactactgaaacagcacactcttgtaatgtcaaccgcttcaatgtggctatcacaagggcaaaaattggcattttgtgcataatgtctgatagagatctttatgacaaactgcaatttacaagtctagaaataccacgtcgcaatgtggctacattacaagcagaaaatgtaactggactttttaaggactgtagtaagatcattactggtcttcatcctacacaggcacctacacacctcagcgttgatataaagttcaagactgaaggattatgtgttgacataccaggcataccaaaggacatgacctaccgtagactcatctctatgatgggtttcaaaatgaattaccaagtcaatggttaccctaatatgtttatcacccgcgaagaagctattcgtcacgttcgtgcgtggattggctttgatgtagagggctgtcatgcaactagagatgctgtgggtactaacctacctctccagctaggattttctacaggtgttaacttagtagctgtaccgactggttatgttgacactgaaaataacacagaattcaccagagttaatgcaaaacctccaccaggtgaccagtttaaacatcttataccactcatgtataaaggcttgccctggaatgtagtgcgtattaagatagtacaaatgctcagtgatacactgaaaggattgtcagacagagtcgtgttcgtcctttgggcgcatggctttgagcttacatcaatgaagtactttgtcaagattggacctgaaagaacgtgttgtctgtgtgacaaacgtgcaacttgcttttctacttcatcagatacttatgcctgctggaatcattctgtgggttttgactatgtctataacccatttatgattgatgttcagcagtggggctttacgggtaaccttcagagtaaccatgaccaacattgccaggtacatggaaatgcacatgtggctagttgtgatgctatcatgactagatgtttagcagtccatgagtgctttgttaagcgcgttgattggtctgttgaataccctattataggagatgaactgagggttaattctgcttgcagaaaagtacaacacatggttgtgaagtctgcattgcttgctgataagtttccagttcttcatgacattggaaatccaaaggctatcaagtgtgtgcctcaggctgaagtagaatggaagttctacgatgctcagccatgtagtgacaaagcttacaaaatagaggaactcttctattcttatgctacacatcacgataaattcactgatggtgtttgtttgttttggaattgtaacgttgatcgttacccagccaatgcaattgtgtgtaggtttgacacaagagtcttgtcaaacttgaacttaccaggctgtgatggtggtagtttgtatgtgaataagcatgcattccacactccagctttcgataaaagtgcatttactaatttaaagcaattgcctttcttttactattctgatagtccttgtgagtctcatggcaaacaagtagtgtcggatattgattatgttccactcaaatctgctacgtgtattacacgatgcaatttaggtggtgctgtttgcagacaccatgcaaatgagtaccgacagtacttggatgcatataatatgatgatttctgctggatttagcctatggatttacaaacaatttgatacttataacctgtggaatacatttaccaggttacagagtttagaaaatgtggcttataatgttgttaataaaggacactttgatggacacgccggcgaagcacctgtttccatcattaataatgctgtttacacaaaggtagatggtattgatgtggagatctttgaaaataagacaacacttcctgttaatgttgcatttgagctttgggctaagcgtaacattaaaccagtgccagagattaagatactcaataatttgggtgttgatatcgctgctaatactgtaatctgggactacaaaagagaagccccagcacatgtatctacaataggtgtctgcacaatgactgacattgccaagaaacctactgagagtgcttgttcttcacttactgtcttgtttgatggtagagtggaaggacaggtagacctttttagaaacgcccgtaatggtgttttaataacagaaggttcagtcaaaggtctaacaccttcaaagggaccagcacaagctagcgtcaatggagtcacattaattggagaatcagtaaaaacacagtttaactactttaagaaagtagacggcattattcaacagttgcctgaaacctactttactcagagcagagacttagaggattttaagcccagatcacaaatggaaactgactttctcgagctcgctatggatgaattcatacagcgatataagctcgagggctatgccttcgaacacatcgtttatggagatttcagtcatggacaacttggcggtcttcatttaatgataggcttagccaagcgctcacaagattcaccacttaaattagaggattttatccctatggacagcacagtgaaaaattacttcataacagatgcgcaaacaggttcatcaaaatgtgtgtgttctgtgattgatcttttacttgatgactttgtcgagataataaagtcacaagatttgtcagtgatttcaaaagtggtcaaggttacaattgactatgctgaaatttcattcatgctttggtgtaaggatggacatgttgaaaccttctacccaaaactacaagcaagtcaagcgtggcaaccaggtgttgcgatgcctaacttgtacaagatgcaaagaatgcttcttgaaaagtgtgaccttcagaattatggtgaaaatgctgttataccaaaaggaataatgatgaatgtcgcaaagtatactcaactgtgtcaatacttaaatacacttactttagctgtaccctacaacatgagagttattcactttggtgctggctctgataaaggagttgcaccaggtacagctgtgctcagacaatggttgccaactggcacactacttgtcgattcagatcttaatgacttcgtctccgacgcagattctactttaattggagactgtgcaacagtacatacggctaataaatgggaccttattattagcgatatgtatgaccctaggaccaaacatgtgacaaaagagaatgactctaaagaagggtttttcacttatctgtgtggatttataaagcaaaaactagccctgggtggttctatagctgtaaagataacagagcattcttggaatgctgacctttacaagcttatgggccatttctcatggtggacagcttttgttacaaatgtaaatgcatcatcatcggaagcatttttaattggggctaactatcttggcaagccgaaggaacaaattgatggctataccatgcatgctaactacattttctggaggaacacaaatcctatccagttgtcttcctattcactctttgacatgagcaaatttcctcttaaattaagaggaactgctgtaatgtctcttaaggagaatcaaatcaatgatatgatttattctcttctggaaaaaggtaggcttatcattagagaaaacaacagagttgtggtttcaagtgatattcttgttaacaactaaacgaacatgaactccttctccacaagcgccttcggtccagttgccttctccctgggcctgctcctggtgttgcctgctgccttccctgccccagtcttcacactcgaagatttcgttggggactggcgacagacagccggctacaacctggaccaagtccttgaacagggaggtgtgtccagtttgtttcagaatctcggggtgtccgtaactccgatccaaaggattgtcctgagcggtgaaaatgggctgaagatcgacatccatgtcatcatcccgtatgaaggtctgagcggcgaccaaatgggccagatcgaaaaaatttttaaggtggtgtaccctgtggatgatcatcactttaaggtgatcctgcactatggcacactggtaatcgacggggttacgccgaacatgatcgactatttcggacggccgtatgaaggcatcgccgtgttcgacggcaaaaagatcactgtaacagggaccctgtggaacggcaacaaaattatcgacgagcgcctgatcaaccccgacggctccctgctgttccgagtaaccatcaacggagtgaccggctggcggctgtgcgaacgcattctggcgtaaacgaactaactattattattattctgtttggaactttaacattgcttatcatgattgaacaagatggattgcacgcaggttctccggccgcttgggtggagaggctattcggctatgactgggcacaacagacaatcggctgctctgatgccgccgtgttccggctgtcagcgcaggggcgcccggttctttttgtcaagaccgacctgtccggtgccctgaatgaactgcaagacgaggcagcgcggctatcgtggctggccacgacgggcgttccttgcgcagctgtgctcgacgttgtcactgaagcgggaagggactggctgctattgggcgaagtgccggggcaggatctcctgtcatctcaccttgctcctgccgagaaagtatccatcatggctgatgcaatgcggcggctgcatacgcttgatccggctacctgcccattcgaccaccaagcgaaacatcgcatcgagcgagcacgtactcggatggaagccggtcttgtcgatcaggatgatctggacgaagagcatcaggggctcgcgccagccgaactgttcgccaggctcaaggcgagcatgcccgacggcgaggatctcgtcgtgacccatggcgatgcctgcttgccgaatatcatggtggaaaatggccgcttttctggattcatcgactgtggccggctgggtgtggcggaccgctatcaggacatagcgttggctacccgtgatattgctgaagagcttggcggcgaatgggctgaccgcttcctcgtgctttacggtatcgccgctcccgattcgcagcgcatcgccttctatcgccttcttgacgagttcttctgaaacatgcacacctaatgttactatcaactgtcaagatccagctggtggtgcgcttatagctaggtgttggtaccttcatgaaggtcaccaaactgctgcatttagagacgtacttgttgttttaaataaacgaacaaattaaaatgtctgataatggaccccaatcaaaccaacgtagtgccccccgcattacatttggtggacccacagattcaactgacaataaccagaatggaggacgcaatggggcaaggccaaaacagcgccgaccccaaggtttacccaataatactgcgtcttggttcacagctctcactcagcatggcaaggaggaacttagattccctcgaggccagggcgttccaatcaacaccaatagtggtccagatgaccaaattggctactaccgaagagctacccgacgagttcgtggtggtgacggcaaaatgaaagagctcagccccagatggtacttctattacctaggaactggcccagaagcttcacttccctacggcgctaacaaagaaggcatcgtatgggttgcaactgagggagccttgaatacacccaaagaccacattggcacccgcaatcctaataacaatgctgccaccgtgctacaacttcctcaaggaacaacattgccaaaaggcttctacgcagagggaagcagaggcggcagtcaagcctcttctcgctcctcatcacgtagtcgcggtaattcaagaaattcaactcctggcagcagtaggggaaattctcctgctcgaatggctagcggaggtggtgaaactgccctcgcgctattgctgctagacagattgaaccagcttgagagcaaagtttctggtaaaggccaacaacaacaaggccaaactgtcactaagaaatctgctgctgaggcatctaaaaagcctcgccaaaaacgtactgccacaaaacagtacaacgtcactcaagcatttgggagacgtggtccagaacaaacccaaggaaatttcggggaccaagacctaatcagacaaggaactgattacaaacattggccgcaaattgcacaatttgctccaagtgcctctgcattctttggaatgtcacgcattggcatggaagtcacaccttcgggaacatggctgacttatcatggagccattaaattggatgacaaagatccacaattcaaagacaacgtcatactgctgaacaagcacattgacgcatacaaaacattcccaccaacagagcctaaaaaggacaaaaagaaaaagactgatgaagctcagcctttgccgcagagacaaaagaagcagcccactgtgactcttcttcctgcggctgacatggatgatttctccagacaacttcaaaattccatgagtggagcttctgctgattcaactcaggcataaacactcatgatgaccacacaaggcagatgggctatgtaaacgttttcgcaattccgtttacgatacatagtctactcttgtgcagaatgaattctcgtaactaaacagcacaagtaggtttagttaactttaatctcacatagcaatctttaatcaatgtgtaacattagggaggacttgaaagagccaccacattttcatcgaggccacgcggagtacgatcgagggtacagtgaataatgctagggagagctgcctatatggaagagccctaatgtgtaaaattaattttagtagtgctatccccatgtgattttaatagcttcttaggagaatgacaaaaaaaaaaaaaaaaaaaaaaaaggccggcatggtcccagcctcctcgctggcgccggctgggcaacattccgaggggaccgtcccctcggtaatggcgaatgggacccactgtgccttctagttgccagccatctgttgtttgcccctcccccgtgccttccttgaccctggaaggtgccactcccactgtcctttcctaataaaatgaggaaattgcatcgcattgtctgagtaggtgtcattctattctggggggtggggtggggcaggacagcaagggggaggattgggaagacaatagcaggcatgctggggatgcggtgggctctatgg

SEQ ID NO: 18 - DNA, 25464 bp, synthetic construct
  source 1..25464: mol_type = other DNA
gttgacattgattattgactagttattaatagtaatcaattacggggtcattagttcatagcccatatatggagttccgcgttacataacttacggtaaatggcccgcctggctgaccgcccaacgacccccgcccattgacgtcaataatgacgtatgttcccatagtaacgccaatagggactttccattgacgtcaatgggtggagtatttacggtaaactgcccacttggcagtacatcaagtgtatcatatgccaagtacgccccctattgacgtcaatgacggtaaatggcccgcctggcattatgcccagtacatgaccttatgggactttcctacttggcagtacatctacgtattagtcatcgctattaccatggtgatgcggttttggcagtacatcaatgggcgtggataggggtttgactcacggggatttccaagtctccaccccattgacgtcaatgggagtttgttttggcaccaaaatcaacgggactttccaaaatgtcgtaacaactccgccccattgacgcaaatgggcggtaggcgtgtacggtgggaggtctatataagcagagctcgtttagtgaaccgatttaagtgaatagcttggctatctcacttcccctcgttctcttgcagaactttgattttaacgaacttaaataaaagccctgttgtttagcgtatcgttgcacttgtctggtgggattgtggcattaatttgcctgctcatctaggcagtggacatatgctcaacactgggtataattctaattgaatactatttttcagttagagcgtcgtgtctcttgtacgtctcggtcacaatacacggtttcgtccggtgcgtggcaattcggggcacatcatgtctttcgtggctggtgtgaccgcgcaaggtgcgcgcggtacgtatcgagcagcgctcaactctgaaaaacatcaagaccatgtgtctctaactgtgccactctgtggttcaggaaacctggttgaaaaactttcaccatggttcatggatggcgaaaatgcctatgaagtggtgaaggccatgttacttaaaaaggagccacttctctatgtgcccatccggctggctggacacactagacacctcccaggtcctcgtgtgtacctggttgagaggctcattgcttgtgaaaatccattcatggttaaccaattggcttatagctctagtgcaaatggcagcctggttggcacaactttgcagggcaagcctattggtatgttcttcccttatgacatcgaacttgtcacaggaaagcaaaatattctcctgcgcaagtatggccgtggtggttatcactacaccccattccactatgagcgagacaacacctcttgccctgagtggatggacgattttgaggcggatcctaaaggcaaatatgcccagaatctgcttaagaagttgattggcggtgatgtcactccagttgaccaatacatgtgtggcgttgatggaaaacccattagtgcctacgcatttttaatggccaaggatggaataaccaaactggctgatgttgaagcggacgtcgcagcacgtgctgatgacgaaggcttcatcacattaaagaacaatctatatagattggtttggcatgttgagcgtaaagacgttccatatcctaagcaatctatttttactattaatagtgtggtccaaaaggatggtgttgaaaacactcctcctcactattttactcttggatgcaaaattttaacgctcaccccacgcaacaagtggagtggcgtttctgacttgtccctcaaacaaaaactcctttacaccttctatggtaaggagtcacttgagaacccaacctacatttaccactccgcattcattgagtgtggaagttgtggtaatgattcctggcttacagggaatgctatccaagggtttgcctgtggatgtggggcatcatatacagctaatgatgtcgaagtccaatcatctggcatgattaagccaaatgctcttctttgtgctacttgcccctttgctaagggtgatagctgttcttctaattgcaaacattcagttgctcagttggttagttacctttctgaacgctgtaatgttattgctgattctaagtccttcacacttatctttggtggcgtagcttacgcctactttggatgtgaggaaggtactatgtactttgtgcctagagctaagtctgttgtctcaaggattggagactccatctttacaggctgtactggctcttggaacaaggtcactcaaattgctaacatgttcttggaacagactcagcattcccttaactttgtgggagagttcgttgtcaacgatgttgtcctcgcaattctctctggaaccacaactaatgttgacaaaatacgccagcttctcaaaggtgtcacccttgacaagttgcgtgattatttagctgactatgacgtagcagtcactgccggcccattcatggataatgctattaatgttggtggtacaggattacagtatgccgccattactgcaccttatgtagttctcactggcttaggtgagtcctttaagaaagttgcaaccataccgtataaggtttgcaactctgttaaggatactctggcttattatgctcacagcgtgttgtacagagtttttccttatgacatggattctggtgtgtcatcctttagtgaactactttttgattgcgttgatctttcagtagcttctacctattttttagtccgcatcttgcaagataagactggcgactttatgtctacaattattacttcctgccaaactgctgttagtaagcttctagatacatgttttgaagctacagaagcaacatttaacttcttgttagatttggcaggattgttcagaatctttctccgcaatgcctatgtgtacacttcacaagggtttgtggtggtcaatggcaaagtttctacacttgtcaaacaagtgttagacttgcttaataagggtatgcaacttttgcatacaaaggtgtcctgggctggttctaaaatcattgctgttatctacagcggcagggagtctctaatattcccatcgggaacctattactgtgtcaccactaaggctaagtccgttcaacaagatcttgacgttattttgcctggtgagttttccaagaagcagttaggactgctccaacctactgacaattctacaactgttagtgttactgtatccagtaacatggttgaaactgttgtgggtcaacttgagcaaactaatatgcatagtcctgatgttatagtaggtgactatgtcattattagtgaaaaattgtttgtgcgtagtaaggaagaagacggatttgccttctaccctgcttgcactaatggtcatgctgtaccgactctctttagacttaagggaggtgcacctgtaaaaaaagtagcctttggcggtgatcaagtacatgaggttgctgctgtaagaagtgttactgtcgagtacaacattcatgctgtattagacacactacttgcttcttctagtcttagaacctttgttgtagataagtctttgtcaattgaggagtttgctgacgtagtaaaggaacaagtctcagacttgcttgttaaattactgcgtggaatgccgattccagattttgatttagacgattttattgacgcaccatgctattgctttaacgctgagggtgatgcatcctggtcttctactatgatcttctctcttcaccccgtcgagtgtgacgaggagtgttctgaagtagaggcttcagatttagaagaaggtgaatcagagtgcatttctgagacttcaactgaacaagttgacgtttctcatgagacttctgacgacgagtgggctgctgcagttgatgaagcgttccctctcgatgaagcagaagatgttactgaatctgtgcaagaagaagcacaaccagtagaagtacctgttgaagatattgcgcaggttgtcatagctgacaccttacaggaaactcctgttgtgcctgatactgttgaagtcccaccgcaagtggtgaaacttccgtctgcacctcagactatccagcccgaggtaaaagaagttgcacctgtctatgaggctgataccgaacagacacagaatgttactgttaaacctaagaggttacgcaaaaagcgtaatgttgaccctttgtccaattttgaacataaggttattacagagtgcgttaccatagttttaggtgacgcaattcaagtagccaagtgctatggggagtctgtgttagttaatgctgctaacacacatcttaagcatggcggtggtatcgctggtgctattaatgcggcttcaaaaggggctgtccaaaaagagtcagatgagtatattctggctaaagggccgttacaagtaggagattcagttctcttgcaaggccattctctagctaagaatatcctgcatgtcgtaggcccagatgcccgcgctaaacaggatgtttctctccttagtaagtgctataaggctatgaatgcatatcctcttgtagtcactcctcttgtttcagcaggcatatttggtgtaaaaccagctgtgtcttttgattatcttattagggaggctaagactagagttttagtcgtcgttaattcccaagatgtctataagagtcttaccatagttgacattccacagagtttgactttttcatatgatgggttacgtggcgcaatacgtaaagctaaagattatggttttactgtttttgtgtgcacagacaactctgctaacactaaagttcttaggaacaagggtgttgattatactaagaagtttcttacagttgacggtgtgcaatattattgctacacgtctaaggacactttagatgatatcttacaacaggctaataagtctgttggtattatatctatgcctttgggatatgtgtctcatggtttagacttaatgcaagcagggagtgtcgtgcgtagagttaacgtgccctacgtgtgtctcctagctaataaagagcaagaagctattttgatgtctgaagacgttaagttaaacccttcagaagattttataaagcacgtccgcactaatggtggttacaattcttggcatttagtcgagggtgaactattggtgcaagacttacgcttaaataagctcctgcattggtctgatcaaaccatatgctacaaggatagtgtgttttatgttgtaaagaatagtacagcttttccatttgaaacactttcagcatgtcgtgcgtatttggattcacgcacgacacagcagttaacaatcgaagtcttagtgactgtcgatggtgtaaattttagaacagtcgttctaaataataagaacacttatagatcacagcttggatgcgttttctttaatggtgctgatatttctgacaccattcctgatgagaaacagaatggtcacagtttatatctagcagacaatttgactgctgatgaaacaaaggcgcttaaagagttatatggccccgttgatcctactttcttacacagattctattcacttaaggctgcagtccatgggtggaagatggttgtgtgtgataaggtacgttctctcaaattgagtgataataattgttatcttaatgcagttattatgacacttgatttattgaaggacattaaatttgttatacctgctctacagcatgcatttatgaaacataagggcggtgattcaactgacttcatagccctcattatggcttatggcaattgcacatttggtgctccagatgatgcctctcggttacttcataccgtgcttgcaaaggctgagttatgctgttctgcacgcatggtttggagagagtggtgcaatgtctgtggcataaaagatgttgttctacaaggcttaaaagcttgttgttacgtgggtgtgcaaactgttgaagatctgcgtgctcgcatgacatatgtatgccagtgtggtggtgaacgtcatcggcaattagtcgaacacaccaccccctggttgctgctctcaggcacaccaaatgaaaaattggtgacaacctccacggcgcctgattttgtagcatttaatgtctttcagggcattgaaacggctgttggccattatgttcatgctcgcctgaagggtggtcttattttaaagtttgactctggcaccgttagcaagacttcagactggaagtgcaaggtgacagatgtacttttccccggccaaaaatacagtagcgattgtaatgtcgtacggtattctttggacggtaatttcagaacagaggttgatcccgacctatctgctttctatgttaaggatggtaaatactttacaagtgaaccacccgtaacatattcaccagctacaattttagctggtagtgtctacactaatagctgccttgtatcgtctgatggacaacctggcggtgatgctattagtttgagttttaataaccttttagggtttgattctagtaaaccagtcactaagaaatacacttactccttcttgcctaaagaagacggcgatgtgttgttggctgagtttgacacttatgaccctatttataagaatggtgccatgtataaaggcaaaccaattctttgggtcaataaagcatcttatgatactaatcttaataagttcaatagagctagtttgcgtcaaatttttgacgtagcccccattgaactcgaaaataaattcacacctttgagtgtggagtctacaccagttgaacctccaactgtagatgtggtagcacttcaacaggaaatgacaattgtcaaatgtaagggtttaaataaacctttcgtgaaggacaatgtcagtttcgttgctgatgattcaggtactcccgttgttgagtatctgtctaaagaagacctacatacattgtatgtagaccctaagtatcaagtcattgtcttaaaagacaatgtactttcttctatgcttagattgcacaccgttgagtcaggtgatattaacgttgttgcagcttccggatctttgacacgtaaagtgaagttactatttagggcttcattttatttcaaagaatttgctacccgcactttcactgctaccactgctgtaggtagttgtataaagagtgtagtgcggcatctaggtgttactaaaggcatattgacaggctgttttagttttgccaagatgttatttatgcttccactagcttactttagtgattcaaaactcggcaccacagaggttaaagtgagtgctttgaaaacagccggcgttgtgacaggtaatgttgtaaaacagtgttgcactgctgctgttgatttaagtatggataagttgcgccgtgtggattggaaatcaaccctacggttgttacttatgttatgcacaactatggtattgttgtcttctgtgtatcacttgtatgtcttcaatcaggtcttatcaagtgatgttatgtttgaagatgcccaaggtttgaaaaagttctacaaagaagttagagcttacctaggaatctcttctgcttgtgacggtcttgcttcagcttatagggcgaattcctttgatgtacctacattctgcgcaaaccgttctgcaatgtgtaattggtgcttgattagccaagattccataactcactacccagctcttaagatggttcaaacacatcttagccactatgttcttaacatagattggttgtggtttgcatttgagactggtttggcatacatgctctatacctcggccttcaactggttgttgttggcaggtacattgcattatttctttgcacagacttccatatttgtagactggcggtcatacaattatgctgtgtctagtgccttctggttattcacccacattccaatggcgggtttggtacgaatgtataatttgttagcatgcctttggcttttacgcaagttttatcagcatgtaatcaatggttgcaaagatacggcatgcttgctctgctataagaggaaccgacttactagagttgaagcttctaccgttgtctgtggtggaaaacgtacgttttatatcacagcaaatggcggtatttcattctgtcgtaggcataattggaattgtgtggattgtgacactgcaggtgtggggaataccttcatctgtgaagaagtcgcaaatgacctcactaccgccctacgcaggcctattaacgctacggatagatcacattattatgtggattccgttacagttaaagagactgttgttcagtttaattatcgtagagacggtcaaccattctacgagcggtttcccctctgcgcttttacaaatctagataagttgaagttcaaagaggtctgtaaaactactactggtatacctgaatacaactttatcatctacgactcatcagatcgtggccaggaaagtttagctaggtctgcatgtgtttattattctcaagtcttgtgtaaatcaattcttttggttgactcaagtttggttacttctgttggtgattctagtgaaatcgccactaaaatgtttgattcctttgttaatagtttcgtctcgctgtataatgtcacacgcgataagttggaaaaacttatctctactgctcgtgatggcgtaaggcgaggcgataacttccatagtgtcttaacaacattcattgacgcagcacgaggccccgcaggtgtggagtctgatgttgagacgaatgaaattgttgactctgtgcagtatgctcataaacatgacatacaaattactaatgagagctacaataattatgtaccctcatatgttaaacctgatagtgtgtctaccagcgatttaggtagtctcattgattgtaatgcggcttcagttaaccaaattgtcttgcgtaattctaatggtgcttgcatttggaacgctgctgcatatatgaaactctcggatgcacttaaacgacagattcgcattgcatgccgtaagtgtaatttagctttccggttaaccacctcaaagctacgcgctaatgataatatcttatcagttagattcactgctaacaaaattgttggtggtgctcctacatggtttaatgcgttgcgtgactttacgttaaagggttatgttcttgctaccattattgtgtttctgtgtgctgtactgatgtatttgtgtttacctacattttctatggcacctgttgaattttatgaagaccgcatcttggactttaaagttcttgataatggtatcattagggatgtaaatcctgatgataagtgctttgctaataagcaccggtccttcacacaatggtatcatgagcatgttggtggtgtctatgacaactctatcacatgcccattgacagttgcagtaattgctggagttgctggtgctcgcattccagacgtacctactacattggcttgggtgaacaatcagataattttctttgtttctcgagtctttgctaatacaggcagtgtttgctacactcctatagatgagataccctataagagtttctctgatagtggttgcattcttccatctgagtgcactatgtttagggatgcagagggccgtatgacaccatactgccatgatcctactgttttgcctggggcttttgcgtacagtcagatgaggcctcatgttcgttacgacttgtatgatggtaacatgtttattaaatttcctgaagtagtatttgaaagtacacttaggattactagaactctgtcaactcagtactgccggttcggtagttgtgagtatgcacaagagggtgtttgtattaccacaaatggctcgtgggccatttttaatgaccaccatcttaatagacctggtgtctattgtggctctgattttattgacattgtcaggcggttagcagtatcactgttccagcctattacttatttccaattgactacctcattggtcttgggtataggtttgtgtgcgttcctgactttgctcttctattatattaataaagtaaaacgtgcttttgcagattacacccagtgtgctgtaattgctgttgttgctgctgttcttaatagcttgtgcatctgctttgttacctctataccattgtgtatagtaccttacactgcattgtactattatgctacattctattttactaatgagcctgcatttattatgcatgtttcttggtacattatgttcgggcctatcgttcccatatggatgacctgcgtctatacagttgcaatgtgctttagacacttcttctgggttttagcttattttagtaagaaacatgtagaagtttttactgatggtaagcttaattgtagtttccaggacgctgcctctaatatctttgttattaacaaggacacttatgcagctcttagaaactctttaactaatgatgcctattcacgatttttggggttgtttaacaagtataagtacttctctggtgctatggaaacagccgcttatcgtgaagctgcagcatgtcatcttgctaaagccttacaaacatacagcgagactggtagtgatcttctttaccaaccacccaactgtagcataacctctggcgtgttgcaaagcggtttggtgaaaatgtcacatcccagtggagatgttgaggcttgtatggttcaggttacctgcggtagcatgactcttaatggtctttggcttgacaacacagtctggtgcccacgacacgtaatgtgcccggctgaccagttgtctgatcctaattatgatgccttgttgatttctatgactaatcatagtttcagtgtgcaaaaacacattggcgctccagcaaacttgcgtgttgttggtcatgccatgcaaggcactcttttgaagttgactgtcgatgttgctaaccctagcactccagcctacacttttacaacagtgaaacctggcgcagcatttagtgtgttagcatgctataatggtcgtccgactggtacattcactgttgtaatgcgccctaactacacaattaagggttcctttctgtgtggttcttgtggtagtgttggttacaccaaggagggtagtgtgatcaatttctgttacatgcatcaaatggaacttgctaatggtacacataccggttcagcatttgatggtactatgtatggtgcctttatggataaacaagtgcaccaagttcagttaacagacaaatactgcagtgttaatgtagtagcttggctttacgcagcaatacttaatggttgcgcttggtttgtaaaacctaatcgcactagtgttgtttcttttaatgaatgggctcttgccaaccaattcactgaatttgttggcactcaatccgttgacatgttagctgtcaaaacaggcgttgctattgaacagctgctttatgcgatccaacaactgtatactgggttccagggaaagcaaatccttggcagtaccatgttggaagatgaattcacacctgaggatgttaatatgcagattatgggtgtggttatgcagagtggtgtgagaaaagttacatatggtactgcgcattggttgtttgcgacccttgtctcaacctatgtgataatcttacaagccactaaatttactttgtggaactacttgtttgagactattcccacacagttgttcccactcttatttgtgactatggccttcgttatgttgttggttaaacacaaacacacctttttgacacttttcttgttgcctgtggctatttgtttgacttatgcaaacatagtctacgagcccactactcccatttcgtcagcgctgattgcagttgcaaattggcttgcccccactaatgcttatatgcgcactacacatactgatattggtgtctacattagtatgtcacttgtattagtcattgtagtgaagagattgtacaacccatcactttctaactttgcgttagcattgtgcagtggtgtaatgtggttgtacacttatagcattggagaagcctcaagccccattgcctatctggtttttgtcactacactcactagtgattatacgattacagtctttgttactgtcaaccttgcaaaagtttgcacttatgccatctttgcttactcaccacagcttacacttgtgtttccggaagtgaagatgatacttttattatacacatgtttaggtttcatgtgtacttgctattttggtgtcttctctcttttgaaccttaagcttagagcacctatgggtgtctatgactttaaggtgtcaacacaagagttcagattcatgactgctaacaatctaactgcacctagaaattcttgggaggctatggctctgaactttaagttaataggtattggcggtacaccttgtataaaggttgctgctatgcagtctaaacttacagatcttaaatgcacatctgtggttctcctctctgtgctccaacagttacacttagaggctaatagtagggcctgggctttctgtgttaaatgccataatgatatattggcagcaacagaccccagtgaggctttcgagaaattcgtaagtctctttgctactttaatgactttttctggtaatgtagatcttgatgcgttagctagtgatatttttgacactcctagcgtacttcaagctactctttctgagttttcacacttagctacctttgctgagttggaagctgcgcagaaagcctatcaggaagctatggactctggtgacacctcaccacaagttcttaaggctttgcagaaggctgttaatatagctaaaaacgcctatgagaaggataaggcagtggcccgtaagttagaacgtatggctgatcaggctatgacttctatgtataagcaagcacgtgctgaagacaagaaagcaaaaattgtcagtgctatgcaaactatgttgtttggtatgattaagaagctcgacaacgatgttcttaatggtatcatttctaacgctaggaatggttgtatacctcttagtgtcatcccactgtgtgcttcaaataaacttcgcgttgtaattcctgacttcaccgtctggaatcaggtagtcacatatccctcgcttaactacgctggggctttgtgggacattacagttataaacaatgtggacaatgaaattgttaagtcttcagatgttgtagacagcaatgaaaatttaacatggccacttgttttagaatgcactagggcatccacttctgccgttaagttgcaaaataatgagatcaaaccttcaggtctaaaaaccatggttgtgtctgcgggtcaagagcaaactaactgtaatactagttccttagcttattacgaacctgtgcagggtcgtaaaatgctgatggctcttctttctgataatgcctatctcaaatgggcgcgtgttgaaggtaaggacggatttgtcagtgtagagctacaacctccttgcaaattcttgattgcgggaccaaaaggacctgaaatccgatatctctattttgttaaaaatcttaacaaccttcatcgcgggcaagtgttagggcacattgctgcgactgttagattgcaagctggttctaacaccgagtttgcctctaattcctcggtgttgtcacttgttaacttcaccgttgatcctcaaaaagcttatctcgatttcgtcaatgcgggaggtgccccattgacaaattgtgttaagatgcttactcctaaaactggtacaggtatagctatatctgttaaaccagagagtacagctgatcaagagacttatggtggagcttcagtgtgtctctattgccgtgcgcatatagaacatcctgatgtctctggtgtttgtaaatataagggtaagtttgtccaaatccctgctcagtgtgtccgtgaccctgtgggattttgtttgtcaaataccccctgtaatgtctgtcaatattggattggatatgggtgcaattgtgactcgcttaggcaagcagcactgccccaatctaaagattccaattttttaaacgagtccggggttctattgtaaatgcccgaatagaaccctgttcaagtggtttgtccactgatgtcgtctttagggcatttgacatctgcaactataaggctaaggttgctggtattggaaaatactacaagactaatacttgtaggtttgtagaattagatgaccaagggcatcatttagactcctattttgtcgttaagaggcatactatggagaattatgaactagagaagcactgttacgacttgttacgtgactgtgatgctgtagctccccatgatttcttcatctttgatgtagacaaagttaaaacacctcatattgtacgtcagcgtttaactgagtacactatgatggatcttgtatatgccctgaggcactttgatcaaaatagcgaagtgcttaaggctatcttagtgaagtatggttgctgtgatgttacctactttgaaaataaactctggtttgattttgttgaaaatcccagtgttattggtgtttatcataaacttggagaacgtgtacgccaagctatcttaaacactgttaaattttgtgaccacatggtcaaggctggtttagtcggtgtgctcacactagacaaccaggaccttaatggcaagtggtatgattttggtgacttcgtaatcactcaacctggttcaggagtagctatagttgatagctactattcttatttgatgcctgtgctctcaatgaccgattgtctggccgctgagacacatagggattgtgattttaataaaccactcattgagtggccacttactgagtatgattttactgattataaggtacaactctttgagaagtactttaaatattgggatcagacgtatcacgcaaattgcgttaattgtactgatgaccgttgtgtgttacattgtgctaatttcaatgtattgtttgctatgaccatgcctaagacttgtttcggacccatagtccgaaagatctttgttgatggcgtgccatttgtagtatcttgtggttatcactacaaagaattaggtttagtcatgaatatggatgttagtctccatagacataggctctctcttaaggagttgatgatgtatgccgctgatccagccatgcacattgcctcctctaacgcttttcttgatttgaggacatcatgttttagtgtcgctgcacttacaactggtttgacttttcaaactgtgcggcctggcaattttaaccaagacttctatgatttcgtggtatctaaaggtttctttaaggagggctcttcagtgacgctcaaacattttttctttgctcaagatggtaatgctgctattacagattataattactattcttataatctgcctactatgtgtgacatcaaacaaatgttgttctgcatggaagttgtaaacaagtacttcgaaatctatgacggtggttgtcttaatgcttctgaagtggttgttaataatttagacaagagtgctggccatccttttaataagtttggcaaagctcgtgtctattatgagagcatgtcttaccaggagcaagatgaactttttgccatgacaaagcgtaacgtcattcctaccatgactcaaatgaatctaaaatatgctattagtgctaagaatagagctcgcactgttgcaggcgtgtccatacttagcacaatgactaatcgccagtaccatcagaaaatgcttaagtccatggctgcaactcgtggagcgacttgcgtcattggtactacaaagttctacggtggctgggatttcatgcttaaaacattgtacaaagatgttgataatccgcatcttatgggttgggattaccctaagtgtgatagagctatgcctaatatgtgtagaatcttcgcttcactcatattagctcgtaaacatggcacttgttgtactacaagggacagattttatcgcttggcaaatgagtgtgctcaggtgctaagcgaatatgttctatgtggtggtggttactacgtcaaacctggaggtaccagtagcggagatgccaccactgcatatgccaatagtgtctttaacattttgcaggcgacaactgctaatgtcagtgcacttatgggtgctaatggcaacaagattgttgacaaagaagttaaagacatgcagtttgatttgtatgtcaatgtttacaggagcactagcccagaccccaaatttgttgataaatactatgcttttcttaataagcacttttctatgatgatactgtctgatgacggtgtcgtttgctataatagtgattatgcagctaagggttacattgctggaatacagaattttaaggaaacgctgtattatcagaacaatgtctttatgtctgaagctaaatgctgggtggaaaccgatctgaagaaagggccacatgaattctgttcacagcatacgctttatattaaggatggcgacgatggttacttccttccttatccagacccttcaagaattttgtctgccggttgctttgtagatgatatcgttaagactgacggtacactcatggtagagcggtttgtgtctttggctatagatgcttaccctctcacaaagcatgaagatatagaataccagaatgtattctgggtctacttacagtatatagaaaaactgtataaagaccttacaggacacatgcttgacagttattctgtcatgctatgtggtgataattctgctaagttttgggaagaggcattctatagagatctctatagttcgcctaccactttgcaggctgtcggttcatgcgttgtatgccattcacagacttccctacgctgtgggacatgcatccgtagaccatttctctgctgtaaatgctgctatgatcatgttatagcaactccacataagatggttttgtctgtttctccttacgtttgtaatgcccctggttgtggcgtttcagacgttactaagctatatttaggtggtatgagctacttttgtgtagatcatagacctgtgtgtagttttccactttgcgctaatggtcttgtattcggcttatacaagaatatgtgcacaggtagtccttctatagttgaatttaataggttggctacctgtgactggactgaaagtggtgattacacccttgccaatactacaacagaaccactcaaactttttgctgctgagactttacgtgccactgaagaggcgtctaagcagtcttatgctattgccaccatcaaagaaattgttggtgagcgccaactattacttgtgtgggaggctggcaagtccaaaccaccactcaatcgtaattatgtttttactggttatcatataaccaaaaatagtaaagtgcagctcggtgagtacattttcgagcgcattgattatagtgatgctgtatcctacaagtctagtacaacgtataaactgactgtaggtgacatcttcgtacttacctctcactctgtggctaccttgacggcgcccacaattgtgaatcaagagaggtatgttaaaattactgggttgtacccaaccattacggtacctgaagagttcgcaagtcatgttgccaacttccaaaaatcaggttatagtaaatatgtcactgttcagggaccacctggcactggcaaaagtcattttgctatagggttagcgatttactaccctacagcacgtgttgtttatacagcatgttcacacgcagctgttgatgctttgtgtgaaaaagcttttaaatatttgaacattgctaaatgttcccgtatcattcctgcaaaggcacgtgttgagtgctatgacaggtttaaagttaatgagacaaattctcaatatttgtttagtactattaatgctctaccagaaacttctgccgatattctggtggttgatgaggttagtatgtgcactaattatgatctttcaattattaatgcacgtattaaagctaagcacattgtctatgtaggagatccagcacagttgccagctcctaggactttgttgactagaggcacattggaaccagaaaatttcaatagtgtcactagattgatgtgtaacttaggtcctgacatatttttaagtatgtgctacaggtgtcctaaggaaatagtaagcactgtgagcgctcttgtctacaataataaattgttagccaagaaggagctttcaggccagtgctttaaaatactctataagggcaatgtgacgcatgatgctagctctgccattaatagaccacaactcacatttgtgaagaattttattactgccaatccggcatggagtaaggcagtctttatttcgccttacaattcacagaatgctgtgtctcgttcaatgctgggtcttaccactcagactgttgattcctcacagggttcagaataccagtacgttatcttctgtcaaacagcagatacggcacatgctaacaacattaacagatttaatgttgcaatcactcgtgcccaaaaaggtattctttgtgttatgacatctcaggcactctttgagtccttagagtttactgaattgtcttttactaattacaagctccagtctcagattgtaactggcctttttaaagattgctctagagaaacttctggcctctcacctgcttatgcaccaacatatgttagtgttgatgacaagtataagacgagtgatgagctttgcgtgaatcttaatttacccgcaaatgtcccatactctcgtgttatttccaggatgggctttaaactcgatgcaacagttcctggatatcctaagcttttcattactcgtgaagaggctgtaaggcaagttcgaagctggataggcttcgatgttgagggtgctcatgcttcccgtaatgcatgtggcaccaatgtgcctctacaattaggattttcaactggtgtgaactttgttgttcagccagttggtgttgtagacactgagtggggtaacatgttaacgggcattgctgcacgtcctccaccaggtgaacagtttaagcacctcgtgcctcttatgcataagggggctgcgtggcctattgttagacgacgtatagtgcaaatgttgtcagacactttagacaaattgtctgattactgtacgtttgtttgttgggctcatggctttgaattaacgtctgcatcatacttttgcaagataggtaaggaacagaagtgttgcatgtgcaatagacgcgctgcagcgtactcttcacctctgcaatcttatgcctgctggactcattcctgcggttatgattatgtctacaaccctttctttgtcgatgttcaacagtggggttatgtaggcaatcttgctactaatcacgatcgttattgctctgtccatcaaggagctcatgtggcttctaatgatgcaataatgactcgttgtttagctattcattcttgttttatagaacgtgtggattgggatatagagtatccttatatctcacatgaaaagaaattgaattcctgttgtagaatcgttgagcgcaacgtcgtacgtgctgctcttcttgccggttcatttgacaaagtctatgatattggcaatcctaaaggaattcctattgttgatgaccctgtggttgattggcattattttgatgcacagcccttgaccaggaaggtacaacagcttttctatacagaggacatggcctcaagatttgctgatgggctctgcttattttggaactgtaatgtaccaaaatatcctaataatgcaattgtatgcaggtttgacacacgtgtgcattctgagttcaatttgccaggttgtgatggcggtagtttgtatgttaacaagcacgcttttcatacaccagcatatgatgtgagtgcattccgtgatctgaaacctttaccattcttttattattctactacaccatgtgaagtgcatggtaatggtagtatgatagaggatattgattatgtacccctaaaatctgcagtctgtattacagcttgtaatttagggggcgctgtttgtaggaagcatgctacagagtacagagagtatatggaagcatataatcttgtctctgcatcaggtttccgcctttggtgttataagacctttgatatttataatctctggtctacttttacaaaagttcaaggtttggaaaacattgcttttaatgttgttaaacaaggccattttattggtgttgagggtgaactacctgtagctgtagtcaatgataagatcttcaccaagagtggcgttaatgacatttgtatgtttgagaataaaaccactttgcctactaatatagcttttgaactctatgctaagcgtgctgtacgctcgcatcccgatttcaaattgctacacaatttacaagcagacatttgctacaagttcgtcctttgggattatgaacgtagcaatatttatggtactgctactattggtgtatgtaagtacactgatattgatgttaattcagctttgaatatatgttttgacatacgcgataattgttcattggagaagttcatgtctactcccaatgccatctttatttctgatagaaaaatcaagaaatacccttgtatggtaggtcctgattatgcttacttcaatggtgctatcatccgtgatagtgatgttgttaaacaaccagtgaagttctacttgtataagaaagtcaataatgagtttattgatcctactgagtgtatttacactcagagtcgctcttgtagtgacttcctacccctttctgacatggagaaagactttctatcttttgatagtgatgttttcattaagaagtatggcttggaaaactatgcttttgagcacgtagtctatggagacttctctcatactacgttaggcggtcttcacttgcttattggtttatacaagaagcaacaggaaggtcatattattatggaagaaatgctaaaaggtagctcaactattcataactattttattactgagactaacacagcggcttttaaggcggtgtgttctgttatagatttaaagcttgacgactttgttatgattttaaagagtcaagaccttggcgtagtatccaaggttgtcaaggttcctattgacttaacaatgattgagtttatgttatggtgtaaggatggacaggttcaaaccttctaccctcgactccaggcttctgcagattggaaacctggtcatgcaatgccatccctctttaaagttcaaaatgtaaaccttgaacgttgtgagcttgctaattacaagcaatctattcctatgcctcgcggtgtgcacatgaacatcgctaaatatatgcaattgtgccagtatttaaatacttgcacattagccgtgcctgccaatatgcgtgttatacattttggcgctggttctgataaaggtatcgctcctggtacctcagttttacgacagtggcttcctacagatgccattattatagataatgatttaaatgagttcgtgtcagatgctgacataactttatttggagattgtgtaactgtacgtgtcggccaacaagtggatcttgttatttccgacatgtatgatcctactactaagaatgtaacaggtagtaatgagtcaaaggctttattctttacttacctgtgtaacctcattaataataatcttgctcttggtgggtctgttgctattaaaataacagaacactcttggagcgttgaactttatgaacttatgggaaaatttgcttggtggactgttttctgcaccaatgcaaatgcatcctcatctgaaggattcctcttaggtattaattacttgggtactattaaagaaaatatagatggtggtgctatgcacgccaactatatattttggagaaattccactcctatgaatctgagtacttactcactttttgatttatccaagtttcaattaaaattaaaaggaacaccagttcttcaattaaaggagagtcaaattaacgaactcgtaatatctctcctgtcgcagggtaagttacttatccgtgacaatgatacactcagtgtttctactgatgttcttgttaacacctacagaaagttacgttgaatgaactccttctccacaagcgccttcggtccagttgccttctccctgggcctgctcctggtgttgcctgctgccttccctgccccagtcttcacactcgaagatttcgttggggactggcgacagacagccggctacaacctggaccaagtccttgaacagggaggtgtgtccagtttgtttcagaatctcggggtgtccgtaactccgatccaaaggattgtcctgagcggtgaaaatgggctgaagatcgacatccatgtcatcatcccgtatgaaggtctgagcggcgaccaaatgggccagatcgaaaaaatttttaaggtggtgtaccctgtggatgatcatcactttaaggtgatcctgcactatggcacactggtaatcgacggggttacgccgaacatgatcgactatttcggacggccgtatgaaggcatcgccgtgttcgacggcaaaaagatcactgtaacagggaccctgtggaacggcaacaaaattatcgacgagcgcctgatcaaccccgacggctccctgctgttccgagtaaccatcaacggagtgaccggctggcggctgtgcgaacgcattctggcgtaaaacgaactccttcataatgattgaacaagatggattgcacgcaggttctccggccgcttgggtggagaggctattcggctatgactgggcacaacagacaatcggctgctctgatgccgccgtgttccggctgtcagcgcaggggcgcccggttctttttgtcaagaccgacctgtccggtgccctgaatgaactgcaagacgaggcagcgcggctatcgtggctggccacgacgggcgttccttgcgcagctgtgctcgacgttgtcactgaagcgggaagggactggctgctattgggcgaagtgccggggcaggatctcctgtcatctcaccttgctcctgccgagaaagtatccatcatggctgatgcaatgcggcggctgcatacgcttgatccggctacctgcccattcgaccaccaagcgaaacatcgcatcgagcgagcacgtactcggatggaagccggtcttgtcgatcaggatgatctggacgaagagcatcaggggctcgcgccagccgaactgttcgccaggctcaaggcgagcatgcccgacggcgaggatctcgtcgtgacccatggcgatgcctgcttgccgaatatcatggtggaaaatggccgcttttctggattcatcgactgtggccggctgggtgtggcggaccgctatcaggacatagcgttggctacccgtgatattgctgaagagcttggcggcgaatgggctgaccgcttcctcgtgctttacggtatcgccgctcccgattcgcagcgcatcgccttctatcgccttcttgacgagttcttctgagctctttagtaagagtatcttaattgattttaacgaatctcaatttcattgttatggcatcccctgctgcacctcgtgctgtttcctttgccgataacaatgatataacaaatacaaacctatctcgaggtagaggacgtaatccaaaaccacgagctgcaccaaataacactgtctcttggtacactgggcttacccaacacgggaaagtccctcttacctttccacctgggcagggtgtacctcttaatgccaattctacccctgcgcaaaatgctgggtattggcggagacaggacagaaaaattaataccgggaatggaattaagcaactggctcccaggtggtacttctactacactggaactggacccgaagcagcactcccattccgggctgttaaggatggcatcgtttgggtccatgaagatggcgccactgatgctccttcaacttttgggacgcggaaccctaacaatgattcagctattgttacacaattcgcgcccggtactaagcttcctaaaaacttccacattgaggggactggaggcaatagtcaatcatcttcaagagcctctagcttaagcagaaactcttccagatctagttcacaaggttcaagatcaggaaactctacccgcggcacttctccaggtccatctggaatcggagcagtaggaggtgatctactttaccttgatcttctgaacagactacaagcccttgagtctggcaaagtaaagcaatcgcagccaaaagtaatcactaagaaagatgctgctgctgctaaaaataagatgcgccacaagcgcacttccaccaaaagtttcaacatggtgcaagcttttggtcttcgcggaccaggtgacctccagggaaactttggtgatcttcaattgaataaactcggcactgaggacccacgttggccccaaattgctgagcttgctcctacagccagtgcttttatgggtatgtcgcaatttaaacttacccatcagaacaatgatgatcatggcaaccctgtgtacttccttcggtacagtggagccattaaacttgacccaaagaatcccaactacaataagtggttggagcttcttgagcaaaatattgatgcctacaaaaccttccctaagaaggaaaagaaacaaaaggcaccaaaagaagaatcaacagaccaaatgtctgaacctccaaaggagcagcgtgtgcaaggtagcatcactcagcgcactcgcacccgtccaagtgttcagcctggtccaatgattgatgttaacactgattagtgtcactcaaagtaacaagatcgcggcaatcgtttgtgtttggcaaccccatctcaccatcgcttgtccactcttgcacagaatggaatcatgttgtaattacagtgcaataaggtaattataacccatttaattgatagctatgctttattaaagtgtgtagctgtagagagaatgttaaagactgtcacctctgcttgattgcaagtgaacagtgccccccgggaagagctctacagtgtgaaatgtaaataaaaaatagctattattcaattagattaggctaattagatgatttgcaaaaaaaaaaaaaaaaaaaaaaaaaaaaaaaaggccggcatggtcccagcctcctcgctggcgccggctgggcaacattccgaggggaccgtcccctcggtaatggcgaatgggacccactgtgccttctagttgccagccatctgttgtttgcccctcccccgtgccttccttgaccctggaaggtgccactcccactgtcctttcctaataaaatgaggaaattgcatcgcattgtctgagtaggtgtcattctattctggggggtggggtggggcaggacagcaagggggaggattgggaagacaatagcaggcatgctggggatgcggtgggctctatgg

SEQ ID NO: 19 - DNA, 26216 bp, synthetic construct
  source 1..26216: mol_type = other DNA
gttgacattgattattgactagttattaatagtaatcaattacggggtcattagttcatagcccatatatggagttccgcgttacataacttacggtaaatggcccgcctggctgaccgcccaacgacccccgcccattgacgtcaataatgacgtatgttcccatagtaacgccaatagggactttccattgacgtcaatgggtggagtatttacggtaaactgcccacttggcagtacatcaagtgtatcatatgccaagtacgccccctattgacgtcaatgacggtaaatggcccgcctggcattatgcccagtacatgaccttatgggactttcctacttggcagtacatctacgtattagtcatcgctattaccatggtgatgcggttttggcagtacatcaatgggcgtggataggggtttgactcacggggatttccaagtctccaccccattgacgtcaatgggagtttgttttggcaccaaaatcaacgggactttccaaaatgtcgtaacaactccgccccattgacgcaaatgggcggtaggcgtgtacggtgggaggtctatataagcagagctcgtttagtgaaccttaagcttcggcttgttgcataggaccggaaaggtactatctaccctaactcttgtagttagactctctaaacgaactttaaaactggttgtgtccttcagtagtctgtatggccattggaggcacaccggtaattatcaaatactaagaagattcatagtacatccttgtctagcttttggttggcagtgagcctacggtttcgtccgtgtcgctcacaattatccacacagtaggtttcgtccgctgtggttgagttgctagtccgttgctgtttcgtcagccatctacaactcgacaccatgtgtagcaaggggtatgaactgaatcagaaaactcacttttctgtggaactgccatggatccaaattggtgagaatcctatcaaaccttggtcggttacaccggctgaggccttgaacactgtatatgctgccattgctgaaggcaaggctgcatttatcccaccattcaaggggatgcataagtatctccctgaattgtgtgtctttctagtgagaaaccatgggaacccaacacgcccttttgacctgcaagaacttgctgtccgcgaaggtgacgtgaactatggtcgctcaggtgaaacagtaggcgcaattgtaccgcttgatggacaggagccctacggaactataacaatccaactccgcagacgcgggaaaaatgcgggtggagtctatgcctggactaacacccgtgatacggttacagatgatttggttcatgaaccaatcgatctgtatactgaagatcctaaagggaaacatgcccagggaaacctgcgcaaattccttactggcggtaacgatttccatcgttacgtcgataactactattgcactggagacgggaaaccgctgccatgcatagtgactttgctcgagaaggctggccatgccaataagcctctcgacgacgctatggactatctccgaggcttgaaccgtatgggacaaccttgtagagatcatgaccatgagcgtgtttgggaagtggagcgcgataatgctccttatcctgaacaatctctcttctcaatcagtgctatcaagaccttgggtgaaataccccactgtgtctttgcacctgattgtgccgtcaaagtaatgaaacctcgcaaggtcaaacgcggggctgacggctttatgacgaaactcagaagagtgtacaatatcaatggctttgatgaagtcaagccaatggcgctctgtgcactccattactgtgaggattgtggcatggaaatgtggtgtcactcaaattttgaggaagcctactgtccatgtggtaaaatttacaccaacacaccttgcacactaacttcagctggttatgttgttgaaggttcagttgttgctatgccgtgcgatgcatgtaagagcgatagcgaccattctaatgggaccttctatgacagctgtaagtatcttgctgaagacaaagcagaacctggtaatagggaaaactttgtctattttggaggatgttgctttgcctatgttggctgccgcaatggtaatgccatctgggtacccagagcacattcagatattggtaacaatcactcaggcattgttggagctgatgttgctttgcttaatgatgacctcaaggccattgttgctcaagaggttatacctgttgtgatccctgaagactttaaggtcaatgagactgtggttgctcttgtagcagcagtttcaggttcagtggaccagttcattaagaactgtaaaggactgacagctgaaaccttcaagtgtttgcttgaagcttctggcaaattcagagtcactgttgatcatgttattgacggttgtatttgtgttgctacagatagcgccgttacggcccttgaaccagcattggctttttgtactgctgccaatatcatgtaccgcacccttgtggctacatctgttgtcatcagtgctcatactttagatgctttggctcaacgtgtgcgtgatgcttgtaaacacgtgcaccctcaggctatgcgtcttcttaatactcttaatgagtatgtggattacagcactaactccacacttgtactgtgccatgacgtcattaatttgccaattgtgcttggtgatatcctggacagacttttctgtggatgcaaaaagattgtcgagtctgtcacaacatggctctacaactttagcatctctactattgacacaatatttgaccttaaggcttttattagtcttattgtacgtaataagtacaagtttgtcaagggtaagtttgtgttacttgctaaaaatgtcagttctgtagtgcaatctgttgttgcctacctaaacaatgttatctcagctttttaccaacaagtgcagtttgctggcacctacgtaggagcctttgaaattcatcaaacgttacttgagctgggtggtgctatctacacgcgtgtgcaggttgcagcaaacagtattcaagaccttgttttgccttctacagtgtccaaaaaggaattaacctttgtggatggacatgctattgacacagaattgacttctgaagaagttactgtgttggaaggtatagttgaacaacttgacactgataccaataagattgctggtgacagtatcaagggtgatttagtcacggtgaataattgtgttttcgtacgctttggcgatggaaacctttcaccggctactactgactgtcaagccacaaaaggagtttttaaactcaaaggtggcaaccctgacaaggttaaaaccgtgaccttcggtgaaaacgaggtcaaggaaatcactccatatattacagtgaatgtgaagtacaccgttcatgaccttcttgataagattctcaatgtgcggcttccatcatttactgttgaaaagggcttaacgctccaagaacttactgcagttgttgaagacgcagttgtcacacaattggaagctatgcgtgctatcctacttgaagcgggtgtcgacattgatattgacgatcttattgactcgccatattatatgtttgacaacgcaggtgactctgttattggacctgtgatgtacttttccaaccaacagcccgttgactcagatgagttgacaacggcatcagagactgaagaagtagtcgaagatgctaaacatgctgcaactaaacgttcaagtcaagattggcttgacgatagttgttctgaagacgattgtgaagaggaagacgcagtcactgaagctgaaagcgctgctgatagtgcaccagcgttggttgtggttatagaggaacctaagtctactgtttcgtcagttagcgaggaaccaaagtttcccttacctgaacagtgttctgttgaaacccacatagtcgtggatgacacaaatagcaaacgcctcttatggtcggacatggttgaagcaacttgtgggtctgccactgatggaaacgaaggaactgtgggtgaggttgacacgtgtgcggtagctgtaaatcgtgacaacactccatcaacgcagtccatcgtaaccgtttctccacagagagaagtgcatcactatgtcgtaactgaagagaagtgggacgaacacgtgtgcggtagctgtaaaccgtgtgaaatccccttgagcgtaaaagctaagcgtgtgaaccaaaattctgtaaattgtggtgaaaaggctgtcgttacagttaactccactacagttttcaacacgcctgttccacgtgaagtggaagccaaaacggcgaatgaacaacctaaggttgatagtactactgtagctaaagtcactcgtacaaagagtgggcacagtcaggaattcaaacccaaaggttacaccaagcttaccgacaatgtgtacattaagtgtgccgacattgttgaggaagctcgcaatacaaaaccacctattcttgtaaatgcagcgaattgcaaactcaagcatggtggtggtgtggcaggtgcgataaggaaggccgtaggaaactccattcaggaggattctgacctttacattaaagaaaatggtgctatacccgttggaggggcagcattactaccaggttataacttggctactaatatcctacatgtagtaggacctaatattacaatgaatgaggattcctcactcatcgttaatgcttactcaaacttgaatagttttagtactgttgtaacaccactgttatcagctggtatatttggtatgaagcctattgatagtcttactgccttactttctacatgtaagaagacagtctatgttgttgtcaacgacaagactattttcgatgcatgttgtagccacattaataacaaggatgtcaaaacaccatctaagcctgtttacatgatgggcgaagtagaagtgttttgtagtactaaagttgcatattgcaaccaggataaagaattttgtcctggtacatctaccttatttaaacctgagcagcttgatgagattagacttaagttgccagaagactttctgattggagattgccacaaagtggatgatgtctacgttttgtgcatacctgaccgtagaaagggacaagaccttacaggttttaagggtcttaaacaattaaagaaagtcactgccgcttcatgtctaccaggacagggaaaatttggctttactatacaggatgtgacgccacttatgacggcatgtcctgatatttaccttgtcaaaactagtgttgacaatgatgttcaattgttgtgtccgacagtgacatacaatgttaaacaaatgttggcacgcgctaagcaagaaaaattgcttatgtgtgtcaatattgacaacaagtcttttaccaggaacgttgttcatttggcaaaaaattttcaacacaaaccaggctgtcaaactgtggacggctatgagttttactgttacactgagaaacaaccattgagttctatcattgatgaacttaatgcgttgggcaaggacatcataacaacgccattaggttgtattacacaccaattatccttaccagagtcagcagcaaaaatgcgtgctctgaagtgcaaatttctcgcagtgtgtacttcgccaggtgctgaaaagcaattctgtgctgcattcacagctgcctctagctctacagaagaagagttatttatggcagattgtgtttctaacggttcctacatggattggatcgttataaacaaagccgatggtgacacaattcatttccttcagagggatgaagacatcatcgattatcacacaagcactaacaagttcagtatgagtggtgttagtgggcttgtgtttaaagatgtgaagatactcaagcggtatctcgaaaaaactaagcctatgctgaaagaggttaccgtctatacaactgtagacggtactaatgttaacaccaagattttgatttgttctaaatcttttggcagccagctaggcacatgttacattgatggagaggacgttacaagtgtcttccctacaaaacaacatgaaggtaagattgtcaacataactcaagttgacgatgttactagtagtcaggttaaagaatactatggtgttgaagacactagtttcctgactcgttataactcagccttgatgcatgtcaatcgctggtcgtttgcagaagtacctagtacaggtattttctgcattaaatgggtggctaacaattgctatcttaatgctgcgatactcatgctacagcagctcaatgtcgaatacgagacacctgctgtgcgtgaagcggcttttgaaatgcgtgctggcaaacctcaacggtttgtggcactcatgattgcttacttaaaggctaccattggtcacactggtgatgctagagaagcagttagaactatgctttcacatgccaaagtgcaaggtgaaaggcattttgttatgatgtgcaaaaagtgtgggattagacgtagtcagtttcacggtcttgatgcagtcatgtgtttcacaaccaacacacaactaagtgatttccttagtggtgacgaagctggttgcacttgtggtgatattgtgcctgtgtatcagacacatatcagagtaccctttttgattctttcaaccacagagcccaaaatgcaaatgcttaactgtgaagacactaagtttctttgcgctaataattacatgggcaccttaagtagtggacactacacccatgttttcaacaagacactcttgtacagtgtaaacggtacacgagtaacaaaaatgtcagaaacaacaacagctgttgctgacgctgtgtataaagacataaaatatgacactgaagaccaattcgtcacatacagactggatggtgtttggtgtcatgaaaagaatccagacttgagcgtgtattacaaatcaggttctgattattacacatcagcacctatagacttgactcctacagagccattgtctggtgctgaatacgacaatttccatcttaaacttgttgggacacttgatgacaacaaagttaagtttgtgcaagagtttaatcacatggtcaaatatgacaaaaccaagcctacgaggcctgttactatatctttctatcctgagatggaaggtgatgttgtagcactatctgcggataagttgcaacaacattttaagaagggggcaaaatttggttccaaatttatagtttggcacacaggttacaaaatcactagagatcttgtcaagccaaacatggcagctatgcgctgtataaccacctctaaacctgtgactacacaaaactcgtttcaagctctttctgttgaacctcttccagagacaaaacatagcgagcatgaattagccacagaacaaaaaccaatcctgaaactcaggacagagaaaccagttgttacggctgcagtgacaataattcctgctcccaaaaacgctgatgctcctgttttaattgaatccttgactactgatgatgcgctagctatgtatgtcaagggtactcgagattttgttgttaataaggctaacagcctgtctaagctgtttggtattaacacaattgaacagaatggtgtcgatgcgctaaatatgtgctacgacaggctagctgtctttgactatgtcaaaccatttttaacagttactaaaactgctagtgatgtgacaatcaaagcaggaaaagtagcatgctcactattgcaaagaacagtaccactgttatatgctttagtagtgtcttatttagtacccttgttcacaagaacaaaacaacgtgtgtcagttaaagtccctatggtcttaactaaaaacacatgcagaagtgtctttggtttattgatgaatggagttgctaattacttcacgtcacccaaattcaagtcttgtgtaagagtctttgcattggcaacatgcatagcagcgattctatatatggctatgtttgtatatttgttctttgacatatggctatcaaaagctaacgtgtggacagatgtgcaaacactgaaagataattttggtcttggaacggtttgtgataaattccagacagcttataataactctggtatttatgatgccaccgagtattgtactggtaagagttttatgtgtagtctgtgtctgcgtggcatggatagtctcaacttttacacagaattgtctacatcccaaaagacggtttcatggtcttcttttgattttagtaacattaacactgcggctgaatggtgtttggcgtatttgctttacactaagatgtttgtggttttgttggcgactgcaatcttccaatggtttgctgtctattttggcctctacctcacacaatctagttggttgatgtggactatggttagagtcatcagtcttgttcctacgagcattcttgttcgtatgtatatttattgtgcatccttttactttgtctacagagcttatgttcacgtcgttagtggctgtcaagatacacgttgtctgatgtgctacaagcgtaacttagctcgcagagtggaatgtcatacagttgtccagggttctcgcaaatcattttatgtgcacgctaatggcggtactggattttgtgaaaaacatgcctggaattgtatcaactgtgattcttatggacctggtaacactttcatctgtgacgaagttgctgttgatttgtctaccacttttaagcgacctgttaagcctaccgacaagtctcattattttgtggattctgtagaggttaaagacacctttgtacacctttactactcaaaaaatgacacacgtgtttacgacagatatccattgtctgtgttctctagtgtggatttccttaaacttgctaacatcaaaactatgccatctaccaatgtgcttgtttttgatgctagtaataaaactgaagaaaacactactgtcgcagctagtgtatactactctcaactatgttgccaacctatgctgttgatcgaacagaaactattgtccaacataggtgatgctacagaagtgtcgaagaagatgcttgatgcttatattgaaaaattcatgagcacgttcggtgtcaccatggaaaaacttaaaacatttgtcagcgcagctaaaaatagtctgaatgacggtgtgcctcttgaaaaagtacttaaagagtttgttgcagcagctaaacaaaattgtgctgagactgatgtcgaagctgactctattgttaatgcactgcaactcacttttaaggatgatgttgacatcacaaaagattcttacaatgactttgtacttacttataacaaagttgattctatgactccatacgacttaggtgtgtgtattgaggttggtgctagacatgtcaatgcaaatgtagcaaaagcaaatgcggctgcactcatttggaacattgaccactacttactgctttccgagtcttttagacgccagattcgttcttcggcgcgtaaaaatggtttgcagtttaaactgacgtgtagcaagaatagacaagttacaccttttcttactacaaaaattatgtttagcggtggtgcaacgtatacaacatggctaaaaaggttattaaaggttgcaatggttatgctgcttgtttgctgcatactctattgtttgcttccatcatttaagtctcaaccactgaatatgtatagtgacgagattatcgacttcaaagttattgaagatgggtctttgcgtgacataactgcagatgacacttgtttttcaaacaagcatagtagttttgtgtcatggctgtctcgtaatggtttcaaaatgacaaccacttcaagacattgtcccattactgtagctgtagtggctaagaaagttggtgatgttataccgagcctaccaggcgtggttacacgtgttctagttcgtggccaaattatgcacttcctagcacgtgtctttagtgcagcagctaacatctgttacacacctggtaccttgattgaatacgaagactttctcacaagcgcatgtgtgctccctgcagaatgtactatctttaaggattctaatggcattgcagtgccttactgttacgatgttaatgcactgcaaggatcactaccatattctagcttgaagcatgatgtgctttaccagctggtggataattctttcatcaagttccctaaagttctcgttgaaggtgcgtttcgtattgtgcgtacaatgacaacacaatattgtagacatggagtttgcgaagactctatggctggactatgcctgtctcttcgtggctcatgggttttgaacaacccatattacacatcgcaaagcggagtctattgcggtaatgatgttgtggatcttctgatgaacatcctagcgcctatgtttagaccggctggtggtatggatataacctcatccatagtagcaggtggtatactatctcttgttattacagtcgtggcctactacatactcaagttgcgtagagcttttggagattaccaacaggtggttgtagtcaatacactagcttttctgtgttccttcctcgtgctctgcgtatccacacagtatcctgtattgccaactgtttattctatcttgtacttctacatgtctctttacatggctaatgaagtttctttcattatgcactgctcgtggtgtgtgatgtttgtaccaatagtacccttttggtgtacagctgtgtatataacaatgacatgctctaagcatgtgtactggtttttccagacattttgcaagaaaaatgttgttgtacatgatgctacatttagcagttttgctgaggccgcattatccacattcatgatcacaagagatgtgtatgtgaaattacgtgctgaagcttttctctctgctgcacaatacaataggtatttgtccatgttcaacagatataagtacttcagtggttctatggatactgaatcttatagagaagctgcttgttgtcatctcgctaaggccatgaaagacttcagtgagcaagggtctgatattctttatcaaccacccagttgttcactggcatctgctgttttacagtccggtattagaaagatgtcttgtcctacaggcaaagtagaacgttgcatggtgcgcgtaacttgtggtactatgacacttaatggcttgtggctggacaatactgtctactgccctcgccatgtcatgtgtacaccagaagaactacttgcccctgattatgacagtatccttttgcgtaaggctactcatagttttactgttcaatatggaacagcatatcttaaagtagtgtcctacaaaatgacaggatcagtacttcagttgggtgttgaccaaattaaccctgaaaccccaaaatataagtttgtaagggctaagcctggcgctacattctccgttttggcttgttacaatggtatgcctgctggtgtatatcaagttgcaatgaggccaaaccatactatcaaaggtagctttttgaacggctcatgtggtagtgttggttatactctaggttatgatagagtagaattttgctatatgcatcacatggaactacctacaggtgtacacactggtacagacctggaaggtactttctatggtgattttgttgaccggcaaacgtcgcagtcagctggttcagataatacacttacgctcaatgtgttggcttggctctatgcagctgtcatcaacggagaacgttggtttattgttccacaaacttgtgctttaacagacttcaatacagccgtcttgaagtacgggtatcaaagtcttactgaagacggtgttgcagcattagacccactggtggcccagacaggaatctcagttcagactatgtgtgcatcacttaaagatttgcttgttcatggtatgagaggcagatgtatactgagctcgcccacactcgaggatgagttcacaccctttgacattgtacgccaatgttctggtgttactttgcaaagtactgttagaagtgtttcttctaaattctttcagtggatgctaatgacagcacttacttttactatactatttttacaactgtgggaaatgtccatttttagttggtttgctatgcatgctactattccagttgtaatcctacttatgggtgtgtctgcttttgtgactatgttagtcaaacacaagcatgcctttacaacactgttcctgatgccaacattggctgttgtcttttattataattgtatttatgtacctgagcattggctcattgaaatggtcagcaagtatgttgacttgactgatacaattcagctgttctacggctattctataagagaacttatcgctctttttgctgtggtcatagctatgagtgtcctgtctctgcgtattgtctatgacgacaatactagacgagtatggcttgctactaatgtgctcacatggttgtacaggttgtacgctggcacaacagtagagaaggctatggcttactgggcactccttatgagtctcaccacaaattatagtggttgtgttacagttataatgtttgctgctaaaggtgtcacaacattaatttactaccaatttccttttctaggattgcttattgcagaattcaaattccttatgttagtgtatacttgcattggatatttgtgctgcgtttattatggcatcttttgtatgttgaacaaatacttacgttgcacttttggtgtgtatccatacctggtttccacacaggagttcagatatatgaattcacaaggcttaactccccctaccaacagctgggatgctctgaaaatgaacatcaaattgtcaggtgttggtggtgtgccatgcattaaggtttctaatgtgcaatctaagatgtctgacatcaaatgcacgtctgtggtgttgttatcagttttgcaacaactccggattgaagccaattcaagaatctggtcactgtgtgtcacacttcacaatgacattttgctggctaaagatgctacagaggcttttgaaaagcttacaacgttgttgtctgtattgctatctatgccaggtgctgttgaccttactaagttgtgtgatgatgtctttgagaacccagcaattttgcaggcggtttcaaatgaatttaataatctgcccacgtttgttgaatacgagtgtgcacagaaagcttatgatgaggctttagcaaatggtgaaggacctattgtcctgaagcagttgaaaaaggcagttaattgtgccaaatctgcatttgaaagagatgcagctgtggcaagaaagttagagcgtatggcagaccttgccatgacacaaatgtacaaagaagcgcgtgctgaagataaacgtgctcgcgtcacatctgctatgcaatctatgttattcagcatgcttcgtcgtcttgacaatgatgctttgaataatataatcactaatgctagagatggctgtgtaccattgaatgtgatacccatgttagcctctagcaaactgcttattgtcgtacctgacattagtgtttataacaacacagtggaaggaacactcttaacttatgctggcgccgtgtgggacgtagtccaagttaccgacgctgacaacaaacctattgccatgggtgatatcacgatagatacagcacctacattggcttggcctttagtactttcagctgtaagacgtgtttcagcaacaaagttacaaaataatgagttggcacctcagcttttgaatcaaaaagctgttactggaggttctgaacaaaacatatgcgaccaaccagcgttagcatattataacacagtccaaggcaaacatgtcattttggcagttgtcagtgatcatgacggattacgttggactcgtgttgataaatctgatggtaatggtattgttatgattgaacttgaccctccatgcagatttataacgcaaacatcaagtggtcccaaagtgaagtacttgtacttcatcaaaggactaaacaacttatgtcgtggcatggtactaggtactgtagctgcgactgttagattgcaagctggcaaaccaactgaagtggctgccaactctaaatgcttgacattttgtgcctttgctgtagatcctgaaaaggcatactttgacttcgtgaacagcggaggccaaccgcttaataattgtgtgcgtgttttatgcactcacactggtacaggtcgtgctataactgcagatccagaggctacagcagatcaagaatcatatggtggttcttcttgttgcctctactgtagatgtcacatttcccacccaagtcataacgggttgtgtaagtataaaggcaaatatgtgcaaataccaaatgtatgcactaatgatccagtagggtttttgcttaaaaacactgtttgcaatgtatgcgcttgttggatagggtatggttgcaattgtgacacactccgccagccagtgcttcatgctgcagatgacagttttttaaacgggtgcgcggtgtaagtgcagcccgtcttacaccgtgtggcagtggtctttccactgacgtcgtcgtaagggctttcgacctgtacaatagtaaaataggaggctttggtcttcgttataagggcaattgctgccgatttcaagaaatcgacgaagacggcaaagccttagactcttttttcattgtcaagagacatactgaagacaactttaagctagaacaggaaatgtatgatttgctgaaggacagtggtgttgtggcagtccacgacttctttcactttagagtggagggacgaatggagcctcacatcacgcgtcagcgacttacaaagtacactatggctgatcttgtttacgcttttagacacttcgatgaaaatagttgtgaagtgctaaaagaaattcttgttacatataattgttgtggctcggattatttcgagaagaaagattggtatgactatgtagagaatcctgatatacttaatgtgtatgcccgtcttggtgagcgcattaggtgtaatttacttaagactgtaaagttctgtgatgccatgaaaagacatggtattgtgggagttttgacgctagacaaccaagaccttaatggtaattggtgtgattttggtgactttgtacgcggctttcctgggaatggagtacctgtcgtggactcatactactcattgcttatgcctttaatgacaatgactaaaatgcttgaggcagagacacatgtagattgtgacctgactaaggatcatgtgaagtgggacttgctccagtatgattatacagagcatagactcaacttgcaccaaaagtactttaagtactgggatatgccataccatcccaattgtcagagttgtcctgatgaccgttgtattttgcattgtgcaaatttcaatgtgttatacagtacaactataccacaaacatcatttggaccaatcgtcaaacgcatttatgtggatggcgttccatttgttgtctctgctggttaccattataaagagcttggcgttgtcatgaatcaagatattcatgtacacaacgctaggctatctcttagagaattgctagtctatgcagctgaccctgccatgcatgccgcatctggtactctgttgctagacaaaagaaccacatgttttagtgtggcatctcttaccaacacagttagcttccaaacagtgaagccaggcaattttaataaggacttctacgactttgctgtgtctaaaggtttctttaaggaaggtagttccgtggaccttaaacacttcttctttgcacaggatggtaatgctgctataactgattacagttattacaggtacaaccttcctactatgtgcgatataaaacagcttctgttcactatggaagtggtagataaatatttcgactgctatgatggtggttgcttaaacgccaatcaagttgttgtaaattcattagataagtcagccggtttcccatttaacaaatggggtaaggctagactttactatgaatctctgagttatgaagatcaggatgcactctttgcgtatacaaagaggaatgtgcttccaacaataactcaaatgaatttgaaatatgctattagcgctaagaatagagcccgcactgtagctggggtgtctatatgtagcactatgactaatcgtcaattccatcagaagatgcttaagtctatagctgctacacgtaatgtgtccgttgtcattggaactacaaagttctatggtggatggaataacatgctcaaaacactttatgcagatgtggataatgcacaactaatgggttgggattatcctaagtgtgacagagctatgcctaatatgttgcgtattttcgcttcattgattttagccagaaagcacaacacgtgttgtaatgtaagtgaaagatactacagactggctaatgagtgcgctcaagtattgagtgagatggttctatgtggtggtgctttgtatgtgaaaccaggtggtacttcctccggtgacgcaaccactgcatatgcaaattctgttttcaatatctgtcaagcagtaacggccaacattagtgccttgctagcagctaatggaaacaagatagtcgatgtttacattcgagacttacagcgtaaactgtatgcgaatgtttatcgtagtgtccatgttgattataagttcgtagatgagtactacgcctttttgcgtaaacacttttctatgatgatactgtctgacgatggtgtcgtatgttacaatagtgactacgtagctagaggctatattgctggaataaaagacttcaagcaagttctttattaccagaataatgtttttatgtcggaagccaagtgttgggtggaaccagacctgactaaaggcccacatgaattttgttcacaacacactatgctagttgagcataatggtgaacaagtgtatctaccttaccccgacccctcaagaattttaggggcttgttgttttgtagatgatgttgtcaaaactgacgggactatcatgattgagcgtttcgtcgccttggctattgatgcttatcctcttaccaaacatgagaaccctgagtataagcaggtcttttacttgttgttacaatacatcaagaaacttcatgaagagttaacgggccatttgttggacatgtactctgttatgatttcgggtgacaatgctcagagatactgggaagaagatttctatgaagcaatgtacactcaatcagtcactttacaggctgtcggcgcgtgtgtgttgtgtaattcacaaacatctttgcgttgcggtgactgtattagacgtccatttttgtgttgcaaatgttgttatgatcacgtcctttcaacgccacacaaactggtcttgtctgtatcaccttacgtctgtaatgcaccgggttgcgaagttacagatgttacacaactctacctcggaggtatgagttatttttgcaagtcccataaaccacctattagtttcccattgtgtgctaatggtcaggtgttcggactttataaaaatacatgtgtcggtagcattaatgtcgcagactttaacgctattgccacatgtgattggagtagtagtggtgattatgttttagctaacaccacaactgagcgtctgaaactgtttgctgcagagacgcttaaagctgtcgaagagactgctaaacaatcatatggtgttgctgttgtacgagaagtcgtcagcgacaaagaagttattttacggtgggaagctgacaaaccgcgtccgcctctaaaccgaaattacgtgtttactggttataggataactaaaaacagtaaaacacaaattggcgaatacacctttgagaagtcagattatggcgactcagtgttgtataaagcctctactacttataagttacaggtgggagactactttgtgttgacctctcactctgtcctgcctctttctgcacctacattgttgccgcaagagacatatacacgaattgtagggctctatcctacgttcaacattcctgacgattatgctggtaatgttgtaaattaccagaaaatcggaatggctaagtacaccacggttcaaggtccacctggcacaggtaaaagtcacctcgccattggtgtagcagtttattatcctacagcacgcatagtctacactgcttgtagtcatgctgctgttgatgccttatgtgaaaaggcattcagaacattgcctatttctaaatgctcacgcatagtgcccgcaaaggcccgcgtagagtgttttgataaattcaaagtcaatgatggtacagcacaatatgtgtttagcaccatcaatgccttaccagaaacctcaactgatgtactcgttgtggatgaagtcagcatgtgtactaattatgatcttagcataattaatgcgcgtgttcgagcaaagcatattgtgtatgtgggagatccagctcaattgccagcgccacgtacattacttacaagaggctcactagaaccagaaaatttcaattctgtgtgccgtcttatgaaaacattaggtcctgacatattcttaggagtatgtcgtcgttgtcctaaggaaattgtagacactgtttcagagctagtttatgaaaacaagcttaaggcacataagccagaatctggacagtgtttcaaaatgttttacaagggtactgttacccatgatgtatcaagcgccattaatagaccacaagtcggcgtcgtgagagagtttctaagccgcaatccccagtggaagaaggctgtgtttatttcaccatataatagccaaaatgcagtggctagtaagattctgggtttacagacccaaactgtggactcatcacaaggttcagagtatgattatgtgattttcgcccagactacagatactgcacactcttgcaatgttaataggtttaatgttgctatcacaagagctaagaagggtatactctgcatcatgtcggatcctgacatgttcgaacggttaaagttcgtagagctggctgtcccttctcgtagtcagataaggcttcaggcaactgaaattactggcttgtttaaggattgcagcaaactcattacgggtttgagtcctgcaatggcaccaacatatatggccgtagatgataaattcaagactaatggtggtctttgcgtgcatctacccggcatagaaaaagaagttagctatagacgcttgatttccatgatggggttcaagcttgactatagcgttcaagactacccgcgcttgtttatcacccgggatgaggcgattaaacaagttagagcgtgggtaggtttcgatgttgaaggtgctcatgctacaaaagatgcagttggtactaatgtaccacttcagttaggtttctcaaccggcatcaattttgtagcaacacctaccggttttgttgatactgagactggcacagaatgttgccgtatcttcgcgaaaccgccaccaggagagcaattcaagcatttaataccactaatgcaccgtgggatgccatggaatatagtgcgtgctagaattgtacagatgatgagtgacactcttaaaggtgttactgatagagtagtactggtaacttgggctcacggctttgagcttacaagtatgcagtacttctgtaaattaggtcgcgagcgcacatgttgtatgtgtgctgagcgtgcaacttgttactcctcagtgcatgacaattttggatgttggcatcactgtacaggttttgattatttgtacaacccctttattgtagatgtacagcaatggggttattcaggaaatttgcagagcaatcatgacaatcattgttctgtccattcaggagcacatgtggctagtagcgatgctattatgaccagatgtctcgccatttatgattgcttcgtaaaagaagtacactgggacattgagtatcctttcattgccgatgaagaattcatcaacaagtcatgtagaaaagtccaaaatatggtcgcaagagctgcattgctaggtgacaaatttggtaccatacatgatatcggcaatccaaaagcactcaagtgtgtccttgatgcagaggtgaattggaaattttatgatgctaaacccgttgctggaagagcacataaggttgaaactctctactaccagtatgaggtccataaagaccagtttcaggatggtgtttgcatgttctggaactgtaatgtggaccattatcctaaaaactccatcgtttgtcgctttgacactaggagtctttcaaaattaaatttaccaggttgtgatggaggtagtttatacgtaaataaacatgctttccacacgcctgcatttcaaaagtctgcatttactgatcttcagcaattgccattctttttctactcggatactgagtgtgatagtacaggacaacaagttgttgctgatattaattatgttccacttaaatccaatgtgtgcattactaggtgcaacctcggtggtgcggtgtgtaagaaacatgccaatgaataccgagagtacttgacttgttataatgctgtcattgaagcaggttttagtctttggatatacaagtggttcaacatttacaacttgtggagtactttcacaaagttgcaaggtttggaaaatgtagcatacaatgttgtcaataaaggtcattttgatggcacacagggtgaaatccctactgccgtgattggcgacaaagtatttgtaaaacgtgaaggcgtggatgtttgtgtgtttactaacaacaccacattgcctactaacgttgcatttgagctttacgcgaagcgtaatgtaaatccagttcctgaagtgaaattactccgtaacataggtgttgacatatgtaacggattcacactttgggactatgagcaacaagctccagtgtttaacagcactataggagtctgtaaatatacagacatcgctgctaagttctcagaaaagaattgtaaaccacttacaatactattcgatgcgaggcttagtggtcatattgatcaattctgcaatgcagataatgctgtcttgtacagcgattaccctattaagcgtttacaaggttctaagggacctgagcactgttctattaatggtgtcattgtaaactctacaccagatggcggggaaaaacctgccataaattgtacattctacttttacaagcgtgaaaatggtcagcttgtgaatgtaggaaatagttattttacacaaagccgtgttaagagctcttttgaaccccgtaccactatggagcgtgacttcttagagctcgacatgcatggatttattcaacgctacaatcttgaaaaatatgcttttgagcacattgtttatggtgactttagtcacaaacagatcggtggtttacatcttcttatcggcttgataaaacgctgcaatgagagtaccattgatattgaagagttcctcactatggactctactattcacaattactttgtaacagaccaaaataccggttcaagcaaagctgtatgttctgtaattgacttgctccttgacgatttcgttgaaataatcaagagccaagacttaactgtagtctctaaagtagtcaaagttttcattgacttcagagatttcgatttcatgctgtggtgcaaagatggagttgtgcaaacattctatcctagattgcagtcttcatcagaatggcagcctggccaatctatgcctaggctctacaaaatccaaaccatgtgtatggaaaagtgtgagcttcttaactatggtcaacctcctaaattgcctaatggcatacttatgaatgttgccaagtacactcaattgtgccagtacttgaacaaaaccaccatagcagttccagctaaaatgcgtgtcatccattttggtgcaggaagtgaaaaaggtattgcgcctggttccactgtgcttaagcaatggttacctaaagacgctattctagttgacaatgatttgaatgacttcgcatcagatgcagatgtcaccatcattggcaactgtgttacattccacacagagactaagtgggatcttttggtaagtgacatgtatgattgtgactttaaaagtacaactatgggcgaaaactattcaaaggatagtttcttcccatatttgtgtggtttcataaaaaacaagttatctataggcggttcggttgccattaagataacagaacactcttggagtgcagatctttataaccttatgggacattttgcatggtggacagctttctgcaccaatgtaaatgcctcatcatcggaagcatacctaatcggcgtaaactacgtcggtaaagaggttgaaaagattgatggcaacataatgcatgccaattatattttctggaggaattactctccatttaatgtatccaattattctctctttgacatgagcaagtttgcactaaaagccaaagggactcctgtaatgtctctaaaaaaagagcagataaatgaaatggttttgggtcttgttgaaaaaggaagactccttatacgcgacacaaattcatttgttctcaccaatgatatgatggtgaattgttaactaaacgaactttatgaactatttcaacaaaattgtctcgcatagcagacaatttaattttcaaagaccacgcataatcgtagcccgcaaagaagggctttacgagtgtgtgatattttatcggacttacgccgttaaaggttacggaacaacatgaactccttctccacaagcgccttcggtccagttgccttctccctgggcctgctcctggtgttgcctgctgccttccctgccccagtcttcacactcgaagatttcgttggggactggcgacagacagccggctacaacctggaccaagtccttgaacagggaggtgtgtccagtttgtttcagaatctcggggtgtccgtaactccgatccaaaggattgtcctgagcggtgaaaatgggctgaagatcgacatccatgtcatcatcccgtatgaaggtctgagcggcgaccaaatgggccagatcgaaaaaatttttaaggtggtgtaccctgtggatgatcatcactttaaggtgatcctgcactatggcacactggtaatcgacggggttacgccgaacatgatcgactatttcggacggccgtatgaaggcatcgccgtgttcgacggcaaaaagatcactgtaacagggaccctgtggaacggcaacaaaattatcgacgagcgcctgatcaaccccgacggctccctgctgttccgagtaaccatcaacggagtgaccggctggcggctgtgcgaacgcattctggcgtaatctaaacgaacgtttagttattgcacttttattcgtcccgatagctcttgtagccatgattgaacaagatggattgcacgcaggttctccggccgcttgggtggagaggctattcggctatgactgggcacaacagacaatcggctgctctgatgccgccgtgttccggctgtcagcgcaggggcgcccggttctttttgtcaagaccgacctgtccggtgccctgaatgaactgcaagacgaggcagcgcggctatcgtggctggccacgacgggcgttccttgcgcagctgtgctcgacgttgtcactgaagcgggaagggactggctgctattgggcgaagtgccggggcaggatctcctgtcatctcaccttgctcctgccgagaaagtatccatcatggctgatgcaatgcggcggctgcatacgcttgatccggctacctgcccattcgaccaccaagcgaaacatcgcatcgagcgagcacgtactcggatggaagccggtcttgtcgatcaggatgatctggacgaagagcatcaggggctcgcgccagccgaactgttcgccaggctcaaggcgagcatgcccgacggcgaggatctcgtcgtgacccatggcgatgcctgcttgccgaatatcatggtggaaaatggccgcttttctggattcatcgactgtggccggctgggtgtggcggaccgctatcaggacatagcgttggctacccgtgatattgctgaagagcttggcggcgaatgggctgaccgcttcctcgtgctttacggtatcgccgctcccgattcgcagcgcatcgccttctatcgccttcttgacgagttcttctgatcagattaattttactaaatctaaaattaaaataaacgaactattctctcacatcctaaatggctgctgaggggcaaagagtcacttttttgactcaaggttcaaaccaaaataacaacaaccaggaaaaccaagatggacgtggcgctagacccaaaactagaaagcctcgtccagctccacaaaataacgtatcttggtttacgcctcttacccaacatggaaaacaagcgcttacttttaacccaggacaaggagtgccgctcaacgcaaatgacgatcctgacagccgcatcggctactggcgtcgcaacattcgcacagttacaaagaacggcaaaccacagaaattggacccgcgctggtacttttactatcttggcacaggccctgagcaaaacctcaagtacctccagcaaaaggacggaattgtctgggttgcagctcacggtgcccttaatgttccagttaaaacagttgggaccagaaatccagcaaacgatcaagctatcgttgctgcatttgcgccaggtaccgaactgcccaagggtttctatgttgaaggtagcagatctacatcatccgcttcttcagcagcgtcttcaagatcaaattcgcgcagcagaaactctagcctctctcgcagctcttctcccggacgaggattgccaccagcaaccgaccctaacggagttctagctgccttgctcctgactaaattggaagcgcttgatgcaaaagtaaatggcccaaaacaacccccagttgtcacaaagaaaacagcagctgaaattgctgccaaacctaggcagaaacgcgtagcccataaaggttacaatgtaaatgctgcctatggacgccgaggcccaggaccataccagggtaatttcggcacacaagaattcaacaaattgggaacagactatccaaaatggccccaaattgctcaacttgcccctacaccgtcagcattcttcggaatgagtcgattcgcagttcagaagaacgacgatggcacttggctgacataccatgggcatattaaaatggatgaaagtgatcctaacttccaagtatggatgactgaactccagcaaaatattgatgcttacaagaacttcccccagaaagaggaaaagaaaagccgtaagccaaaaaccaagaatgtcgacatggcaccccaagatgtaatgggagctgcagctgtcgaccttgaatgggactcgtctattgaccagacgggacctaatacaattgttgtaaaacctaagaagcagcgcaaacctgctgccgacaacaacatctctgaaatctgaaaaattcgcaagtagtaaggcgtagtataccctaccagtaggactgggttgctattcctacacttgtgctgaatggattctatgtatagtgtagcacaagaagacactatacacgtttactatcactgtctttgacatttagtgtatagttgattggagtaattacaaagaatacacaccgaggccacgccgagtaggaacgagggtacagtgtgaaaagccgatgtcaatgaccggaagagccaatcaatgtaaaattaataatcaaagaacccccagtgattttaatagctttttagtagaattgcaaaaaaaaaaaaaaaaaaaaaaaaaaaaaaaaggccggcatggtcccagcctcctcgctggcgccggctgggcaacattccgaggggaccgtcccctcggtaatggcgaatgggacccactgtgccttctagttgccagccatctgttgtttgcccctcccccgtgccttccttgaccctggaaggtgccactcccactgtcctttcctaataaaatgaggaaattgcatcgcattgtctgagtaggtgtcattctattctggggggtggggtggggcaggacagcaagggggaggattgggaagacaatagcaggcatgctggggatgcggtgggctctatgg

SEQ ID NO: 20 - DNA, 25746 bp, synthetic construct
  source 1..25746: mol_type = other DNA
gttgacattgattattgactagttattaatagtaatcaattacggggtcattagttcatagcccatatatggagttccgcgttacataacttacggtaaatggcccgcctggctgaccgcccaacgacccccgcccattgacgtcaataatgacgtatgttcccatagtaacgccaatagggactttccattgacgtcaatgggtggagtatttacggtaaactgcccacttggcagtacatcaagtgtatcatatgccaagtacgccccctattgacgtcaatgacggtaaatggcccgcctggcattatgcccagtacatgaccttatgggactttcctacttggcagtacatctacgtattagtcatcgctattaccatggtgatgcggttttggcagtacatcaatgggcgtggataggggtttgactcacggggatttccaagtctccaccccattgacgtcaatgggagtttgttttggcaccaaaatcaacgggactttccaaaatgtcgtaacaactccgccccattgacgcaaatgggcggtaggcgtgtacggtgggaggtctatataagcagagctcgtttagtgaaccgagtttgagcgattgacgttcgtaccgtctatcagcttacgatctcttgtcagatctcattaaatctaaactttttaaacaagattccctgttatccatgcttgtgagtgtggtttaatcataatcttgtattttactttccacacttttcatctctctgccagtgacgtgttggttgtcctcagcgtccctcccataggtcgcaatgattaaaaccagcaaatacgggctcggcttcaagtgggcgccagaatttcgttggctgcttccggatgcagcggaggagttggctagtcctatgaagtcagatgagggtgggttatgcccctctactggtcaagcgatggaaagtgttggattcgtttatgataatcatgtgaagatagattgtcgctgcattcttggacaagaatggcatgtgcagtcaaatcttatccgtgatatttttgttcatgaagatctacatgttgtagaagttctaactaaaacagccgtaaagtccggtacggcaattttaattaaatcacctttgcatagcttgggtggttttcctaaagggtatgttatgggcttgttccgttcatacaagactaaacgttatgttgtacatcatctttctatgactacatctactactaattttggtgaagattttttgggttggattgtaccttttggttttatgccatcttatgttcacaaatggtttcaattctgtaggttgtatattgaagagagtgatttaataatttcaaattttaaatttgatgattatgattttagtgtagaagatgcttatgctgaggttcatgctgagcctaaaggtaaatattcacaaaaagcttatgctttacttagacaatatcgtggtattaaacccgtactttttgtagaccagtatggttgtgactattctggtaaattagcagattgtcttcaagcttatggtcattattctttgcaagatatgagacaaaagcagtctgtatggcttgccaattgtgactttgatattgtagtggcttggcatgtagttcgtgattcacgatttgttatgcgcctgcagactatagctactatttgtggtattaaatatgttgcacaacctacagaagatgtagtagatggagatgtagttatacgtgaacctgtacatttattatctgctgatgcaatagttttaaagcttcctagtttgatgaaagttatgactcatatggatgatttttctattaaatctatatataatgttgatttgtgtgattgtggttttgttatgcagtatggttatgtagattgttttaatgataattgtgatttttatggttgggtttcaggtaatatgatggatggtttttcttgtccattgtgttgtacagtttatgactctagcgaagttaaagcccaatcatctggtgttattcctgaaaatcctgtgttatttactaatagtactgatactgttaaccatgattcttttaatttgtatggttattctgtcacaccatttggttcttgtatatattggtcgccgcgtcctggattgtggattcctataattaaatcttcagtcaagtcttatgatgatttggtttattcaggtgtagtaggttgtaaatctattgttaaagaaactgctcttattactcatgcactttacttagattatgttcaatgtaagtgtggtaatcttgaacaaaatcatattcttggcgttaataattcttggtgtaggcaactgttgcttaatagaggtgattataatatgcttctaaaaaatattgacttgtttgttaagcgtcgtgctgattttgcttgcaagtttgcagtttgtggagatggttttgtaccttttttactagatggtttaattccccgtagttattatctaattcagagtggtattttctttacatctttgatgtctcaattttcacaagaagtttctgatatgtgtttaaaaatgtgtattttgtttatggacagagtttcagttgctacattttatatagagcattatgttaataggttggttactcaatttaagttattgggtactacacttgttaataaaatggttaattggtttaataccatgttagatgctagtgcacctgctacaggctggcttctttaccaattattgaatggtctttttgtagtatctcaagccaactttaattttgttgctttaatacctgattatgctaaaattttagttaataaattttacactttttttaagttattattagagtgtgttacagttgatgttttaaaagatatgcctgttcttaaaactattaatggtttagtttgtattgtaggcaataagttttataacgttagtacagggttaattcctggttttgttttaccatgtaatgcacaggaacaacaaatttatttttttgaaggcgttgcagaatctgttatagtagaagatgatgttattgagaatgtcaaatcttctttatcatcttatgagtattgtcaaccacctaaatctgtagaaaaaatttgtattatagataatatgtacatgggtaagtgtggtgataaatttttccctattgtcatgaatgataaaaatatttgtcttttagatcaggcttggcgttttccatgtgcaggtagaaaagttaattttaacgagaaacctgttgttatggagattccgtctttgatgacagttaaggttatgtttgatttagattctacttttgatgatattttaggtaaagtttgttcagaatttgaagtagaaaagggtgttactgtagatgattttgttgctgttgtttgtgatgctatagagaatgctttaaactcttgtaaagagcatccagtggttggttatcaagttcgtgcatttttaaataaacttaatgagaatgttgtttatttatttgatgaggctggtgatgaagcaatggcctctcgtatgtattgtacttttgctattgaggatgttgaagacgttatcagtagtgaagctgtcgaagatactattgatggtgtcgttgaagacactattaatgacgatgaagatgttgttactggtgacaatgacgatgaagatgttgttactggtgacaatgacgatgaagatgttgttactggtgacaatgacgatgaagatgttgttactggtgacaatgacgatgaagatgttgttactggtgacaatgacgatgaagatgttgttactggtgacaatgacgatgaagatgttgttactggtgacaatgacgatgaagatgttgttactggtgacaatgacgatgaagatgttgttactggtgacaatgacgatgaagatgttgttactggtgacaatgacgatgaagatgttgttactggtgacaatgacgatgaagatgttgttactggtgacaatgacgatgaagatgttgttactggtgacaatgacgatgaagatgttgttactggtgacaataacgatgaagagattgttactggtgacaatgatgaccaaattgttgttactggtgatgatgtagatgatattgaaagtatttatgactttgatacttataaagctcttttagtttttaatgatgtctataatgatgctttgtttgttagttatggttctagtgttgaaacagaaacatattttaaagttaatggtttatggtcacctactattacacatactaattgttggttgcgttctgtgttacttgtaatgcagaaattaccttttaagtttaaggatttagctattgaaaatatgtggttatcttataaggtgggttataatcaaagttttgttgattatttactgaccactattcctaaagctattgttttgcctcaaggtggttttgtagctgattttgcttattggtttttaaaccagtttgatattaatgcgtatgctaattggtgttgtttaaaatgtggtttttcttttgatttaaatggtttggatgctttgtttttttatggagatattgtgtctcatgtttgtaagtgtggacataatatgactctaatagcagcggacttaccttgtacattacatttttcattatttgatgacaatttttgtgctttttgcacccctaaaaaaatttttattgctgcatgtgctgtggatgtaaacgtttgtcattctgtagctgttataggtgatgaacaaatagatggtaagtttgttactaaatttagtggtgataaatttgattttatagtaggttatggaatgtcatttagtatgtcttcttttgagttacctcaattgtatggtttgtgtataacacctaatgtatgttttgttaaaggtgatattataaatgttgctagacttgttaaagctgatgttattgttaatcctgctaatgggcatatgctccatggtggtggagttgcaaaagctatagctgtagctgcaggtaaaaaattttctaaagaaactgctgctatggttaaatctaaaggtgtttgccaagtaggagattgttatgtttctaccggtggtaaattatgtaaaacaattcttaatattgtaggccctgatgctagacaagatggaagacaatcttatgttttgttagcacgtgcttataagcatcttaataattatgattgttgtttgtctactctcatatcggctggtatatttagtgttcctgctgatgtgtcattaacttaccttctaggtgttgttgataaacaagttatccttgttagtaataataaagaagattttgatattattcaaaaatgtcaaattacttcagttgttggtactaaagcattggctgttagattaactgctaatgtaggccgtgttattaaatttgagacagatgcatacaaactttttttgagtggtgatgattgttttgtttcaaattcttctgttatacaagaagttttattgcttcgtcatgatatacaattgaataatgacgttcgtgattatttgttgtctaagatgactagtcttcctaaagattggcgtcttatcaataaatttgatgttattaacggtgttaaaactgttaagtattttgagtgtcctaattctatttatatatgtagtcagggtaaagactttggttatgtatgtgatggttctttttataaagcaactgttaatcaagtttgtgttttattagctaagaagatagatgttttgcttactgtagatggtgttaattttaaatctatttctcttactgtaggtgaagtttttggtaaaatacttggtaatgttttctgtgatggcattgatgttactaagttaaagtgtagtgatttttatgccgataaaattttatatcagtatgaaaatttgtctttagctgatatttctgctgtacaaagttcatttgggtttgatcagcaacaattgcttgcttattataattttttaacagtatgtaaatggtctgtagttgttaacggtccatttttttcttttgaacagtctcataataattgttatgtgaatgtagcttgtcttatgttgcagcatattaatcttaaatttaataaatggcagtggcaggaagcatggtatgaatttcgtgctggcagaccacataggttagttgctcttgttttagctaaaggtcattttaaatttgatgaaccatcagatgctactgattttattcgtgttgttttgaaacaagctgatttatcaggtgcaatttgtgaattagaacttatttgtgattgtggtattaaacaagaaagtcgtgttggtgttgatgctgttatgcattttggtacattagcaaagactgatctttttaatggttataagattggctgtaattgtgcaggtagaattgtccattgtactaaattgaatgtaccatttttgatttgttctaatactcctctgagtaaggatttacctgatgatgttgttgcagctaacatgtttatgggtgtaggtgtaggccattatacacatttgaaatgtggttcaccttaccaacattatgatgcttgtagtgttaaaaaatatacaggtgttagtggttgtttaactgactgcttgtatcttaaaaatttaacccagacttttacatctatgttgactaattattttttggatgatgttgaaatggttgcttataaccctgatctttcacaatattattgtgataatggtaagtattatacaaaacctattataaaggctcagtttaaaccatttgctaaagttgacggtgtttatactaactttaagttagttggacatgatatttgtgctcaattgaatgataagttaggttttaatgtagatttgccgtttgttgagtacaaagtaacagtctggcctgtagctactggtgatgttgttttggcatctgatgatttatatgtgaaacgttattttaaaggatgtgaaacttttggtaagcctgttatttggttttgtcatgatgaagcatcattgaattctcttacttattttaataaacctagttttaaatctgaaaatagatatagtgttttgtctgttgattctgtatctgaggagtcacaaggtaatgtggttacttctgttatggaatcgcagattagtactaaagaggttaagttaaagggtgttagaaagactgttaaaatagaagatgctattattgttaatgatgaaaatagttctattaaggttgttaaaagtttatctttagttgatgtttgggatatgtatttgacaggttgtgattatgttgtttgggttgctaatgaattgtcacgcctagttaaatcaccaacagttagggaatatatacgatatggtattaaacctattactatacctatagatttgttatgtttaagagatgataatcaaactcttttagttcctaaaatttttaaagcaagagctatagaattttatggttttttgaagtggttgtttatttatgtttttagtttattacattttacaaatgataaaaccattttttatactacagaaatagcttctaagtttacttttaatttgttttgtttggctcttaaaaatgcttttcagacatttagatggagtatatttataaaaggttttcttgttgtagccactgtgtttttgttttggtttaattttttgtatataaatgttatttttagtgacttttatcttcctaatattagtgtttttcctatttttgtgggaagaattgttatgtggataaaggctacttttggtttggttacaatttgtgatttttattctaagttaggtgtaggttttacaagtcatttttgtaatggtagttttatatgtgaattgtgtcattctggttttgatatgttggatacatatgcagctatagattttgttcagtatgaagtagatagacgtgttttatttgattatgttagtttagtcaaattaattgttgaactcgttattggttattcattatacacagtatggttttatccattattttgtcttattggtttacaattatttactacatggttgcctgatttgtttatgttagaaactatgcattggttgattagatttattgtatttgtagctaatatgttacctgcttttgtcttgttgcggttttatatagttgttactgctatgtataaagtagttggttttattaggcatattgtctatggttgtaataaagctggttgtttattttgttataaacgaaattgtagtgttcgtgttaagtgtagtactattgttggtggtgtaattcgttattatgatattactgctaatggtggtactggtttttgtgttaaacatcaatggaattgttttaattgccattcttttaaaccaggtaacacttttataactgtagaagctgctatagaactttctaaagagcttaaacgacctgtaaatccaactgatgcttcacattatgtagttactgatattaagcaagttggttgtatgatgcgtttgttctatgatagagatggacagcgtgtttacgatgatgttgatgctagtttatttgtagatattaataatctgttacattctaaagttaaagttgttcctaatttgtatgtagttgtagtagagagtgatgctgatagagctaattttctgaatgctgttgtgttttatgcacaatcattgtataggcctatattacttgtagacaaaaagttaattactacagcttgtaatggtatctctgtaacccagactatgtttgatgtttatgttgatacttttatgtctcattttgatgttgatagaaagagttttaataattttgttaacattgctcatgcttctcttagagagggtgtgcaattagaaaaggttttagatacttttgtgggatgtgtacgtaaatgttgttccattgattcagatgttgaaacaagatttattactaaatctatgatatctgcagtagctgctggtttggaatttactgatgaaaattataacaatttggtacctacatatttaaagagtgataatattgtagctgctgatttaggtgttcttatacagaatggtgctaagcatgtacagggtaatgttgctaaggcagctaatatttcttgtatatggtttattgatgcttttaatcaacttactgctgatttacagcataaattaaaaaaagcatgtgttaaaactggcttgaagttaaaattgacttttaataagcaagaggcaagtgtccctattcttacaacacccttttcacttaaaggaggtgttgtattgagtaatttgttatatatattattttttgttagtttaatctgttttatattattgtgggctttattgcctacatatagtgtttataagtctgatattcatttgcctgcttatgctagttttaaagttattgataatggtgttgttagagatatttcagttaatgatttatgttttgctaataaatttttccaatttgatcaatggtatgagtccacttttgggtctgtttactatcataattctatggattgccctattgtagtggcagttatggatgaagatatcggttctactatgtttaatgttcctactaaagttttgagacatggctttcatgttttacattttttaacttatgcatttgctagtgatagtgttcagtgctatacaccacatattcagatttcttataatgatttttatgctagtggttgtgttttatcatctttgtgtactatgtttaaaagaggtgatggtacaccacatccttattgttattcagatggtgttatgaagaatgcttctttgtatacatctttggttccacatacacgttatagccttgctaattctaatggttttataagatttcctgatgttattagtgaaggtattgtacgtattgtaagaacgcgctctatgacttattgtagagtgggtgcatgtgaatacgccgaagagggtatatgttttaattttaatagttcctgggttttgaataatgattattatagaagtatgcctggaactttttgtggtagagatctttttgatttgttttatcaattttttagtagtttaattcgtcctatagatttcttttctcttactgctagttctatttttggagctatattggctatagttgttgtcttggttttttattatttaataaaacttaagcgtgcttttggagattatactagtgttgtagttataaatgttgttgtttggtgtattaattttcttatgctttttgtttttcaagtttatcctatttgtgcatgtgtttatgcttgtttttatttttatgtaacattgtattttccttctgaaattagtgtaattatgcatttgcaatggattgttatgtatggtgctataatgcctttttggttttgtgtcacatatgtagctatggttattgcaaaccatgttttatggttattttcatattgtaggaaaattggtgttaatgtatgtagtgatagtacatttgaagaaacatctcttactacttttatgattactaaagattcttattgtagattaaagaattctgtttctgatgttgcctacaatagatatttgagtttgtataataagtatcgttactatagtggtaaaatggatactgctgcctatagagaagcggcgtgttctcagttagctaaagctatggaaacatttaatcacaataatggtaatgatgtcttataccaacctcctacagcatctgtttctacatcttttttgcaatcaggtattgtaaagatggtatctcctacgtcaaaaattgaaccttgtattgttagtgttacttatggtagtatgactttgaatggtttatggttagatgacaaagtttattgtcctcgtcatgttatatgttcatcctctaatatgaacgaacctgattattctgccttattgtgtagagttactctaggtgattttactataatgtctggtcggatgagtttaacagttgtgtcttaccagatgcagggctgtcaacttgttttgacagtctctttacaaaatccttacactccaaaatatacttttggtaatgttaaacctggtgaaacttttactgttttagctgcgtataatggccgaccacaaggggcatttcatgttactatgcgtagtagttatactattaaaggttcttttttgtgtgggtcatgtggatctgttggttatgtattaacaggtgatagtgttaagtttgtatatatgcatcaattagagctcagtactggttgtcacactggcactgattttactggtaatttttatggtccatatagagatgctcaagttgtacagttgccagttaaggactacgtccagactgttaatgttattgcttggctctatgcagctatacttaataattgtgcttggtttgtacaaaatgatgtttgttctactgaagattttaatgtttgggctatggcaaatggttttagccaagtaaaagcagatcttgtcttagatgctttggcttcaatgacaggtgtttctattgaaactttattggctgctattaagcgtctatatatgggatttcaaggtcgtcaaatactaggaagttgtacttttgaagatgaattggcaccttctgacgtttatcaacaattggctggtgttaaattgcaatctaaaacaaaaagatttattaaagaaacaatttattggattttgatatctacatttttgtttagttgtataatttctgcatttgttaaatggactatatttatgtatattaatacacatatgattggtgttacattatgtgtactttgttttgttagttttatgatgttactagttaaacataagcatttttatttgactatgtatataattcctgtactctgtaccttgttttatgtaaattatttagttgtttataaggaaggttttagaggttttacttatgtctggctctcatattttgttcctgctgtgaattttacttatgtttatgaagtattttatggttgtattttatgtgtttttgctatttttataactatgcatagtattaatcatgacattttttctttgatgtttttggttggtagaatagttactttaatttctatgtggtattttgggtcgaatttagaagaggatgttttgttatttattacagcctttttaggtacttatacatggaccactattttgtcattagctatagcaaaaattgttgctaattggttgtctgttaatatattttattttacagatgtaccttatattaaattgattctcttgagttacttatttatagggtatattttatcttgttattggggatttttctctcttttaaacagtgtttttagaatgcctatgggtgtttataattataaaatttctgttcaagaattgcgttatatgaatgctaatggcttacgtccacctcgtaatagttttgaggctattttgttaaatttaaaactgcttggaataggtggcgtgccagttattgaagtctcccaaattcaatcaaaattgactgatgtgaaatgtgctaatgttgttttgttaaattgtttacagcatttgcatgttgcttctaattctaagttgtggcagtattgtagtgttttacataatgaaatactatctacttcagatttgagtgtagcttttgataagcttgctcaattattgattgttttattcgccaatcctgctgcagttgatactaagtgtcttgcaagtatagatgaagttagcgatgattatgttcaagatagtaccgttttgcaggctttgcaaagtgagtttgtaaatatggctagttttgttgaatatgaagtcgcaaagaaaaatttggctgatgctaaaaatagtggttctgttaatcaacaacagataaaacagttagaaaaagcatgtaatatagctaagtctgtgtatgaacgtgataaagctgtagctcgcaaacttgaacgtatggcagacctagcacttactaacatgtataaagaggctcggattaatgataagaagagtaaagttgtttccgctttgcagacaatgctttttagcatggttcgtaaattggataatcaggctttaaattctattctggataatgctgttaaaggttgtgtacctttgagtgctattccagcattggctgctaatactttaactatagtaataccagataaacaagtttttgataaagttgttgataatgtttatgttacatatgctggtagtgtatggcatatacagactgttcaagatgctgatggtattaataaacagttaactgatattagtgttgattctaattggcctcttgttatcattgcgaacaggtataatgaagttgctaatgctgttatgcagaataatgagttgatgcctcataaattaaaaatacaagttgttaatagtggttctgatatgaattgtaatattcctactcaatgttattataataatggtagtagtggtagaatagtttatgctgttcttagtgatgttgatggtcttaagtatactaagataatgaaagatgatggaaattgtgttgttttagagcttgatcctccttgtaaattttctatacaagatgttaagggacttaaaattaagtatctttattttattaaaggatgtaacactttagctagagggtgggttgttggtactttatcttcaacaattagattgcaggctggtgttgctactgagtatgcagctaattcttctatactttcattatgtgcattttctgtagatcctaagaaaacttatttagattatatacaacaaggtggtgtacctataattaattgtgttaaaatgctctgtgatcatgctggtactggtatggccattactattaaacctgaggctactattaaccaagattcttatggtggtgcctcagtttgtatttattgccgtgcacgtgtagagcatccagatgtagatggtatatgtaaattacgtggtaaatttgtacaagtccctttgggtataaaagatcctattctttatgtgttaacacatgatgtttgtcaagtctgtggtttttggagagatggcagttgttcctgtgtaggttcaagtgtcgctgttcaatctaaagatttaaattttttaaacgggttcggggtactagtgtgaatgcccggctagtaccctgtgctagtggtttatctactgatgttcaattaagggcatttgacatttgtaataccaatagagctggtataggtttatattataaagtgaattgttgccgttttcagcgtatagatgacgacggtaataaattggataagttctttgttgtcaaaagaactaatttagaagtttataataaagagaaaacttattatgagttgactaaaagttgtggtgttgtggctgaacatgatttctttacatttgatattgatggtagtcgcgtgccacatatagttcgtaggaatctttcaaagtatactatgttagatctttgctatgcattgcgtcattttgatcgtaatgattgttcaatattgtgtgaaattctttgtgagtatgctgattgtaaagaatcctacttttctaagaaagattggtatgattttgttgaaaatcctgatattattaatatatataaaaaattaggccctatttttaatagagctttacttaatactgtcatttttgcagacaccttagttgaagtaggtttagttggtgttttaactttagataaccaagatttgtatggtcaatggtatgattttggtgattttatacaaacagccccagggtttggtgtggcagttgcagattcttactattcttatatgatgcctatgttgactatgtgtcatgtattagattgtgaattatttgttaatgatagttatagacaattcgatcttgtacagtatgattttactgattacaagttagagttgtttaataagtattttaagtattggggtatgaagtatcatcctaatactgtggattgtgataatgataggtgtattattcattgtgctaattttaatatactatttagtatggttttacctaatacttgttttggtccccttgttagacaaatttttgtagatggtgtaccgtttgttgtttctattggttaccattacaaagagttaggtgtagttatgaacttagatgttgacacacaccgttatcgtttgtctcttaaagatttacttctttatgcagcagatcctgctatgcacgttgcatctgctagtgctctgcttgatttacgaacttgttgttttagtgtagctgccattacaagtggtataaaatttcaaactgtaaaaccaggtaactttaaccaagacttttacgagtttgttaaaagtaaaggcttgtttaaagagggtagtacagttgatttgaaacattttttctttactcaagatggtaatgctgcaattactgattataattattataagtataatttacctactatggttgatattaagcagttattgtttgtattagaagttgtttataaatattttgaaatttatgatggtggttgtataccagcatcacaagttattgttaataattatgataaaagtgctggttatccatttaataaatttggtaaagccagactttattatgaggcattatcatttgaggaacagaatgaaatttatgcatatactaaacgtaatgttctgcccaccttaactcaaatgaatttaaaatatgctatcagtgctaagaatagagctcgcactgtagcaggtgtttctattcttagtactatgacaggccgaatgttccatcaaaaatgtttgaagagtatagcagctacccgaggtgttcctgttgttataggaaccactaaattttatggtggttgggacgatatgttacgtcatcttataaaggatgttgacaaccctgttcttatgggttgggattatcctaaatgtgatcgtgctatgccaaatattttgcgtattgttagtagtttagttttggcccgcaaacatgaattttgttgttcacatggtgatagattttatcgccttgcgaatgaatgtgctcaagttttgagtgaaatagttatgtgtggcggttgctattatgttaagcctggtggtactagcagtggtgatgcaactactgcttttgctaattctgtttttaatatatgtcaggctgttactgctaatgtttgttctcttatggcctgtaatggccataagattgaagatttaagtatacgcaatttacaaaaacgcttatactctaatgtttatcgtacagattatgttgattatacatttgttaatgagtattatgaatttttatgtaagcattttagtatgatgattttgagtgatgatggtgttgtctgttataactctgattatgctagtaagggttatatagctaatataagtgtttttcaacaagttttgtactatcagaataatgtctttatgtctgaatctaaatgttgggttgaaaatgatattactaatggtcctcatgaattttgttcccaacatactatgttagttaagatagatggtgattatgtttatttaccatatccagatccttctagaattttaggagctggttgttttgttgatgatttattgaagactgacagtgttcttttgatagagcgctttgtaagtctagctatagatgcttaccctttagtacatcatgaaaatgaagaataccaaaaagtctttcgtgtatatttagaatatataaaaaaactgtataatgatcttggtactcagatcttagatagttatagtgttattttaagtacttgtgatggtttaaagtttactgaagaatcattttacaagaatatgtatttaaaaagtgccgtgatgcagagtgtaggtgcatgcgttgtttgttcatcacaaacttctttgcgttgtggcagttgtatacgtaagcctttgttatgttgtaaatgttgttatgaccatgttatggcaactaatcataaatatgttttgagtgtctcaccttacgtttgtaatgcacctaactgtgatgtgagtgatgtcaccaaattatatttgggcggtatgtcttactattgtgaaaaccataaaccccattattcatttaagttagttatgaatggtatggtctttggtttgtataaacaatcttgcacgggttcaccttatatagatgattttaataagatagctagttgtaaatggacagaagttgatgattatgttctggcaaatgagtgtattgaacgtttaaagttatttgctgcagaaactcaaaaggcaactgaagaggcttttaaacaaagctatgcttctgctaccattcaagagattgttagtgatagagaagttattttgtgttgggagacaggtaaagttaaaccaccacttaataaaaattatgttttcacaggctaccattttactagtactggtaagacagttttaggtgagtatgtttttgataaaagtgaattaactaacggtgtgtattaccgcgctacaactacttataaactttctataggtgatgtttttgttttaacatcacattctgtagctagtttaagtgcacctacacttgtcccacaagagaactatgctagtataagattttctagtgtttatagtgttccattggtgtttcaaaataatgttgctaattatcagcacattggaatgaaacgttattgcactgttcaaggtccccctggtacgggaaagtctcatcttgctataggtctagctgtttattactacacagcacgtgtagtttatactgctgctagtcatgctgctgtagatgcattgtgtgaaaaagcttataagtttttaaatattaacgattgtacacgtattattcctgctaaagttcgtgtagattgttatgataagtttaaaattaatgataccacttgtaagtatgtttttaccacaataaatgcattaccagagttggttacagatattgttgttgttgatgaagttagtatgcttactaattatgaattgtctgttataaatgctcgtattaaagctaaacattatgtatatattggagatcctgctcaattacctgcaccacgtgtgctgttgagcaagggttctttagaacctaggcacttcaattctattactaaaataatgtgttgtttaggtcctgatatctttttgggaaattgttataggtgtcctaaagaaattgtagaaactgtttcagcattggtttatgataataaactcaaggctaaaaatgataatagttcattatgttttaaagtatattttaagggacagacaacacatgagagttcaagtgctgtaaatattcaacagatatatctaattagtaaatttttaaaagctaatccagtttggaatagtgctgtttttattagtccttataatagtcagaattatgttgctaagcgtgttttaggtgttcaaacacaaactgtagattctgctcaaggttcggaatatgattatgttatatattcacaaacagcagaaacagcccattctgttaatgttaatcgatttaatgttgccataactagagccaagaagggcattttttgtgttatgagtaatatgcaattatttgaatctcttaattttattactctacctttagataaaattcaaaatcaaactttacctcgtttgcattgcacaactaatctttttaaagattgtagtaaaagttgcttaggttatcatccagcgcatgccccctcatttttagcagttgatgataaatataaggttaatgaaaatttggctgtaaatttaaatatttgtgaacctgttttaacatattctcgtttaatatctcttatgggttttaaattagatttgactcttgatggttattctaaattgtttattactaaagatgaagccattaaacgtgttagaggttgggttggttttgatgttgagggcgctcatgctactcgcgaaaacattggaacaaactttccactgcaaataggtttttcaactggtgtggattttgtagttgaagctactggcttatttgctgagagagattgttatacttttaaaaaaactgtagctaaagctcctcctggtgaaaaatttaaacatttaataccccttatgtcaaaaggtcaaaagtgggatattgttagaattagaattgttcaaatgttatctgattatcttttagacctttctgatagtgtagtatttattacttggtctgccagttttgaacttacttgtttaaggtattttgctaaattaggcagagagcttaattgtaatgtgtgttctaatcgtgctacatgctacaattctagaactggttattatggttgttggcgccatagttatacttgtgattatgtgtataatccacttattgtagatatacaacagtggggttatacaggttctttaactagtaatcacgatataatttgtaatgtacataaaggtgcacatgttgcgtcagctgatgcaattatgactcgttgtttagcaatctatgattgtttttgtaaatctgttaattggaatttagagtatccaataatttctaatgaggtcagtataaatacatcttgtaggttattgcagcgtgtcatgcttaaagctgccatgctatgtaatagatacaacttatgttatgacataggcaatcctaaaggtttagcttgtgtcaaagattatgaatttaaattttatgatgcttttcctgtagccaagtctgttaaacagttattttatgtctatgatgtgcataaagataattttaaagatggtttatgtatgttttggaattgtaatgttgataaatatccatctaattcaattgtttgtagatttgacactcgagtgttaaataaattaaaccttcctggatgtaatggtggtagtttgtatgttaataaacatgcattccatactaatccttttactagaactgtttttgaaaatcttaagcctatgccttttttctattattcagatacgccttgtgtgtacgtagatggtttagaatctaaacaagttgattacgttcctttaagaagcgccacttgtatcacacggtgtaatctaggtggagctgtttgttcaaagcatgctgaagaatattgtaactaccttgagtcttataatatagttactacagcaggctttactttttgggtttataagaattttgatttttataatttatggaacacttttactacgttacagagtttagaaaacgtaatatataacttggttaatgttggtcattatgatggacgtacaggtgaattaccttgtgctattatgaatgacaaagttgttgttaagattaataatgtagatactgttatttttaaaaataatacatcatttcctactaatatagctgttgaattgtttacaaaacgtagtatccggcaccaccctgaacttaagattcttagaaatttgaacattgatatttgttggaagcatgtcctgtgggattatgttaaagatagtttgttttgtagttccacttatggtgtttgtaaatacacagatttgaagttcatcgaaaatttgaatatactttttgatggtcgtgacactggcgctttagaagcttttagaaaagcaagaaatggtgtttttattagtactgaaaaattaagtaggttatcaatgattaaaggtccgcaacgagctgatttaaatggtgtgattgtggataaagttggagaactcaaagttgagttttggttcgctatgagaaaagatggtgacgatgttatcttcagccgaacagacagcctatgctcaagccattactggagcccacaaggtaatctaggtggtaattgcgcgggtaatgtcattggtaatgatgctctaacacgttttactatctttactcagagtcgtgtattgtcaagttttgaacctcgctcagatttagaacgggattttattgatatggatgataatctgtttattgctaaatatggtttagaagactatgcatttgatcatatagtttatggtagttttaaccataaagttataggaggtttgcatttgcttataggcttatttcgtaggaaaaaaaaatctaatttgttaattcaagagtttttacagtatgattctagtattcattcatattttattactgatcaggagtgtggtagtagtaagagtgtttgtacagttattgatttattattagatgattttgtttctattgttaagtcattaaatttgagttgtgttagtaaagttgttaatattaatgttgattttaaggattttcaatttatgttgtggtgtaatgataataaaattatgactttttatcctaaaatgcaagccactaatgattggaaacctggctattctatgcctgttttgtataagtatttgaatgttccattagagagagtctctttatggaattatggtaaacctattaatttgcctacaggctgtatgatgaatgttgctaagtacactcaattatgtcagtatttgaatactacaacattagctgttcctgttaatatgcgtgttttacatttaggtgcagggtctgataaagaagtagctccaggttctgctgttttaagacagtggttaccatctggtagtattcttgtagataatgatttaaacccatttgttagcgatagtttagttacttattttggagattgtatgactttaccatttgattgtcattgggatttgataatatctgatatgtatgatcctcttactaaaaatattggtgattataatgtgagtaaggatgggttttttacttacatttgtcatttaattcgtgataaattatctttgggtggtagtgtagctataaaaattacagagttttcttggaatgctgatttatataaattaatgagttgttttgcattttggacagttttttgtactaatgtaaatgcttcttctagtgaagggtttttaataggtataaattacctgggtaaatcttcttttgaaatagatggcaatgttatgcatgctaactatttgttttggagaaatagtacaacatggaatggcggtgcttatagtttatttgatatgactaaattttctttgaaattggctggcactgctgttgttaatttaagaccagatcaattaaatgatttagtttattctcttattgaaagaggtaaattattagttcgcgatacgcgtaaagagatttttgttggtgatagtcttgtaaatacttgttagatctaaacatgaactccttctccacaagcgccttcggtccagttgccttctccctgggcctgctcctggtgttgcctgctgccttccctgccccagtcttcacactcgaagatttcgttggggactggcgacagacagccggctacaacctggaccaagtccttgaacagggaggtgtgtccagtttgtttcagaatctcggggtgtccgtaactccgatccaaaggattgtcctgagcggtgaaaatgggctgaagatcgacatccatgtcatcatcccgtatgaaggtctgagcggcgaccaaatgggccagatcgaaaaaatttttaaggtggtgtaccctgtggatgatcatcactttaaggtgatcctgcactatggcacactggtaatcgacggggttacgccgaacatgatcgactatttcggacggccgtatgaaggcatcgccgtgttcgacggcaaaaagatcactgtaacagggaccctgtggaacggcaacaaaattatcgacgagcgcctgatcaaccccgacggctccctgctgttccgagtaaccatcaacggagtgaccggctggcggctgtgcgaacgcattctggcgtaaatctaaacattatgattgaacaagatggattgcacgcaggttctccggccgcttgggtggagaggctattcggctatgactgggcacaacagacaatcggctgctctgatgccgccgtgttccggctgtcagcgcaggggcgcccggttctttttgtcaagaccgacctgtccggtgccctgaatgaactgcaagacgaggcagcgcggctatcgtggctggccacgacgggcgttccttgcgcagctgtgctcgacgttgtcactgaagcgggaagggactggctgctattgggcgaagtgccggggcaggatctcctgtcatctcaccttgctcctgccgagaaagtatccatcatggctgatgcaatgcggcggctgcatacgcttgatccggctacctgcccattcgaccaccaagcgaaacatcgcatcgagcgagcacgtactcggatggaagccggtcttgtcgatcaggatgatctggacgaagagcatcaggggctcgcgccagccgaactgttcgccaggctcaaggcgagcatgcccgacggcgaggatctcgtcgtgacccatggcgatgcctgcttgccgaatatcatggtggaaaatggccgcttttctggattcatcgactgtggccggctgggtgtggcggaccgctatcaggacatagcgttggctacccgtgatattgctgaagagcttggcggcgaatgggctgaccgcttcctcgtgctttacggtatcgccgctcccgattcgcagcgcatcgccttctatcgccttcttgacgagttcttctgaatctaaactattaggatgtcttatactcccggtcattatgctggaagtagaagctcctctggaaatcgttcaggaatcctcaagaaaacttcttgggctgaccaatctgagcgaaattaccaaacctttaatagaggcagaaaaacccaacctaaattcactgtgtctactcaaccacaaggaaatactatcccacattattcctggttctccgggatcactcaatttcaaaaaggtagagactttaaattttcagatggtcaaggagttcccattgctttcggagtacccccttctgaagcaaaaggatattggtatagacacagccggcgttcttttaaaacagctgatggtcaacaaaagcagttgttaccgagatggtatttctactatctcggtaccggcccatatgccaatgcatcctatggtgaatccctcgaaggggtcttctgggttgctaatcaccaagctgacacttctactccctccgatgtttcgtcaagggatcctactactcaagaagctatccctactaggtttccgcctggtacgattttgcctcaaggctattatgttgaaggctcaggaaggtctgcttctaatagtcgaccaggttcacgttctcaatcacgtggacccaataatcgttcattaagtagaagtaattctaattttagacattcagattctatagtaaaacctgatatggctgatgagatcgctaatcttgttttagccaagcttggtaaagattctaaacctcagcaagtcactaagcaaaatgccaaggaaatcaggcataaaattttaacaaaacctcgccaaaagcgaactcctaataaacattgtaatgttcaacagtgttttggtaaaagaggaccttctcaaaattttggtaatgctgaaatgttaaagcttggtactaatgatcctcagtttcctattcttgcagaattagctcctacaccaggtgcttttttctttggttctaaattagacttggttaaaagagattccgaggctgactcacctgttaaagatgtttttgaacttcattattctggttctattaggtttgatagtactttaccaggctttgagacaattatgaaagttcttgaagagaatttaaatgcttacgttaattctaatcagaacactgattctgattcgttgagttctaaacctcagcgtaaaagaggtgttaaacaattaccagaacagtttgactctcttaatttaagtgctggtactcagcacatttcaaatgattttactcctgaggatcatagtttacttgctactcttgatgatccttatgtagaagactctgttgcttaatgagaatgaatcctaattcgacactaggtggtaacccctcgctattattcggaataggacactctctatcagaatgaattcttgctgtaataacagatagagtaggttgttacagactatatattaattagtagaaattttatatttagacatttgattgttagagtagttataaggtttagctgtagtataaacgcctccgggaagagctatcaattgtagtgtttaatatatatattagtatatgattgaaattaattatagccttttggaggaattacaaaaaaaaaaaaaaaaaaaaaaaaaaaaaaaaaaaaaaaaaaaaaggccggcatggtcccagcctcctcgctggcgccggctgggcaacattccgaggggaccgtcccctcggtaatggcgaatgggacccactgtgccttctagttgccagccatctgttgtttgcccctcccccgtgccttccttgaccctggaaggtgccactcccactgtcctttcctaataaaatgaggaaattgcatcgcattgtctgagtaggtgtcattctattctggggggtggggtggggcaggacagcaagggggaggattgggaagacaatagcaggcatgctggggatgcggtgggctctatgg

SEQ ID NO: 21 - DNA, 42 bp, synthetic construct
  source 1..42: mol_type = other DNA
ggaattcggtctcaatggcagttaacccctacattctacgac

SEQ ID NO: 22 - DNA, 964 bp, synthetic construct
  source 1..964: mol_type = other DNA
ggaattcggtctcaatggcagttaacccctacattctacgacaatagctgtcccaacgtgtccaacatcgttcgcgacacaatcgtcaacgagctcagatccgatcccaggatcgctgcttcaatattacgtctgcacttccatgactgcttcgtgaatggttgcgacgctagcatattactggacaacaccaccagtttccgcactgaaaaggatgcattcgggaacgctaacagcgccaggggctttccagtgatcgatcgcatgaaggctgccgttgagtcagcatgcccacgaacagtcagttgtgcagacctgctgactatagctgcgcaacagagcgtgactcttgcaggcggaccgtcctggagagtgccgctcggtcgacgtgactccctacaggcattcctagatctggccaacgccaacttgcctgctccattcttcaccctgccccagctgaaggatagctttagaaacgtgggtctgaatcgctcgagtgaccttgtggctctgtccggaggacacacatttggaaagaaccagtgtaggttcatcatggataggctctacaatttcagcaacactgggttacctgaccccacgctgaacactacgtatctccagacactgagaggcttgtgcccactgaatggcaacctcagtgcactagtggactttgatctgcggaccccaaccatcttcgataacaagtactatgtgaatctagaggagcagaaaggcctgatacagagtgatcaagaactgtttagcagtccaaacgccactgacaccatcccactggtgagaagttttgctaactctactcaaaccttctttaacgccttcgtggaagccatggaccgtatgggtaacattacccctctgacgggtacccaaggccagattcgtctgaactgcagagtggtcaacagcaactcttaacctctgagaccggatcccg

SEQ ID NO: 23 - DNA, 42 bp, synthetic construct
  source 1..42: mol_type = other DNA
ggaattcggtctcaattacagttaacccctacattctacgac

SEQ ID NO: 24 - DNA, 44 bp, synthetic construct; identical to SEQ ID NO: 11
  source 1..44: mol_type = other DNA

SEQ ID NO: 25 - DNA, 964 bp, synthetic construct
  source 1..964: mol_type = other DNA
ggaattcggtctcaattacagttaacccctacattctacgacaatagctgtcccaacgtgtccaacatcgttcgcgacacaatcgtcaacgagctcagatccgatcccaggatcgctgcttcaatattacgtctgcacttccatgactgcttcgtgaatggttgcgacgctagcatattactggacaacaccaccagtttccgcactgaaaaggatgcattcgggaacgctaacagcgccaggggctttccagtgatcgatcgcatgaaggctgccgttgagtcagcatgcccacgaacagtcagttgtgcagacctgctgactatagctgcgcaacagagcgtgactcttgcaggcggaccgtcctggagagtgccgctcggtcgacgtgactccctacaggcattcctagatctggccaacgccaacttgcctgctccattcttcaccctgccccagctgaaggatagctttagaaacgtgggtctgaatcgctcgagtgaccttgtggctctgtccggaggacacacatttggaaagaaccagtgtaggttcatcatggataggctctacaatttcagcaacactgggttacctgaccccacgctgaacactacgtatctccagacactgagaggcttgtgcccactgaatggcaacctcagtgcactagtggactttgatctgcggaccccaaccatcttcgataacaagtactatgtgaatctagaggagcagaaaggcctgatacagagtgatcaagaactgtttagcagtccaaacgccactgacaccatcccactggtgagaagttttgctaactctactcaaaccttctttaacgccttcgtggaagccatggaccgtatgggtaacattacccctctgacgggtacccaaggccagattcgtctgaactgcagagtggtcaacagcaactcttaaagcttgagaccggatcccg

SEQ ID NO: 26 - DNA, 42 bp, synthetic construct; identical to SEQ ID NO: 7
  source 1..42: mol_type = other DNA

SEQ ID NO: 27 - DNA, 44 bp, synthetic construct
  source 1..44: mol_type = other DNA
cgggatccggtctcacactttaagagttgctgttgaccactctg

SEQ ID NO: 28 - DNA, 964 bp, synthetic construct
  source 1..964: mol_type = other DNA
ggaattcggtctcaggcccagttaacccctacattctacgacaatagctgtcccaacgtgtccaacatcgttcgcgacacaatcgtcaacgagctcagatccgatcccaggatcgctgcttcaatattacgtctgcacttccatgactgcttcgtgaatggttgcgacgctagcatattactggacaacaccaccagtttccgcactgaaaaggatgcattcgggaacgctaacagcgccaggggctttccagtgatcgatcgcatgaaggctgccgttgagtcagcatgcccacgaacagtcagttgtgcagacctgctgactatagctgcgcaacagagcgtgactcttgcaggcggaccgtcctggagagtgccgctcggtcgacgtgactccctacaggcattcctagatctggccaacgccaacttgcctgctccattcttcaccctgccccagctgaaggatagctttagaaacgtgggtctgaatcgctcgagtgaccttgtggctctgtccggaggacacacatttggaaagaaccagtgtaggttcatcatggataggctctacaatttcagcaacactgggttacctgaccccacgctgaacactacgtatctccagacactgagaggcttgtgcccactgaatggcaacctcagtgcactagtggactttgatctgcggaccccaaccatcttcgataacaagtactatgtgaatctagaggagcagaaaggcctgatacagagtgatcaagaactgtttagcagtccaaacgccactgacaccatcccactggtgagaagttttgctaactctactcaaaccttctttaacgccttcgtggaagccatggaccgtatgggtaacattacccctctgacgggtacccaaggccagattcgtctgaactgcagagtggtcaacagcaactcttaaagtgtgagaccggatcccg

SEQ ID NO: 29 - DNA, 42 bp, synthetic construct
  source 1..42: mol_type = other DNA
ggaattcggtctcaagtgcagttaacccctacattctacgac

SEQ ID NO: 30 - DNA, 964 bp, synthetic construct
  source 1..964: mol_type = other DNA
ggaattcggtctcaagtgcagttaacccctacattctacgacaatagctgtcccaacgtgtccaacatcgttcgcgacacaatcgtcaacgagctcagatccgatcccaggatcgctgcttcaatattacgtctgcacttccatgactgcttcgtgaatggttgcgacgctagcatattactggacaacaccaccagtttccgcactgaaaaggatgcattcgggaacgctaacagcgccaggggctttccagtgatcgatcgcatgaaggctgccgttgagtcagcatgcccacgaacagtcagttgtgcagacctgctgactatagctgcgcaacagagcgtgactcttgcaggcggaccgtcctggagagtgccgctcggtcgacgtgactccctacaggcattcctagatctggccaacgccaacttgcctgctccattcttcaccctgccccagctgaaggatagctttagaaacgtgggtctgaatcgctcgagtgaccttgtggctctgtccggaggacacacatttggaaagaaccagtgtaggttcatcatggataggctctacaatttcagcaacactgggttacctgaccccacgctgaacactacgtatctccagacactgagaggcttgtgcccactgaatggcaacctcagtgcactagtggactttgatctgcggaccccaaccatcttcgataacaagtactatgtgaatctagaggagcagaaaggcctgatacagagtgatcaagaactgtttagcagtccaaacgccactgacaccatcccactggtgagaagttttgctaactctactcaaaccttctttaacgccttcgtggaagccatggaccgtatgggtaacattacccctctgacgggtacccaaggccagattcgtctgaactgcagagtggtcaacagcaactcttaacctctgagaccggatcccg

SEQ ID NO: 31 - DNA, 34 bp, synthetic construct
  source 1..34: mol_type = other DNA
atcatcactagtctcacaggccgggacaagaaac

SEQ ID NO: 32 - DNA, 35 bp, synthetic construct
  source 1..35: mol_type = other DNA
cttggtccgtacggcccagttgaagaggtacttgc